European Patent Specification EP 3 591 042 B1, published January 25, 2023. Title: PRRS virus variant, European PRRS virus cDNA clone, and uses thereof. Applicant: Boehringer Ingelheim Vetmedica GmbH. The sequence listing filed with the application follows.

SEQUENCE LISTING (58 sequences)

SEQ ID NO: 1 - protein, 22 aa, Porcine reproductive and respiratory syndrome virus
  misc_feature (2)..(2): Xaa can be any naturally occurring amino acid
  misc_feature (5)..(19): Xaa can be any naturally occurring amino acid
FXVLXXXXXXXXXXXXXXXQCR

SEQ ID NO: 2 - protein, 21 aa, Porcine reproductive and respiratory syndrome virus
  misc_feature (2)..(2): Xaa can be any naturally occurring amino acid
  misc_feature (5)..(18): Xaa can be any naturally occurring amino acid
FXVLXXXXXXXXXXXXXXQCR

SEQ ID NO: 3 - protein, 20 aa, Porcine reproductive and respiratory syndrome virus
  misc_feature (2)..(2): Xaa can be any naturally occurring amino acid
  misc_feature (5)..(17): Xaa can be any naturally occurring amino acid
FXVLXXXXXXXXXXXXXQCR

SEQ ID NO: 4 - protein, 19 aa, Porcine reproductive and respiratory syndrome virus
  misc_feature (2)..(2): Xaa can be any naturally occurring amino acid
  misc_feature (5)..(16): Xaa can be any naturally occurring amino acid
FXVLXXXXXXXXXXXXQCR

SEQ ID NO: 5 - protein, 18 aa, Porcine reproductive and respiratory syndrome virus
  misc_feature (2)..(2): Xaa can be any naturally occurring amino acid
  misc_feature (5)..(15): Xaa can be any naturally occurring amino acid
FXVLXXXXXXXXXXXQCR

SEQ ID NO: 6 - protein, 17 aa, Porcine reproductive and respiratory syndrome virus
  misc_feature (2)..(2): Xaa can be any naturally occurring amino acid
  misc_feature (5)..(14): Xaa can be any naturally occurring amino acid
FXVLXXXXXXXXXXQCR

SEQ ID NO: 7 - protein, 16 aa, Porcine reproductive and respiratory syndrome virus
  misc_feature (2)..(2): Xaa can be any naturally occurring amino acid
  misc_feature (5)..(13): Xaa can be any naturally occurring amino acid
FXVLXXXXXXXXXQCR

SEQ ID NO: 8 - protein, 15 aa, Porcine reproductive and respiratory syndrome virus
  misc_feature (2)..(2): Xaa can be any naturally occurring amino acid
  misc_feature (5)..(12): Xaa can be any naturally occurring amino acid
FXVLXXXXXXXXQCR

SEQ ID NO: 9 - protein, 14 aa, Porcine reproductive and respiratory syndrome virus
  misc_feature (2)..(2): Xaa can be any naturally occurring amino acid
  misc_feature (5)..(11): Xaa can be any naturally occurring amino acid
FXVLXXXXXXXQCR

SEQ ID NO: 10 - protein, 13 aa, Porcine reproductive and respiratory syndrome virus
  misc_feature (2)..(2): Xaa can be any naturally occurring amino acid
  misc_feature (5)..(10): Xaa can be any naturally occurring amino acid
FXVLXXXXXXQCR

SEQ ID NO: 11 - protein, 12 aa, Porcine reproductive and respiratory syndrome virus
  misc_feature (2)..(2): Xaa can be any naturally occurring amino acid
  misc_feature (5)..(9): Xaa can be any naturally occurring amino acid
FXVLXXXXXQCR

SEQ ID NO: 12 - protein, 11 aa, Porcine reproductive and respiratory syndrome virus
  misc_feature (2)..(2): Xaa can be any naturally occurring amino acid
  misc_feature (5)..(8): Xaa can be any naturally occurring amino acid
FXVLXXXXQCR

SEQ ID NO: 13 - protein, 24 aa, Porcine reproductive and respiratory syndrome virus
  misc_feature (2)..(2): Xaa can be any naturally occurring amino acid
  misc_feature (5)..(6): Xaa can be any naturally occurring amino acid
  misc_feature (8)..(19): Xaa can be any naturally occurring amino acid
  misc_feature (23)..(23): Xaa can be any naturally occurring amino acid
FXVLXXIXXXXXXXXXXXXQCRXA

SEQ ID NO: 14 - protein, 23 aa, Porcine reproductive and respiratory syndrome virus
  misc_feature (2)..(2): Xaa can be any naturally occurring amino acid
  misc_feature (5)..(6): Xaa can be any naturally occurring amino acid
  misc_feature (8)..(18): Xaa can be any naturally occurring amino acid
  misc_feature (22)..(22): Xaa can be any naturally occurring amino acid
FXVLXXIXXXXXXXXXXXQCRXA

SEQ ID NO: 15 - protein, 22 aa, Porcine reproductive and respiratory syndrome virus
  misc_feature (2)..(2): Xaa can be any naturally occurring amino acid
  misc_feature (5)..(6): Xaa can be any naturally occurring amino acid
  misc_feature (8)..(17): Xaa can be any naturally occurring amino acid
  misc_feature (21)..(21): Xaa can be any naturally occurring amino acid
FXVLXXIXXXXXXXXXXQCRXA

SEQ ID NO: 16 - protein, 21 aa, Porcine reproductive and respiratory syndrome virus
  misc_feature (2)..(2): Xaa can be any naturally occurring amino acid
  misc_feature (5)..(6): Xaa can be any naturally occurring amino acid
  misc_feature (8)..(16): Xaa can be any naturally occurring amino acid
  misc_feature (20)..(20): Xaa can be any naturally occurring amino acid
FXVLXXIXXXXXXXXXQCRXA

SEQ ID NO: 17 - protein, 20 aa, Porcine reproductive and respiratory syndrome virus
  misc_feature (2)..(2): Xaa can be any naturally occurring amino acid
  misc_feature (5)..(6): Xaa can be any naturally occurring amino acid
  misc_feature (8)..(15): Xaa can be any naturally occurring amino acid
  misc_feature (19)..(19): Xaa can be any naturally occurring amino acid
FXVLXXIXXXXXXXXQCRXA

SEQ ID NO: 18 - protein, 19 aa, Porcine reproductive and respiratory syndrome virus
  misc_feature (2)..(2): Xaa can be any naturally occurring amino acid
  misc_feature (5)..(6): Xaa can be any naturally occurring amino acid
  misc_feature (8)..(14): Xaa can be any naturally occurring amino acid
  misc_feature (18)..(18): Xaa can be any naturally occurring amino acid
FXVLXXIXXXXXXXQCRXA

SEQ ID NO: 19 - protein, 18 aa, Porcine reproductive and respiratory syndrome virus
  misc_feature (2)..(2): Xaa can be any naturally occurring amino acid
  misc_feature (5)..(6): Xaa can be any naturally occurring amino acid
  misc_feature (8)..(13): Xaa can be any naturally occurring amino acid
  misc_feature (17)..(17): Xaa can be any naturally occurring amino acid
FXVLXXIXXXXXXQCRXA

SEQ ID NO: 20 - protein, 17 aa, Porcine reproductive and respiratory syndrome virus
  misc_feature (2)..(2): Xaa can be any naturally occurring amino acid
  misc_feature (5)..(6): Xaa can be any naturally occurring amino acid
  misc_feature (8)..(12): Xaa can be any naturally occurring amino acid
  misc_feature (16)..(16): Xaa can be any naturally occurring amino acid
FXVLXXIXXXXXQCRXA

SEQ ID NO: 21 - protein, 16 aa, Porcine reproductive and respiratory syndrome virus
  misc_feature (2)..(2): Xaa can be any naturally occurring amino acid
  misc_feature (5)..(6): Xaa can be any naturally occurring amino acid
  misc_feature (8)..(11): Xaa can be any naturally occurring amino acid
  misc_feature (15)..(15): Xaa can be any naturally occurring amino acid
FXVLXXIXXXXQCRXA

SEQ ID NO: 22 - protein, 15 aa, Porcine reproductive and respiratory syndrome virus
  misc_feature (2)..(2): Xaa can be any naturally occurring amino acid
  misc_feature (5)..(6): Xaa can be any naturally occurring amino acid
  misc_feature (8)..(10): Xaa can be any naturally occurring amino acid
  misc_feature (14)..(14): Xaa can be any naturally occurring amino acid
FXVLXXIXXXQCRXA

SEQ ID NO: 23 - protein, 14 aa, Porcine reproductive and respiratory syndrome virus
  misc_feature (2)..(2): Xaa can be any naturally occurring amino acid
  misc_feature (5)..(6): Xaa can be any naturally occurring amino acid
  misc_feature (8)..(9): Xaa can be any naturally occurring amino acid
  misc_feature (13)..(13): Xaa can be any naturally occurring amino acid
FXVLXXIXXQCRXA

SEQ ID NO: 24 - protein, 13 aa, Porcine reproductive and respiratory syndrome virus
  misc_feature (2)..(2): Xaa can be any naturally occurring amino acid
  misc_feature (5)..(6): Xaa can be any naturally occurring amino acid
  misc_feature (8)..(8): Xaa can be any naturally occurring amino acid
  misc_feature (12)..(12): Xaa can be any naturally occurring amino acid
FXVLXXIXQCRXA

SEQ ID NO: 25 - protein, 4 aa, Porcine reproductive and respiratory syndrome virus
  misc_feature (2)..(2): Xaa can be any naturally occurring amino acid
FXVL

SEQ ID NO: 26 - protein, 7 aa, Porcine reproductive and respiratory syndrome virus
  misc_feature (4)..(5): Xaa can be any naturally occurring amino acid
YITXXAN

SEQ ID NO: 27 - protein, 6 aa, Porcine reproductive and respiratory syndrome virus
  misc_feature (2)..(2): Xaa can be any naturally occurring amino acid
  misc_feature (5)..(5): Xaa can be any naturally occurring amino acid
FXVLXD

SEQ ID NO: 28 - protein, 8 aa, Porcine reproductive and respiratory syndrome virus
  misc_feature (5)..(5): Xaa can be any naturally occurring amino acid
VYITXTAN

SEQ ID NO: 29 - protein, 5 aa, Porcine reproductive and respiratory syndrome virus
  misc_feature (2)..(2): Xaa can be any naturally occurring amino acid
FXVLQ

SEQ ID NO: 30 - protein, 8 aa, Porcine reproductive and respiratory syndrome virus
  misc_feature (6)..(6): Xaa can be any naturally occurring amino acid
QYITIXAN

SEQ ID NO: 31 - protein, 22 aa, Porcine reproductive and respiratory syndrome virus
FMVLQKIECLQAPGTRSQCREA

SEQ ID NO: 32 - protein, 23 aa, Porcine reproductive and respiratory syndrome virus
QKIECLQAPGTRSQCREAIGTPQ

SEQ ID NO: 33 - protein, 21 aa, Porcine reproductive and respiratory syndrome virus
DISCLRHGRKSRQCRTAIGTP

SEQ ID NO: 34 - protein, 9 aa, Porcine reproductive and respiratory syndrome virus
ECLQAPGTR

SEQ ID NO: 35 - protein, 10 aa, Porcine reproductive and respiratory syndrome virus
SCLRHGHKSR

SEQ ID NO: 36 - protein, 172 aa, Porcine reproductive and respiratory syndrome virus
MAAAILFFLVGAQHLMVSEAFACKPCFSTHLSDIKTNTTAAAGFMVLQKIECLQAPGTRSQCREAIGTPQYITIQANVTDESYLYNADLLMLSACLFYASEMSEKGFNVIFGNVSGVVSACVNFTDYVAHVTQHTQQHHLVIDHVRLLHFLSPPVMRWATTIACLFAILLAI

SEQ ID NO: 37 - DNA, 519 bp, Porcine reproductive and respiratory syndrome virus
atggctgcggccattcttttcttcctggttggtgctcaacatctcatggtttctgaggcgttcgcctgcaagccctgcttctcgacgcatttatcagatattaagaccaacacgaccgcggctgccggtttcatggtccttcagaaaattgaatgcctccaagcccctgggacacggtcgcaatgtcgtgaagccatcggtaccccccagtacatcacgatacaggccaacgtgaccgacgaatcatacttgtataacgcggacttgctgatgctctctgcgtgcctcttctacgcctcagaaatgagcgagaaaggcttcaacgtcatctttgggaatgtttctggcgttgtttccgcttgtgtcaatttcacagattacgtagcccacgtgactcaacacacccagcagcatcacctggtaatcgaccacgttaggctactacatttcctgtcaccacctgtaatgaggtgggccacaaccatcgcttgtttgttcgccattcttttggcgatatga

SEQ ID NO: 38 - DNA, 14854 bp, Porcine reproductive and respiratory syndrome virus
acctcttggcccctgttctagcccaacaggtatccttctctctcggggcgagtgcgccgcctgctgctctcttgcagcgggaaggacctcccgagtatttccggagagcacctgctttacgggatctccaccctttaaccatgtctgggactctctcccggtgcatgtgcaccccggctgctcgggtattttggaacgccggtcaagtcttctgcacacggtgtctcagtgcgcggtctcttctccctcctgagcttcaggacactgaccttgctgcaattggtttgttttacaagcctaaggacaagatcaaatggaaagttcccattggcattcctcaggtggaatgtactccatccgggtgctgttggctctccgctattttccccttagcgcgcatgacctccggtaatcacaacttccttcaacggcttgtgaaggttgctgacgttttgtaccgtgacggttacttggcaccccaacaccttcgtgaactccaagtctacgaacgcggctgcagctggtacccgatcacggggcctgtgcccggaatgggtttgtatgcaaactccatgcacgtgtctgatcagccgtttcctggtgccactcatgtgttaaccaactcacccttgcctcaacaggcttgtcggcaaccattctgtccatttgaggaggctcattccgacgtgtacaggtggaagaaatttgtgattttcgtggattctcctcttaacggtcgatctcgtatgatgtggacaccggggtccgatgactcggctgccttagaagtgcttccgcctgaactagaacgtcgagtcgaaatcctcattcgaagttttcctgctcatcactctgttgatctcaccgaatgggaactcactgaatcacctgagcacggtttttccttcagcacgttccattctagtggtcacctcgcccaaaaccccgacatgtttgatggcaagtgttggctatcttgctttttgagcctgccgcccgaagtgtggcgccatgaagaacagctggccaacactctcggttaccaaaccaagtggggtgtgcacggtaagtacctccagcgcaggcttcaaattaacggcgtccgtgctgtggttgaccctaatggtcccattcacgttgaagcgctatcttgctcccagtcttggatcagacatctgactctggaagatgatgtaactccggggttcgttcgcctaatgtctctccgtattgtgccgaacacagaacccaccatcctccaggttttccggtttggggcacacaagtggtatggtgctgccggcaagcgagctcgcactaagcgtgcagcaaagaaagggaaggactcgactatcactcccgagactgcccaaccaacctccgcttgcgaaatcatcacctattccccaccggcggacggatcttgtggctggcatgttcttgccgccatagtgaaccgaatgataagtggtgacttcacgtcccccctaactcagtacaataggccagaggatgattgggcttctgattatgatcttgctcaagcgattcaatgcctgcaactgcctgctaccctggttcggggtcgcgcctgtcctaacgccaagtaccttataaaacttaacggggttcactgggaggtagaggtgaggcctggaatggctcctcgctccctttcccgcgaatgcgtggttggcgtctgctctgaaggctgtgtcgcgccgccttatccagaaaacgggctaccaaaacgcgcactcgaggccttggcgtctgcttacaggctaccttccgactgcgttagctgtggtattgctgactttctcgctaaccctccccttccggaattctggaccctcgacaaaatgttgacctccccgtcaccagaacggtccggcttctctagtttgtataaattacttttggaggttgttccgcagaaatgtggtgcctcggagggggcttttatttgtgctgttgaaaggatgttgaaggattgtccgagctccaaacaggccatggcccttttggcaaaaattagaatcccatcctcaagggccccgtctgtttccttggatgagtgttttcctacggatgtcccagccgactttgaatcagcgtctcaggaaaggccccaaacttccggtgtcgctgttgcccagtgtctaccggatgcaaaagagctcgaggaaacagccccgggaaaagttcaagagaatggtcacaaggccatccatcctgcgcctcttgctggttgtcctaacgacgagcaagtacaggtgattgccagcgagcaactgaggcccggcgactgtgtttcgacagtcaggggtgctcgcgatgatgctccagtctcagccggcctgactaacctggcaggcgggaaccccccttttccaaaccccacggaaggaaataggccccatgactgggaagacggacctttggatctatcccgaccgaaaccagttgccgagatgacccttgtaagagagcaagtaccctacaacccaggtcctaacactgatgtctcccccgtcgccgctccgggctttatcccgacggggctcgtatttcgtcatgttgagcattgtggctcggagtccggtgagagcgactcccctctaaacttgtctaatgtgcaaatttcggaccagcccctaaacctttccctgaccgcatggccggtgaaggccaccgcctctgaccccggttgggttcatggtcgacgtgagcctgtctttgcgaagcctcgaaatgccttctctgacggtgactcagttgttcagttcggggagctttctgaatccagctccgtcgtcgagtttgaccgagcaaaaaatgttacaacggttgacgcccctgtcgacttgacgactccgaataaggccctctctgtggtcgatcctttcgagttcgctgagcccaagcgcccacgtttctccgcgcaagccctgattgaccgaggaggtccacttgctgatgtccacgcaaaaataaagaatcgggtatacgaacagtgcctccaggcttgcgagcccggtagtcgcgcaaccccagccactagagactggctcgacaaaatgtgggagagggtggacatgaaaacttggcgctgcacctcacagtttcaagctggtcgcattctcgcgtccctcaagttcctccctgacatgattcaggacacaccgcctcctgctcccaggaagagccgggctggtgacagcaccggcctaaaacaactggtggcacagtgggataggaaattgagtgcggcccctcctccgaaactggttgggtcagtgcctgaccagactgtcctcccgtccgcggacacccagcaagaagacgctgaccctcctgatgggccgccccacgcgccggacattcctagtcgagtaggtacagtcaggaattggaaaggttgcatgctttccggcacccgttttgcggggtccatgagtcagcgcttcatgacatgggtttttgaggttctctcccatctcccagcttttgcgctcacacttttctcgccgcggggctctatggctccaggtgattggctgtttgcaggtgttgttttacttgctctcctgctctgtcgctcttacccaattttcgggtgccttcccttattgggtgtcttttctggttctgtgcggcgcgttcgtctgggtgtttttggttcttggatggcttttgctgtatttctattctcgactccatccaacccagtcggttcttcttgtgaccacgattcgccggagtgtcacgctgagcttttggctcttgagcagcgccaactttgggaacctgtgcgcggccttgtggtgggcccctcaggtctcttatgcgtcgttcttggcaagctactcggtgggtcacgttatctctggcatattctcttacgtttatgcatgcttgcagatttggccctttctcttgtttatgtggtgtcccaagggcgttgtcacaagtgttggggaaagtgtataaggacagctcctgcggaggtggctctcaatgtatttcctttctcgcgcgccacccgttcctctattgtatccttatgtgatcgattccaggcgccaaaaggggttgatcccgtacatttggcaacgggttggcgcgggtgctggtgcggcgatagccccatccatcaaccacaccagaaacccatagcttacgccaacttggatgaaaagaaaatatctgcccagacggtggtcgctgttccatacgatcccagccaggccatcaaatgcctgaaagtcctacaggctggaggagctattgtagaccagccaacacctgaggttgttcgtgtttccgaaatccccttctcagccccattttttccgaaagttccggtcaatccaaactgtagggttgtggtagattcggacacctttgtggccgcggttcgctgcggttactcaacaacacaactggtcctgggccggggcaacttcgccaagttgaatcaaacacctcttgggaactctgtctccaccaaaacgactggtggtgcctcttacacccttgctgtggcgcaagtgtccgtgtggactctcatccatttcatcctcggtctttggttcacatcgcctcaagtgtgcggccgaggtaccgctgatccatggtgttcaaatcctttttcatatcccacctatggccctggagttgtctgctcctctcgactttgcgtgtctgccgatggagtcaccctgccattgttctcagccgtggcacaactctccggtagggaggtgggaattttcattctggtgctcgtctccttgatcgctttggcccaccatatggctcttaaagcagatatgttggtgatctttttggctttctgcgcctacgcctggcctatgagttcttggttaatttgtttctttcccatgcttttgaagtgggttacccttcaccctcttaccatgctttgggtacactctttcttagtgttttgtctgccagcagctggcatcctttcactagggacaactggccttctctgggcagtcggccgcttcacccaggtagccggaattattacaccttatgacattcaccgatacacttctgggccgcgtggtgctgccgctgtagccacagccccagaaggcacttacatggccgccgtccgtagagctgccttaactgggcgaactttgatcttcaccccgtctgcagttgggtcccttctcgagggtgccttcaggactcataaaccctgcctcaacaccgtgaatgtcgtgggttcttcttttggttctggaggagtctttaccattgatgggaaaaaactgttgttactgcgacacatgtgttgaacggcgacacagccagggtcaccggtgactcctataaccgcatgctcaccttcaggaccaacggtgattacgcctggtcccatgctgatgactggcaaggcgttgccccagtggtcaagatcgcgaaagggtatcgcggtcgtgcctattggcaaacatcaactggtgtcgaacccggtgttgttggtgaaggattcgccttctgttttactaactgtggtgactcggggtcacccgtcatttcagaatctggtgatctcattggaatccacaccggttcgaacaaacttggttctggtcttgtgacaacccccgaaggggagacctgcactattaaagaaaccaagctctctgacctttccagacacttcgcgggcccaagcgttccccttggggacataaaattaagcccggccatcatccctgatgtgacgtccatcccaagtgacttggcatcgctcctggcttccgtccctgtagtggaaggcggtctttcgaccgttcaactcttgtgtgtctttttccttctctggcgtatgatggggcatgcttggacacccattgttgccgtgggtttctttttgctgaatgaaattcttccagcagtcttggtccgagccgtgttctcttttgcgctctttgcgtttgcatggctcaccccctggtctgcgcaggtgttgatgatcagactcctcacggcctccctcaaccgcaacaagctttctctggcgttctacgcactcgggggtgtcgtcggtttggccgctgagatcgggactttcgctggtaggttgtctgaattgtctcaagccatttcaacatactgctttttacctagggtccttgctatgaccagctgtgtccccatcatcatcattggtggactccatgctcttggtgtaatcctgtggttgttcaaatatcggtgtctccacaacacgctagttggtgatgggagtttttcaagcgccttcttcctgcggtactttgcagagggtaatctcagaaaaggtgtttcacagtcctgtggcatgagtaatgaatccttgacggctgctttggcttgtaagttgtcacaggctgaccttgactttctgtccggcctaacgaatttcaagtgttttgtgtctgcttcaaatatgaagaatgctgctggccaatatattgaagcagcgtacgccaaggccttgcgccacgagttggcttccttagttcaggtcgacaaaatgaagggggttttgtccaagctagaagcttttgctgagacggccaccccatcccttgatacaggtgacgtagttgttctgcttggacaacatcctcatggatctattcttgacattaacgtagggactgaaaggaaaactgtgtctgtgcaggagactcggagtttgggtggctccaaattcagtgtctgcaccgttgtgtccaacacacctgtagacgccctgaccagcatcccacttcagacaccaactccgcttttcgagaatggcccgcgtcatcgcggtgaggaagacgatcttaaagtcgagaggatgaagaagcactgcatatccctcggctttcataacattaatggcaaagtttactgcaaaatttgggacaagtctaccggtgacaccttctacacggatgactcccgatacacccaagactgtgcctttcaggacaggtcagccgactatagagacagggattatgaaggtgtgcagaccgccccccagcacggatttgacccaaagtccgagacccctgtcggcactgttgtgatcggcggcattacgtataacaggtatctggttaaaggtaaagaggtcttgatccccaagcctgacaactgccttgaagccgccaagctatcccttgaacaagctctcgctggtatgggccagacttgtgacctcacggctgctgaagtggaaaagctaaagcgcattattagccaactccaaggcttgaccaccgagcaggctttaaactgctagccgccagtggcttgacccgctgtggccgcggcggcttagttgtgactgaaacggcggtgaaaattgtgaaataccacagcagaaccttcaccctaggccctttagacctgaaagtcacctctgaagtggaggtgaagaaatcaacagagcagggccacgccgttgtagcaaacctatgctccggtgttgtgttgatgagacctcaccctccgtcccttgttgatgttcttctaaagcctggacttgacacgacacctggcatccaaccggggcatggggctggaaacatgggtgtgaacggttccatttgggattttgaaactgcccccacaaaggcggaactcgagttatccaaacaaataatccaagcgtgtgagattaggcgcggggatgccccgaacctccaactcccttataagctctatcctgttaggggggatcctgagcggcatgaaggtcgccttatcaataccaggttcggggacttaccttataagactcctcaagacaccaagtccgcagtccacgcggcttgttgcctacaccccaatggagccccggtatttgacggtaaatccatgctgggcaccactcttcagcatggttttgagctttatgtccccactgtgccctatagtgttatggagtaccttgactcacgccctgacactccttttatgtgtactaagcatggcacttccagtgctgctgcagaggacctccaaaagtatgacctatccacccaaggatttgtcttgcctggtgtcttgcgcttagtgcgcaggttcatcttcagccatattggtaaagcgccaccattgttcctcccatcaacttaccccgctaagaactccatggcagggattaatggtcagaggtttccgacaaaggatattcagagcatacctgaaatcgatgaaatgtgtgcccgcgctgtcaaggaaaattggcaaactgttacaccttgcaccctcaagaaacagtattgttctaagcccaaaaccaggaccatcctgggcactaacaactttattgccttggcccacagatcagcgcttagtggtgtcacccaggcgttcatgaaaaaggcttggaattccccaattgccttggggaagaataaattcaaggagctgcattgcaccgttgccggcaggtgtcttgaggctgacttggcctcctgcgaccgcagtacccccgccattgtgagatggtttgttgccaacctcctgtatgaacttgcaggatgtgaagagtacctgcccagctacgtgcttaattgctgccatgacctcgtggcaacacaaaatggtgccttcacaaaacgcggtggcctgtcgtctggggaccctgtcaccagtgtgtccaacaccgtatattcactgataatttacgcccagcacatggtgttgtcagccctaaaaatgggtcatgagattggtcttaagtttcttgaggagcaactcaagttcgaagacctccttgaaattcagcctatgttggtgtattctgatgatcttgttttgtatgctgaaaggccctccttccccaattaccattggtgggtcgagcaccttgacttgatgctgggtttcaagacagacccaaagaagaccgttataactgacaagcccagctttctcggttgcagaattgaggcggggcgacagctagcccccaatcgtgaccgcattctggctgctctcgcatatcacatgaaagcgcaggacgcatcagagtactatgcgtctgctgccgcaattctgatggactcgtgtgcttgcattgactatgatcctgagtggtatgaagacctcatctgtggcatcgctcagtgcgcccgccaggatggttatcgcttcccaggaccggcatttttcatgtccatgtgggagagactgagaagccataatgaggggaagaaattccgccattgcggcatctgtgacgccaaagctgatcacgcgtctgcctgtgggcttgacttgtgcttgtttcactcgcactttcatcaacactgccctgttatcttgagttgcggccaccatgccggttccaaagaatgttcgcagtgtcagtcacctgttgggtctggcaagacccctcttgatgccgtgctgaagcaaatcccatacaaacctcctcgtacagcaatcatgagggtaagcgacaaagtgacagccctggatccagggaggtaccagtctcgtcggggcctcgttgcagtcaaaaggggtatcgcaggtaatgaagttgatctccctgatggggactatcaggtagtgcctcttttgccgacctgcaaagacattaatatggtgaaggtggcttgtaatgttctactcagcaaattcatagtggggccaccaggttccgggaagacaacctggctgctgagtcaagtccaggatgatgatgttatttacacacccactcatcagaccatgtttgatatagtcagtgctctcaaagtttgcaggtattccatcccaggggcctcaggactccctttcccaccacctgccaggtccgggccatgggtcaagctcattgccagcggacacgtcccaggccgagtgtcatacctcgatgaggctggatattgtaatcatctggacatcctcagactgctttccaaaacacctcttgtgtgtttgggtgaccttcagcaacttcaccctgttggctttgattcctactgttatgtgttcgatcagatgcctcagaagcagctgaccactatttatagatttggtcctaacatctgtgcagccatccagccttgttacagggaaaaacttgaatctaaggctaggaacaccagggtgggtttcaccacccggcctgtggccttcggtcaggtgttgacaccataccacaaagaccgtactggctctgcgataaccatagattcatcccaaggggccacttttgatattgtgacattgcatctaccatcgccgaagtccttaaacaaatcccgagcacttgtagccattactcgagcaagacatgggttgttcatttatgaccctcataaccagctccaggaattttttaatttaacccctgagagcactgattgcaaccttgtgttttgccacggggatgagctggtagttttggacgccggtaatgcagtcacaactgtggcgaaggccctagaaactggtccgtcgcggttccgtgtgtcggacccgagatgcaagtccctcttagctgcctgttcagccagtctggaagggagctgcatgccactaccgcaagtggcacataacctgggattttacttttcccctgacagcccagcatttgcacctctgccaaaagagctggcgccacactggccagtggtcactcatcagaataatcgggcgtggcctgatcgacttgtcgccagcatgcgcccgctcgacaaccgttacagcaagccaatggtcggtgcagggtatgtggtcgggccgtccacctttctcggtacacccggcgtggtgtcatactatcttacactatacattaagggtgagccccaggccttacctgaaacactcgtttccacgggacgcatagctacagattgtcgggagtacctcgacacagctgaggaagaggcagcaaaagaactcccccacgcattcatgggtgatgtcaaaggcaccacaattggtggttgtcatcacattacatcaaaatacctacccaggtccctacccaaggactccattgccgtagttggggtaagttcacctggcaaggccgccaaagccttatgcactctcactgatgtgtacctcccagaactccggccgtatttgcaacctgagacagcgtcgaaatgctggaaactcaaactggacttcagggacgtccggctaatggtctggaaaggggccaccgcctacttccagttggaagggctcacttggtctgcactgcctgactatgccaggtttattcagctgcccaagaacgccattgtgtacatcgatccgtgcataggaccggcgacagccaaccgtaaagttgtgcgaaccacagattggcgagctgacctggcagtgacaccgtacgactacggtgctcaacacattttgacaaccgcctggttcgaggacctcgggccgcagtggaaaattttggggttgcagcccttcaggcgaacatttggccttgaaaatactgaagattgggcaattcttgcacgccgtatgaatgacggtaaggactacactgattacaactggagttgcgttcgagaacgcccacacgctatctatgggcgtgctcgtgaccatacataccactttgcccttggcacagaattacaagtggagctaggtaaacccagattgtcgcctgagcaagtcccgtgaattcggagggatgcaatggggtcactgtggagcaaaatcagccagttgttcgtggacgctttcactgaattccttgttagtgtggttgacattgtcattttccttgccatattgtttgggttcacagtcgcaggatggttactggtctttcttctcagggtggtttgctccgcgtttctccgttcgcgctctgccattcactctcccgaactatcgaaagtcctatgagggcttgttacccaactgtagaccggatgttccacaatttgcgtttaagcacccattgggcatgttttggcacatgaaggtctcccacttgattgatgagatggtctctcgtcgcgtctaccaaaccatggagcattcgggccaagcggcctggaaacaggtggtcgctgaggccactctcacgaagttgtccaggctcgacattgtcactcacttccaacacctagccgcagtggaggcggattcttgccactttcttagctcgcgactcgtgatgctaaaaaatcttgctgtaggcaatgtaagtctacaatacaacaccacgttggatcgcgttgagctcattttccccacgccaggcacgaggcccaagttgaccgattttaggcaatggctcatcagtgtgcacgcttccattttctcctctgtggcttcatctgttaccttgtttgtagtgctttggcttcgaattccagctctacgctatgtttttggtttccattggcccacggcaacacatcatttgaactaactgtgaattacaccatatgtaagccctgccttaccagtcaagcggccaaacaacggctcgaacccggtcatagcatgtggtgcaggatagggcacaccagctgcgaggagagtgaccatgatgagttgtcaatgaccatcccgcctgggtatgataaccttaagctcgagggctactacgcttggctagccttcttgtccttttcctacgcggcacagttccatccggagctattcggaatagggaatgtatcgcgtgtttttgtggacaagcaacgtcaggccatctgtgcggagcacgacggatccaattcaaccgtgtccactaagtacaacatctccgcatcgtatgcggcgtactatcatcaccagatagacgggggtaattggtttcacctagaatggctgcggccattcttttcttcctggttggtgctcaacatctcatggtttctgaggcgttcgcctgcaagccctgcttctcgacgcatttatcagatattaagaccaacacgaccgcggctgccggtttcatggtccttcagaaaattgaatgcctccaagcccctgggacacggtcgcaatgtcgtgaagccatcggtaccccccagtacatcacgatacaggccaacgtgaccgacgaatcatacttgtataacgcggacttgctgatgctctctgcgtgcctcttctacgcctcagaaatgagcgagaaaggcttcaacgtcatctttgggaatgtttctggcgttgtttccgcttgtgtcaatttcacagattacgtagcccacgtgactcaacacacccagcagcatcacctggtaatcgaccacgttaggctactacatttcctgtcaccacctgtaatgaggtgggccacaaccatcgcttgtttgttcgccattcttttggcgatatgagatgttctcacaaattggggcgcttcttgattccgcactcttgcttttggtggcttttttgctgtgtaccggcttgtcctggtcctttgccgatggcaacggcaacagctcgacataccaatacatatataacttgacgatatgcgagcttaatgggaccacctggctgtctagccattttgattgggcagtcgagacttttgtgctctacccggtcgcgactcacattctctcactgggttttctcacaacaagccatttctttgacgcgctcggtctcagtgctgtgtccgtcacaggattttatgaccagcggtacgtgctcagcagtgtctacggcgtctgtgccctcgcagcgctcgtgtgttttgccatccgtgctgctaaaaattgtatggcttgtcgctacgcccgcacccggttcaccaacttcatcgtggacgaccgggggaggattcatcggtggaaatccccaatagtggtggagaaattgggcaaagctgaggtcggcagcgaccttgtcaccattaaacatgtcgtcctcgaaggggttaaagctcaacccttgacgaggacttcggctgagcaatgggaggcctagatggtttttgttatgaccctactgctgtacaaaagcttgtgttggccttcagcatcacgtatacacctataatgatatatgcccttaaggtgtcacgcggtcgactcctagggctgttgcacatcctgatatttctgaactgttccttcactttcggatacatgacgtatgtgcattttcagtccgccaaccgtgttgtactcactttgggggccgttgttgccctcctgtggggtatttacagcttcacagagtcatggaagttcatcacttccagatgcagattgtgttgccttggccggcgatacattctggcccctgcccaccacgtagaaagtgctgcaggtctccatcctatcccagcgtctggcaaccgagcatacgctgtgaggaagcccggactaacatcagtgaacggcactctggtaccaggacttcggagcctcgtgttgggcggcaaacgagctgttaaacgaggagtggttaacctcgtcaaatatggccggtaaaaaccaaggccagaagaaaaagaaaagtacagctccaatggggaatggccagccagtcaatcaactgtgccagttgctgggtgcaatgataaggacccagcgccagcaacctaggggaggacaggccaaaaagaaaaggcctgagaagccgcattttcccctagctgctgaagatgacatacggcaccacctcacccagactgaacgatccctctgtttgcaatcgatccagacggcttttaatcaaggcgcaggagctgcgtcgctttcgtccagcgggaaagtcagttttcaggttgagttcatgctgccggttgctcatacagtgcgcctgattcgcgtgacttccacatccgccaatc

SEQ ID NO: 39 - protein, 17 aa, Porcine reproductive and respiratory syndrome virus
SSHLQLIYNLTICELNG

SEQ ID NO: 40 - protein, 17 aa, Porcine reproductive and respiratory syndrome virus
QSHRASTAQGTTPLRRS

SEQ ID NO: 41 - DNA, 15111 bp, Porcine reproductive and respiratory syndrome virus
atgatgtgtagggtattccccctacatacacgacacttctagtgtttgtgtaccttggaggcgtgggtacagccccgccccaccccttggcccctgttctagcccaacaggtatccttctctctcggggcgagtgcgccgcctgctgctcccttgcagcgggaaggacctcccgagtatttccggagagcacctgctttacgggatctccaccctttaaccatgtctgggacgttctcccggtgcatgtgcaccccggctgcccgggtattttggaacgccggccaagtcttttgcacacggtgtctcagtgcgcggtctcttctctctccagagcttcaggacactgacctcggtgcagttggcttgttttacaagcctagggacaagcttcactggaaagtccctatcggcatccctcaggtggaatgtactccatccgggtgctgttggctctcagctgttttccctttggcgcgtatgacctccggcaatcacaacttcctccaacgacttgtgaaggttgctgatgttttgtaccgtgacggttgcttggcacctcgacaccttcgtgaactccaagtttacgagcgcggctgcaactggtacccgatcacggggcccgtgcccgggatgggtttgtttgcgaactccatgcacgtatccgaccagccgttccctggtgccacccatgtgttgactaactcgcctttgcctcaacaggcttgtcggcagccgttctgtccatttgaggaggctcattctagcgtgtacaggtggaagaaatttgtggttttcacggactcctccctcaacggtcgatctcgcatgatgtggacgccggaatccgatgattcagccgccctggaggtactaccgcctgagttagaacgtcaggtcgaaatcctcattcggagttttcctgctcatcaccctgtcgacctggccgactgggagctcactgagtcccctgagaacggtttttccttcaacacgtctcattcttgcggtcaccttgtccagaaccccgacgtgtttgatggcaagtgctggctctcctgctttttgggccagtcggtcgaagtgcgctgccatgaggaacatctagctgacgccttcggttaccaaaccaagtggggcgtgcatggtaagtacctccagcgcaggcttcaagttcgcggcattcgtgctgtagtcgatcctgatggtcccattcacgttgaagcgctgtcttgcccccagtcttggatcaggcacctgactctggatgatgatgtcaccccaggattcgttcgcctgacatcccttcgcattgtgccgaacacagagcctaccacttcccggatctttcggtttggagcgcataagtggtatggcgctgccggcaaacgggctcgtgctaagcgtgccgctaaaagtgagaaggattcggctcccacccccaaggttgccctgccggtccccacctgtggaattaccacctactctccaccgacagacgggtcttgtggttggcatgtccttgccgccataatgaaccggatgataaatggtgacttcacgtcccctctgactcagtacaacagaccagaggatgattgggcttctgattatgatcttgttcaggcgattcaatgtctacgactgcctgctaccgtggttcggaatcgcgcctgtcctaacgccaagtaccttataaaacttaacggagttcactgggaggtagaggtgaggtctggaatggctcctcgctccctttctcgtgaatgtgtggttggcgtttgctctgaaggctgtgtcgcaccgccttatccagcagacgggctacctaaacgtgcactcgaggccttggcgtctgcttacagactaccctccgattgtgttagctctggtattgctgactttcttgctaatccacctcctcaggaattctggaccctcgacaaaatgttgacctccccgtcaccagagcggtccggcttctctagtttgtataaattactattagaggttgttccgcaaaaatgcggtgccacggaaggggctttcatctatgctgttgagaggatgttgaaggattgtccgagctccaaacaggccatggcccttctggcaaaaattaaagttccatcctcaaaggccccgtctgtgtccctggacgagtgtttccctacggatgttttagccgacttcgagccagcatctcaggaaaggccccaaagttccggcgctgctgttgtcctgtgttcaccggatgcaaaagagttcgaggaagcagccccggaagaagttcaagagagtggccacaaggccgtccactctgcactccttgccgagggtcctaacaatgagcaggtacaggtggttgccggtgagcaactgaagctcggcggttgtggtttggcagtcgggaatgctcatgaaggtgctctggtctcagctggtctaattaacctggtaggcgggaatttgtccccctcagaccccatgaaagaaaacatgctcaatagccgggaagacgaaccactggatttgtcccaaccagcaccagcttccacaacgacccttgtgagagagcaaacacccgacaacccaggttctgatgccggtgccctccccgtcaccgttcgagaatttgtcccgacggggcctatactctgtcatgttgagcactgcggcacggagtcgggcgacagcagttcgcctttggatctatctgatgcgcaaaccctggaccagcctttaaatctatccctggccgcttggccagtgagggccaccgcgtctgaccctggctgggtccacggtaggcgcgagcctgtctttgtaaagcctcgaaatgctttctctgatggcgattcagcccttcagttcggggagctttctgaatccagctctgtcatcgagtttgaccggacaaaagatgctccggtggttgacgcccctgtcgacttgacgacttcgaacgaggccctctctgtagtcgatcctttcgaatttgccgaactcaagcgcccgcgtttctccgcacaagccttaattgaccgaggcggtccacttgccgatgtccatgcaaaaataaagaaccgggtatatgaacagtgcctccaagcttgtgagcccggtagtcgtgcaaccccagccaccagggagtggctcgacaaaatgtgggatagggtggacatgaaaacttggcgctgcacctcgcagttccaagctggtcgcattcttgcgtccctcaaattcctccctgacatgattcaagacacaccgcctcctgttcccaggaagaaccgagctagtgacaatgccggcctgaagcaactggtggcacagtgggataggaaattgagtgtgaccccccccccaaaaccggttgggccagtgcttgaccagatcgtccctccgcctacggatatccagcaagaagatgtcaccccctccgatgggccaccccatgcgccggattttcctagtcgagtgagcacgggcgggagttggaaaggccttatgctttccggcacccgtctcgcggggtctatcagccagcgccttatgacatgggtttttgaagttttctcccacctcccagcttttatgctcacacttttctcgccgcggggctctatggctccaggtgattggttgtttgcaggtgtcgttttacttgctctcttgctctgtcgttcttacccgatactcggatgccttcccttattgggtgtcttttctggttctttgcggcgtgttcgtctgggtgtttttggttcttggatggcttttgctgtatttttattctcgactccatccaacccagtcggttcttcttgtgaccacgattcgccggagtgtcatgctgagcttttggctcttgagcagcgccaactttgggaacctgtgcgcggccttgtggtcggcccctcaggcctcttatgtgtcattcttggcaagttactcggtgggtcacgttatctctggcatgttctcctacgtttatgcatgcttgcagatttggccctttctcttgtttatgtggtgtcccaggggcgttgtcacaagtgttggggaaagtgtataaggacagctcctgcggaggtggctcttaatgtatttcctttctcgcgcgccacccgtgtctctcttgtatccttgtgtgatcgattccaaacgccaaaaggggttgatcctgtgcacttggcaacgggttggcgcgggtgctggcgtggtgagagccccatccatcaaccacaccaaaagcccatagcttatgccaatttggatgaaaagaaaatgtctgcccaaacggtggttgctgtcccatacgatcccagtcaggctatcaaatgcctgaaagttctgcaggcgggaggggccatcgtggaccagcctacacctgaggtcgttcgtgtgtccgagatccccttctcagccccatttttcccaaaagttccagtcaacccagattgcagggttgtggtagattcggacacttttgtggctgcggttcgctgcggttactcgacagcacaactggttctgggccggggcaactttgccaagttaaatcagaccccccccaggaactctatctccaccaaaacgactggtggggcctcttacacccttgctgtggctcaagtgtctgcgtggactcttgttcatttcatcctcggtctttggttcacatcacctcaagtgtgtggccgaggaaccgctgacccatggtgttcaaatcctttttcatatcctacctatggccccggagttgtgtgctcctctcgactttgtgtgtctgccgacggggtcaccctgccattgttctcagccgtggcacaactctccggtagagaggtggggatttttattttggtgctcgtctccttgactgctttggcccaccgcatggctcttaaggcagacatgttagtggtcttttcggctttttgtgcttacgcctggcccatgagctcctggttaatctgcttctttcctatactcttgaagtgggttacccttcaccctcttactatgctttgggtgcactcattcttggtgttttgtctgccagcagccggcatcctctcactagggataactggccttctttgggcaattggccgctttacccaggttgccggaattattacaccttatgacatccaccagtacacctctgggccacgtggtgcagctgctgtggccacagccccagaaggcacttatatggccgccgtccggagagctgctttaactgggcgaactttaatcttcaccccgtctgcagttggatcccttctcgaaggtgctttcaggactcataaaccctgccttaacaccgtgaatgttgtaggctcttcccttggttccggaggggttttcaccattgatggcagaagaactgtcgtcactgctgcccatgtgttgaacggcgacacagctagagtcaccggcgactcctacaaccgcatgcacactttcaagaccaatggtgattatgcctggtcccatgctgatgactggcagggcgttgcccctgtggtcaaggttgcgaaggggtaccgcggtcgtgcctactggcaaacatcaactggtgtcgaacccggtatcattggggaagggttcgccttctgttttactaactgcggcgattcggggtcacccgtcatctcagaatctggtgatcttattggaatccacaccggttcaaacaaacttggttctggtcttgtgacaacccctgaaggggagacctgcaccatcaaagaaaccaagctctctgacctttccagacattttgcaggcccaagcgttcctcttggggacattaaattgagtccggccatcatccctgatgtaacatccattccgagtgacttggcatcgctcctagcctccgtccctgtagtggaaggcggcctctcgaccgttcaacttttgtgtgtctttttccttctctggcgcatgatgggccatgcctggacacccattgttgccgtgggcttctttttgctgaatgaaattcttccagcagttttggtccgagccgtgttttcttttgcactctttgtgcttgcatgggccaccccctggtctgcacaggtgttgatgattagactcctcacggcatctctcaaccgcaacaagctttctctggcgttctacgcactcgggggtgtcgtcggtttggcagctgaaatcgggacttttgctggcagattgtctgaattgtctcaagctctttcgacatactgcttcttacctagggtccttgctatgaccagttgtgttcccaccatcatcattggtggactccataccctcggtgtgattctgtggttattcaaataccggtgcctccacaacatgctggttggtgatgggagtttttcaagcgccttcttcctacggtattttgcagagggtaatctcagaaaaggtgtttcacagtcctgtggcatgaataacgagtccctaacggctgctttagcttgcaagttgtcacaggctgaccttgattttttgtccagcttaacgaacttcaagtgctttgtatctgcttcaaacatgaaaaatgctgccggccagtacattgaagcagcgtatgccaaggccctgcgccaagagttggcctctctagttcagattgacaaaatgaaaggagttttgtccaagctcgaggcctttgctgaaacagccaccccgtcccttgacataggtgacgtgattgttctgcttgggcaacatcctcacggatccatcctcgatattaatgtggggactgaaaggaaaactgtgtccgtgcaagagacccggagcctaggcggctccaaattcagtgtttgtactgtcgtgtccaacacacccgtggacgccttgaccggcatcccactccagacaccaacccctctttttgagaatggtccgcgtcatcgcagcgaggaagacgatcttaaagtcgagaggatgaagaaacactgtgtatccctcggcttccacaacatcaatggcaaagtttactgcaaaatttgggacaagtctaccggtgacaccttttacacggatgattcccggtacacccaagaccatgcttttcaggacaggtcagccgactacagagacagggactatgagggtgtgcaaaccaccccccaacagggatttgatccaaagtctgaaacccctgttggcactgttgtgatcggcggtattacgtataacaggtatctgatcaaaggtaaggaggttctggtccccaagcctgacaactgccttgaagctgccaagctgtcccttgagcaagctctcgctgggatgggccaaacttgcgaccttacagctgccgaggtggaaaagctaaagcgcatcattagtcaactccaaggtttgaccactgaacaggctttaaactgttagccgccagcggcttgacccgctgtggccgcggcggcctagttgtgactgaaacggcggtaaaaattataaaataccacagcagaactttcaccttaggccctttagacctaaaagtcacttccgaggtggaggtaaagaaatcaactgagcagggccacgctgttgtggcaaacttatgttccggtgtcatcttgatgagacctcacccaccgtcccttgtcgacgttcttctgaaacccggacttgacacaatacccggcattcaaccagggcatggggccgggaatatgggcgtggacggttctatttgggattttgaaaccgcacccacaaaggcagaactcgagttatccaagcaaataatccaagcatgtgaagttaggcgcggggacgccccgaacctccaactcccttacaagctctatcctgttaggggggatcctgagcggcataaaggccgccttatcaataccaggtttggagatttaccttacaaaactcctcaagacaccaagtccgcaatccacgcggcttgttgcctgcaccccaacggggcccccgtgtctgatggtaaatccacactaggtaccactcttcaacatggtttcgagctttatgtccctactgtgccctatagtgtcatggagtaccttgattcacgccctgacaccccttttatgtgtactaaacatggcacttccaaggctgctgcagaggacctccaaaaatacgacctatccacccaaggatttgtcctgcctggggtcctacgcctagtacgcagattcatctttggccatattggtaaggcgccgccattgttcctcccatcaacctatcccgccaagaactctatggcagggatcaatggccagaggttcccaacaaaggacgttcagagcatacctgaaattgatgaaatgtgtgcccgcgctgtcaaggagaattggcaaactgtgacaccttgcaccctcaagaaacagtactgttccaagcccaaaaccaggaccatcctgggcaccaacaactttattgccttggctcacagatcggcgctcagtggtgtcacccaggcattcatgaagaaggcttggaagtccccaattgccttggggaaaaacaaattcaaggagctgcattgcactgtcgccggcaggtgtcttgaggccgacttggcctcctgtgaccgcagcacccccgccattgtaagatggtttgttgccaacctcctgtatgaacttgcaggatgtgaagagtacttgcctagctatgtgcttaattgctgccatgacctcgtggcaacacaggatggtgccttcacaaaacgcggtggcctgtcgtccggggaccccgtcaccagtgtgtccaacaccgtatattcactggtaatttatgcccagcacatggtattgtcggccttgaaaatgggtcatgaaattggtcttaagttcctcgaggaacagctcaagttcgaggacctccttgaaattcagcctatgttggtatactctgatgatcttgtcttgtacgctgaaagacccacatttcccaattaccactggtgggtcgagcaccttgacctgatgctgggtttcagaacggacccaaagaaaaccgtcataactgataaacccagcttcctcggctgcagaattgaggcagggcgacagctagtccccaatcgcgaccgcatcctggctgctcttgcatatcacatgaaggcgcagaacgcctcagagtattatgcgtctgctgccgcaatcctgatggattcatgtgcttgcattgaccatgaccctgagtggtatgaggacctcatctgcggtattgcccggtgcgcccgccaggatggttatagcttcccaggtccggcatttttcatgtccatgtgggagaagctgagaagtcataatgaagggaagaaattccgccactgcggcatctgcgacgccaaagccgactatgcgtccgcctgtgggcttgatttgtgtttgttccattcgcactttcatcaacactgccctgtcactctgagctgcggtcaccatgccggttcaaaggaatgttcgcagtgtcagtcacctgttggggctggcagatcccctcttgatgccgtgctaaaacaaattccatacaaacctcctcgtactgtcatcatgaaggtgggtaataaaacaacggccctcgatccggggaggtaccagtcccgtcgaggtctcgttgcagtcaagaggggtattgcaggcaatgaagttgatctttctgatggggactaccaagtggtgcctcttttgccgacttgcaaagacataaacatggtgaaggtggcttgcaatgtactactcagcaagttcatagtagggccaccaggttccggaaagaccacctggctactgagtcaagtccaggacgatgatgtcatttacacacccacccatcagactatgtttgatatagtcagtgctctcaaagtttgcaggtattccattccaggagcctcaggactccctttcccaccacctgccaggtccgggccgtgggttaggcttattgccagcgggcacgtccctggccgagtatcatacctcgatgaggctggatattgtaatcatctggacattcttagactgctttccaaaacaccccttgtgtgtttgggtgaccttcagcaacttcaccctgtcggctttgattcctactgttatgtgttcgatcagatgcctcagaagcagctgaccactatttacagatttggccctaacatctgcgcagccatccagccttgttacagggagaaacttgaatctaaggctaggaacactagggtggtttttaccacccggcctgtggcctttggtcaggtgctgacaccataccataaagatcgcatcggctctgcgataaccatagattcatcccagggggccacctttgatattgtgacattgcatctaccatcgccaaagtccctaaataaatcccgagcacttgtagccatcactcgggcaagacacgggttgttcatttatgaccctcataaccagctccaggagtttttcaacttaacccctgagcgcactgattgtaaccttgtgttcagccgtggggatgagctggtagttctgaatgcggataatgcagtcacaactgtagcgaaggcccttgagacaggtccatctcgatttcgagtatcagacccgaggtgcaagtctctcttagccgcttgttcggccagtctggaagggagctgtatgccactaccgcaagtggcacataacctggggttttacttttccccggacagtccaacatttgcacctctgccaaaagagttggcgccacattggccagtggttacccaccagaataatcgggcgtggcctgatcgacttgtcgctagtatgcgcccaattgatgcccgctacagcaagccaatggtcggtgcagggtatgtggtcgggccgtccacctttcttggtactcctggtgtggtgtcatactatctcacactatacatcaggggtgagccccaggccttgccagaaacactcgtttcaacagggcgtatagccacagattgtcgggagtatctcgacgcggctgaggaagaggcagcaaaagaactcccccacgcattcattggcgatgtcaaaggtaccacggttggggggtgtcatcacattacatcaaaatacctacctaggtccctgcctaaggactctgttgccgtagttggagtaagttcgcccggcagggctgctaaagccgtgtgcactctcaccgatgtgtacctccccgaactccggccatatctgcaacctgagacggcatcaaaatgctggaaactcaaattagacttcagggacgtccgactaatggtctggaaaggagccaccgcctatttccagttggaagggcttacatggtcggcgctgcccgactatgccaggtttattcagctgcccaaggatgccgttgtatacattgatccgtgtataggaccggcaacagccaaccgtaaggtcgtgcgaaccacagactggcgggccgacctggcagtgacaccgtatgattacggtgcccagaacattttgacaacagcctggttcgaggacctcgggccgcagtggaagattttggggttgcagccctttaggcgagcatttggctttgaaaacactgaggattgggcaatccttgcacgccgtatgaatgacggcaaggactacactgactataactggaactgtgttcgagaacgcccacacgccatctacgggcgtgctcgtgaccatacgtatcattttgcccctggcacagaattgcaggtagagctaggtaaaccccggctgccgcctgggcaagtgccgtgaattcggggtgatgcaatggggtcactgtggagtaaaatcagccagctgttcgtggacgccttcactgagttccttgttagtgtggttgatattgccattttccttgccatactgtttgggttcaccgtcgcaggatggttactggtctttcttctcagagtggtttgctccgcgcttctccgttcgcgctctgccattcactctcccgaactatcgaaggtcctatgaaggcttgttgcccaactgcagaccggatgtcccacaatttgcagtcaagcacccattgggtatgttttggcacatgcgagtttcccacttgattgatgagatggtctctcgtcgcatttaccagaccatggaacattcaggtcaagcggcctggaagcaggtggttggtgaggccactctcacgaagctgtcagggctcgatatagttactcatttccaacacctggccgcagtggaggcggattcttgccgctttctcagctcacgactcgtgatgctaaaaaatcttgccgttggcaatgtgagcctacagtacaacaccacgttggaccgcgttgagctcatcttccccacgccaggtacgaggcccaagttgaccgatttcagacaatggctcatcagtgtgcacgcttccattttttcctctgtggcttcatctgttaccttgttcatagtgctttggcttcgaattccagctctacgctatgtttttggtttccattggcccacggcaacacatcattcgagctgaccatcaactacaccatatgcatgccctgttctaccagtcaagcggctcgccaaaggctcgagcccggtcgtaacatgtggtgcaaaatagggcatgacaggtgtgaggagcgtgaccatgatgagttgttaatgtccatcccgtccgggtacgacaacctcaaacttgagggttattatgcttggctggcttttttgtccttttcctacgcggcccaattccatccggagttgttcgggatagggaatgtgtcgcgcgtcttcgtggacaagcgacaccagttcatttgtgccgagcatgatggacacaattcaaccgtatctaccggacacaacatctccgcattatatgcggcatattaccaccaccaaatagacgggggcaattggttccatttggaatggctgcggccactcttttcttcctggctggtgctcaacatatcatggtttctgaggcgttcgcctgtaagccctgtttctcgacgcatctatcagatattgagaccaacacgaccgcggctgccggtttcatggtccttcaggacatcaattgtttccgacctcacggggtctcagcagcgcaagagaaaatttccttcggaaagtcgtcccaatgtcgtgaagccgtcggtactccccagtacatcacgataacggctaacgtgaccgacgaatcatacttgtacaacgcggacctgctgatgctttctgcgtgccttttctacgcctcagaaatgagcgagaaaggcttcaaagtcatctttgggaatgtctctggcgttgtttctgcttgtgtcaatttcacagattatgtggcccatgtgacccaacatacccagcagcatcatctggtaattgatcacattcggttgctgcatttcctgacaccatctgcaatgaggtgggctacaaccattgcttgtttgttcgccattctcttggcaatatgagatgttctcacaaattggggcgtttcttgactccgcactcttgcttctggtggctttttttgctgtgtaccggcttgtcctggtcctttgccgatggcaacggcgacagctcgacataccaatacatatataacttgacgatatgcgagctgaatgggaccgactggttgtccagccattttggttgggcagtcgagacctttgtgctttacccggttgccactcatatcctctcactgggttttctcacaacaagccatttttttgacgcgctcggtctcggcgctgtatccactgcaggatttgttggcgggcggtacgtactctgcagcgtctacggcgcttgtgctttcgcagcgttcgtatgttttgtcatccgtgctgctaaaaattgcatggcctgccgctatgcccgtacccggtttaccaacttcattgtggacgaccgggggagagttcatcgatggaagtctccaatagtggtagaaaaattgggcaaagccgaagtcgatggcaacctcgtcaccatcaaacatgtcgtcctcgaaggggttaaagctcaacccttgacgaggacttcggctgagcaatgggaggcctagacgatttttgcaacgatcctatcgccgcacaaaagctcgtgctagcctttagcatcacatacacacctataatgatatacgcccttaaggtgtcacgcggccgactcctggggctgttgcacatcctaatatttctgaactgttcctttacattcggatacatgacatatgtgcattttcaatccaccaaccgtgtcgcacttaccctgggggctgttgtcgcccttctgtggggtgtttacagcttcacagagtcatggaagtttatcacttccagatgcagattgtgttgccttggccggcgatacattctggcccctgcccatcacgtagaaagtgctgcaggtctccattcaatctcagcgtctggtaaccgagcatacgctgtgagaaagcccggactaacatcagtgaacggcactctagtaccaggacttcggagcctcgtgctgggcggcaaacgagctgttaaacgaggagtggttaacctcgtcaagtatggccggtaaaaaccagagccagaagaaaaagaaaagtacagctccgatggggaatggccagccagtcaatcaactgtgccagttgctgggtgcaatgataaagtcccagcgccagcaacctaggggaggacaggccaaaaagaaaaagcctgagaagccacattttcccctggctgctgaagatgacatccggcaccacctcacccagactgaacgctccctctgcttgcaatcgatccagacggctttcaatcaaggcgcaggaactgcgtcgctttcatccagcgggaaggtcagttttcaggttgagtttatgctgccggttgctcatacagtgcgcctgattcgcgtgacttctacatccgccagtcagggtgcaagttaatttgacagtcaggtgaatggccgcgattggcgtgtggcctctgagtcacctattcaattagggcgatcacatgggggtcatacttaatcaggcaggaaccatgtgaccgaaattaaaaaaaaaaaaa

SEQ ID NO: 42 - DNA, 15182 bp, Porcine reproductive and respiratory syndrome virus
tttctccacccctttaaccatgtctgggatacttgatcggtgcacgtgtacccccaatgccagggtgtttatggcggagggccaagtctactgcacacgatgcctcagtgcacggtctctccttcccctgaacctccaagtttctgagctcggggtgctaggcctattctacaggcccgaagagccactccggtggacgttgccacgtgcattccccactgttgagtgctcccccgccggggcctgctggctctctgcaatctttccaatcgcacgaatgaccagtggaaacctgaacttccaacaaagaatgatacgggtcgcagctgagctttacagagccggccagctcacccctgcagtcttgaaggctctacaagtttatgaacggggttgccgctggtaccccattgttggacctgcccctggagtggccgtttacgccaattccctacatgtgagtgataaacctttcccgggagcaactcacgtgttgaccaacctgccgctcccgcagagacccaagcctgaagacttttgcccctttgagtgtgctatggctactgtctatgacattggtcatgacgccgtcatgtatgtggccgaaaggaaaatctcctgggcccctcgtggcggggatgaagtgaaatttgaagctgtccccggggagttgaggttgattgcgaaccggctccgcacctccttcccgccccaccacacagtggacatgtctaagttcgccttcacagcccctgggtgtggtgtttctatgcgggttgaacgccaacacggctgccttcccgctgacactgtccctgaaggcaactgctggtggagcttgtttgactcgcttccactggaagttcagaacaaagaaattcgccatgctaaccaatttggctaccagaccaagcatggtgtctctggcaagtacctacagcggaggctgcaagttaatggtctccgagcagtaactgacctaaacggacctatcgtcgtacagtacttctccgttaaggagagttggatccgccatttgaaactggcgggagaacccagctactctgggtttgaggacctcctcagaataagggttgagcctaacacgtcgccattggctgacaaggaagaaaaaattttccggtttggcagtcacaagtggtacggcgctggaaagagagcaagaaaagcacgctcttgtgcgactgccacagtcgctggccgcgctttgtccgttcgtgaaacccggcaggccaaggagcacgaggttgccggcgccaacaaggctgagcacctcaaacactactccccgcctgccgaagggaattgtggttggcattgcatttccgccatcgccaaccggatggtgaattccaaatttgaaaccacccttcccgaaagagtgagacctccagatgactgggctactgacgaggatcttgtgaatgccatccaaatcctcagactccctgcggccttagacaggaacggtgcttgtactagcgccaagtacgtacttaagctggaaggtgagcattggactgtcactgtggcccctgggatgtccccttctttgctccctcttgaatgtgttcagggctgttgtgggcacaagggcggtcttggttccccagatgcagtcgaggtctccggatttgaccctgcctgccttgaccggctggctgaggtgatgcacctgcctagcagtgctatcccagccgctctggccgaaatgtctggcgattccgatcgttcggcttctccggtcaccaccgtgtggactgtttcgcagttctttgcccgtcacagcggagggaatcaccctgatcaagtgcgcttagggaaaattatcagcctttgtcaggtgattgaggactgctgctgttcccagaacaaaaccaaccgggtcaccccggaggaggtcgcagcaaagattgacctgtacctccgtggtgcaacaaatcttgaagaatgcttggccaggcttgagaaagcgcgcccgccacgcgtaatcgacaccttctttgattgggatgttgtgctccctggggttgaggcggcaacccagacgatcaagctgccccaggtcaaccagtgtcgtgctctggtccctgttgtgactcaaaagtccttggacgacaactcggtccccctgaccgccttttcactggctaactactactaccgtgcgcaaggtgacgaagttcgtcaccgtgaaagactaaccgccgtgctctccaagttggaaaaggttgttcgagaagaatatgggctcatgccaaccgagcctggtccacggcccacactgccacgcgggctcgacgaactcaaagaccagatggaggaggacttgctgaagctggctaacgcccagacgacttcggacatgatggcctgggcagtcgagcaggttgacctaaaaacttgggtcaagaactacccgcggtggacaccaccaccccctccgccaaaagttcagcctcgaaaaacgaagcctgtcaagagcttgccggagagaaagcctgtccccgccccgcgcaggaaggttgggtccgattgtggcagcccggtttcattaggcggcgatgtctctaacagttgggaagatttggctgttagtagcccctttgatctcccgaccccacctgagccggcaacaccttcaagtgagctggtgattgtgtcctcaccgcaatgcatcttcaggccggcgacacccttgagtgagccggctccaattcccgcacctcgcggaactgtgtctcgaccggtgacacccttgagtgagccgatccctgtgcccgcaccgcggcgtaagtttcagcaggtgaaaagattgagttcggcggcggcaatcccaccgtaccagaacgagcccctggatttgtctgcttcctcacagactgaacatgaggcctctcccccagcaccgccgcagagcgggggcgttccgggagtagaggggcatgaagctgaggaaaccctgagtgaaatctcggacatgtcgggtaacattaaacctgcgtccgtgtcatcaagcagctccttgtccagcgtgagaatcacacgcccaaaatactcagctcaagccatcatcgactcgggcgggccctgcagtgggcatctccaagaggtaaaggaaacatgccttagtgtcatgcgcgaggcatgtgatgcgactaagcttgatgaccctgctacgcaggaatggctttctcgcatgtgggatcgggtggacatgctgacttggcgcaacacgtctgtttaccaggcgatttgcaccttagatggcaggttaaagttcctcccaaaaatgatactcgagacaccgccgccctatccgtgtgagtttgtgatgatgcctcacacgcctgcaccttccgtaggtgcggagagcgaccttaccattggctcagttgctactgaagatgttccacgcatcctcgagaaaatagaaaatgtcggcgagatggccaaccagggacccttggccttctccgaggataaaccggtagatgaccaacttgtcaacgacccccggatatcgtcgcggaggcctgacgagagcacatcagctccgtccgcaggcacaggtggcgccggctcttttaccgatttgccgccttcagatggcgcggatacggacgggggggggccgtttcggacggcaaaaagaaaagctgaaaggctctttgaccaactgagccgtcaggtttttgacctcgtctcccatctccctgttttcttctcacgccttttctaccctggcggtggttattctccgggtgattggggttttgcagcttttactctattgtgcctctttttatgttacagttacccagcctttggtattgctcccctcttgggtgtgttttctgggtcttctcggcgcgttcgaatgggggtttttggctgctggttggcttttgctgttggtctgttcaagcctgtgtccgacccagtcggcgctgcttgtgagtttgactcgccagagtgtagaaacatccttcattcttttgagcttctcaaaccttgggaccctgttcgcagccttgttgtgggccccgtcggtctcggtcttgccattcttggcaggttactgggcggggcacgctgcatctggcactttttgcttaggcttggcattgttgcagactgtatcttggctggagcttacgtgctttctcaaggtaggtgtaaaaagtgctggggatcttgtataagaactgctcctaatgaggtcgcttttaacgtgtttcctttcacacgtgcgaccaggtcgtcacttatcgacctgtgcgatcggttttgtgcgccaaaaggaatggaccccatttttctcgccactgggtggcgcgggtgctgggccggccgaagccccattgagcaaccctctgaaaaacccatcgcgtttgcccaattggatgaaaagaagattacggctaggactgtggtcgcccagccttatgaccccaaccaagccgtaaagtgcttgcgggtattgcaggcgggtggggcgatggtggctaaggcggtcccaaaagtggttaaggtttccgctgttccattccgagctcccttctttcccactggagtgaaagttgaccctgattgcagggtcgtggttgaccctgacactttcactgcagctctccggtctggctactccaccacaaacctcgtccttggtgtaggggactttgcccagctaaatggattaaaaatcaggcaaatttccaagccttcagggggaggcccacatctcatggctgccctgcatgttgcctgctcgatggctctgcacatgcttgctgggatttatgtgactgcggtgggttcttgcggcaccggcaccaacgacccgtggtgcgctaacccgtttgccgtccctggctacggacctggctctctctgtacgtccagattgtgcatttcccaacacggccttaccctgcccttgtcagcacttgtggcgggattcggtattcaagaaattgccttggtcgttttgatttttgtttccatcggaggcatggctcataggttgagctgtaaggctgacatgctgtgtgttttgcttgcaattgccagctatgtttgggtacctcttacctggttgctttgtgtgtttccttgctggttgcgctgtttttctttgcaccccctcaccatcctatggttggtgtttttcttgatttctgtgaatatgccttcaggaatcttggccatggtgttgttggtttctctttggcttcttggtcgttatactaatgttgctggccttgtcaccccctacgacattcatcattacaccagtggcccccgcggtgttgccgccttggctaccgcaccagatgggacctacttggccgctgtccgccgcgctgcgttgactggccgcaccatgctgtttaccccgtcccagcttgggtctcttcttgagggtgccttcagaactcgaaagccctcactgaacaccgtcaatgtgatcgggtcctccatgggctctggcggggtgtttaccatcgacgggaaagtcaagtgcgtaactgccgcacatgtccttacgggcaattcagctcgggtttccggggtcggcttcaatcaaatgcttgactttgacgtaaagggagatttcgctatcgctgattgcccgaattggcaaggggctgcccccaagacccaattctgcacggatggatggactggccgtgcctattggctaacatcctctggcgtcgaacccggcgtcattggaaaaggattcgccttctgcttcaccgcatgtggcgattccgggtccccagtgatcaccgaggccggtgagcttgtcggcgttcacacgggatcgaataaacaaggggggggcattgttacgcgcccctcaggccagttttgtaatgtggcacccatcaagctaagcgaattaagtgaattctttgctgggcctaaggtcccgctcggtgatgtgaaggtcggcagccacataattaaagacataagcgaggtgccttcagatctttgtgccttgcttgctgccaaacctgaactggaaggaggcctctccaccgtccaacttctttgtgtgttttttctcctgtggagaatgatgggacatgcctggacgcccttggttgctgtgagtttctttattttgaatgaggttctccctgccgtcctggtccggagtgttttctcctttggaatgtttgtgctatcctggctcacgccatggtctgcgcaagttctgatgatcaggcttctgacagcagctcttaacaggaacagatggtcacttgcctttttcagcctcggtgcagtgaccggttttgtcgcagatcttgcggccactcaggggcatccgttgcaggcagtgatgaatttgagcacctatgcattcctgcctcggatgatggttgtgacctcaccagtcccagtgatcacgtgtggtgtcgtgcacctacttgccatcattttgtacttgtttaagtaccgtggcctgcaccatatccttgttggcgatggagtgttctctgcggctttcttcttgagatactttgccgagggaaagttgagggaaggggtgtcgcaatcctgcggaatgaatcatgagtctctgactggtgccctcgctatgagactcaatgacgaggacttggatttccttatgaaatggactgattttaagtgctttgtttctgcgtccaacatgaggaatgcagcgggtcaatttatcgaggctgcctatgctaaagcacttagagtagaactggcccagttggtacaggttgataaagttcgaggtactttggccaaacttgaagcttttgctgataccgtggctcctcaactctcgcccggtgacattgttgtcgctctcggccacacgcctgttggcagtatcttcgacctaaaggttggtagcaccaagcataccctccaagccattgagaccagagtccttgctgggtccaaaatgaccgtggcgcgcgtcgtcgacccgacccccacgcccccacccgcacccgtgcccatccccctcccaccgaaagttctggagaatggccccaacgcttggggggatgaggaccgtttgaataagaagaagaggcgcaggatggaagccctcggcatctatgttatgggcgggaaaaagtaccagaaattttgggacaagaattccggtgatgtgttttatgaggaggtccataataacacagatgagtgggagtgtctcagagttggcgaccctgccgactttgaccctgagaagggaactctgtgtggacatgtcaccattgaaaataaggcttaccatgtttacacctccccatctggtaagaagttcttggtccccgtcaacccagagaatggaagagttcaatgggaagctgcaaagctttccgtggagcaggccctaggtatgatgaatgtcgacggcgaactgactgccaaagaactggagaaactgaaaagaataattgacaaactccagggcctgactaaggagcagtgtttaaactgctagccgccagcgacttgacccgctgtggtcgcggcggcttggttgttactgaaacagcggtaaaaatagtcaaatttcacaaccggaccttcaccctgggacctgtgaatttaaaagtggccagtgaggttgagctaaaagacgcggttgagcacaaccaacacccggttgcgagaccgatcgatggtggagttgtgctcttgcgttccgcggttccttcgcttatagacgtcttgatctccggtgctgatgcatctcccaagttacttgcccatcacgggccgggaaacactgggatcgatggcacgctctgggattttgagtccgaagccactaaagaggaagtcgcactcagtgcgcaaataatacaggcttgtgacattaggcgcggcgacgctcctgaaattggtctcccttacaagctgtaccctgttaggggtaaccctgagcgggtgaaaggagttctgcagaatacaaggtttggagacataccttacaaaacccccagtgacactggaagcccagtgcacgcggctgcctgccttacgcccaacgccactccggtgactgatgggcgctccgtcttggccacgaccatgccccccgggtttgagttatatgtaccgaccataccagcgtctgtccttgattaccttgactctaggcctgactgccctaaacagctgacagagcacggctgcgaagatgccgcactgaaagacctctctaaatatgacttgtccacccaaggctttgttttacctggagttcttcgccttgtgcggaaatacctgtttgcccatgtaggtaagtgcccacccgttcatcggccttctacttaccctgctaagaattctatggctggaataaatgggaacaggttcccaaccaaggacattcagagcgtccctgaaatcgacgttctgtgcgcacaggctgtgcgagaaaactggcaaactgtcaccccttgtactcttaagaaacagtattgcgggaagaagaagactaggaccatactcggcaccaataacttcatcgcactagcccaccgagcagtgttgagtggtgttacccagggcttcatgaaaaaggcgtttaactcgcccatcgccctcggaaagaacaagtttaaggagctacagactccggtcctgggcaggtgccttgaagctgatctcgcatcctgcgatcgatccacgcctgcaattgtccgctggtttgccgccaaccttctttatgaacttgcctgtgctgaagagcatctaccgtcgtacgtgctgaactgctgccacgacttactggtcacgcagtccggcgcagtgactaagagaggtggcctgtcgtctggcgacccgatcacctctgtgtctaacaccatttatagtttggtgatctatgcacagcatatggtgcttagttacttcaaaagtggtcacccccatggccttctgttcttacaagaccagctaaagtttgaggacatgctcaaggttcaacccctgatcgtctattcggacgacctcgtgctgtatgccgagtctcccaccatgccaaactatcactggtgggttgaacatctgaatttgatgctggggtttcagacggacccaaagaagacagcaataacagactcgccatcatttctaggctgtagaataataaatgggcgccagctagtccccaaccgtgacaggatcctcgcggccctcgcctatcacatgaaggcgagtaatgtttctgaatactatgcctcagcggctgcaatactcatggacagctgtgcttgtttggagtatgatcctgaatggtttgaagaacttgtagttggaatagcgcagtgcgcccgcaaggacggctacagttttcccggcacgccgttcttcatgtccatgtgggaaaaactcaggtccaattatgaggggaagaagtcgagagtgtgcgggtactgcggggccccggccccgtacgctactgcctgtggcctcgacgtctgcatttaccacacccacttccaccagcattgtccagtcacaatctggtgtggccatccagcgggttctggttcttgtagtgagtgcaaatcccctgtagggaaaggcacaagccctttagacgaggtgctggaacaagtcccgtataagcccccacggaccgttatcatgcatgtggagcagggtctcaccccccttgatccaggtagataccaaactcgccgcggactagtctctgtcaggcgtggaattaggggaaatgaagttgaactaccagacggtgattatgctagcaccgccttgctccctacctgcaaagagatcaacatggtcgctgtcgcttccaatgtactgcgcagcaggttcatcatcggcccacccggtgctgggaaaacatactggctccttcaacaggtccaggatggtgatgttatttacacaccaactcaccagaccatgcttgacatgattagggctttggggacgtgccggttcaacgtcccggcaggcacaacgctgcaattccccgtcccctcccgcaccggtccgtgggttcgcatcctagccggcggttggtgtcctggcaagaattccttcctagatgaagcagcgtattgcaatcaccttgatgttttgaggcttcttagtaaaactaccctcacctgtctaggagacttcaagcaactccacccagtgggttttgattctcattgctatgtttttgacatcatgcctcaaactcaactgaagaccatctggaggtttggacagaatatctgtgatgccgttcagccagattacagggacaaactcatgtccatggtcaacacaacccgtgtgacctacgtggaaaaacctgtcaggtatgggcaggtcctcaccccctaccacagggaccgagaggacgacgccatcactattgactccagtcaaggcgccacattcgatgtggttacattgcatttgcccactaaagattcactcaacaggcaaagagcccttgttgccatcaccagggcaagacacgctatctttgtgtatgacccacacaggcagctgcagggcttgtttgatcttcctgcaaaaggcacacccgtcaacctcgcagtgcaccgcgacgggcagctgatcgtgctggatagaaataacaaagaatgcacggtcgctcaggctctaggcaacggggataaatttagggccacagataagcgtgttgtagattctctccgcgccatttgtgctgatctagaagggtcgagctctccgctccccaaggtcgcacacaacttgggattttatttctcacctgatttaacacagtttgctaaactcccagtagaacttgcacctcactggcccgtggtgacaacccagaacaatgaaaagtggccagatcggctggttgccagccttcgccctatccataaatacagccgcgcgtgcatcggtgccggctatatggtgggcccttcggtgtttctaggcactcctggggtcgtgtcatactatctcacaaaatttgttaagggcgaggctcaattgcttccggagacggttttcagcaccggccgaattgaggtagactgccgggaatatcttgatgatcgggagcgagaagttgctgcgtccctcccacacgctttcattggcgacgtcaaaggcactaccgttggaggatgtcatcatgtcacctccagatacctcccacgcgtccttcccaaggaatcagttgcggtagtcggggtttcaagccccggaaaagccgcgaaagcattgtgcacactgacagatgtgtacctcccagatcttgacgcctatctccacccggagacccagtccaagtgctggaaaatgatgttggacttcaaagaagttcgactaatggtctggaaagacaaaacagcctatttccaacttgaaggtcgctatttcacctggtatcagcttgccagctatgcctcgtacatccgtgttcctgtcaactctacggtgtacttggacccctgcatgggccccgccctttgcaacaggagagtcgtcgggtccacccactggggggctgacctcgcggtcaccccttatgattacggcgctaaaattatcctgtctagcgcgtaccatggtgaaatgccccccggatacaaaattctggcgtgcgcggagttctcgttggatgacccagttaagtacaaacatacctgggggtttgaatcggatacagcgtatctgtatgagttcaccggaaacggtgaggactgggaggattacaatgatgcgtttcgtgcgcgccaggaagggaaaatttataaggccactgccaccagcttgaagttttattttcccccgggccctgtcattgaaccaactttaggcctgaattgaaatgaaatggggtccatgcaaagccttttttacaaaattggccaactttttgtggatgctttcacggagttcttggtgtccattgttgatatcactatatttttggccattttgtttggcttcaccatcgccggttggctggtggtcttttgcatcagattggtttgctccgcgatactccgtacgcgctctgccattcactctgagcaattacagaagatcttatgaggcctttctttcccagtgccaagtggacattcccacctggggaactaaacatcctttggggatgctttggcaccataaggtgtcaaccctgattgatgaaatggtgtcgcgtcgaatgtaccgcatcatggaaaaagcagggcaggctgcctggaaacaggtggtgagcgaggctacgctgtctcgcattagtagtttggatgtggtggctcattttcagcatctagccgccattgaagccgagacctgtaaatatttggcctcccggctgcccatgctacacaacctgcgcatgacaggttcaaatgtaaccatagtgtataatagcactttgaatcaggtgtttgctatttttccaacccctggttcccggccaaagcttaatgattttcagcaatggttaatagctgtacattcctccatattttcctctgttgcaacttcttgtactctttttgttgtgctgtggttgcgggttccaatactacgtactgcttttggtttccgctggttaggggcaatttttctttcgaactcacagtgaattacacggtgtgtccaccttgcctcacccggcaagcagccgcagagatctacgaacccggtaggtctctttggtgcaggatagggtatgaccgatgtgaggaggatgatcatgacgagctagggtttatggtaccgcctggcctctccagcgaaggccacttgactagtgtttacgcctggttggcgttcttgtccttcagctacacggcccagttccatcccgagatattcgggatagggaatgtgagtcgagtttatgttgacatcaaacatcaactcatctgcgccgaacatgacgggcagaacaccaccttgcctcgtcatgacaacatttcagccgtgtttcagacctattaccaacatcaagtcgacggcggcaattggtttcacctagaatggcttcgtcccttcttttcctcgtggttggttttaaatgtctcttggtttctcaggcgttcgcctgcaaaccatgtttcagttcgagtcttgcagatattaagaccaacaccaccgcagcggcaagctttgctgtcctccaagacatcagttgccttaggcatcgcgactcggcctctgaggcgattcgcaaaatccctcagtgccgtacggcgatagggacacccgtgtatgttaccatcacagccaatgtgacagatgagaattatttacattcttctgatctcctcatgctttcttcttgccttttctatgcttctgagatgagtgaaaagggatttaaggtggtatttggcaatgtgtcaggcatcgtggctgtgtgtgtcaattttaccagctacgtccaacatgtcaaggagtttacccaacgctccctggtggtcgaccatgtgcggttgctccatttcatgacacctgagaccatgaggtgggcaactgttttagcctgtctttttgccattctgttggcaatttgaatgtttaagtatgttggagaaatgcttgaccgcgggctgttactcgcaattgctttctttgtggtgtatcgtgccgttctgttttgctgtgctcgtcaacgccagcaacgacagcagctcccatctacagctgatttacaacttgacgctatgtgagctgaatggcacagattggctagctaacaaatttgattgggcagtggagagttttgtcatctttcccgttttgactcacattgtctcctatggtgccctcactactagccatttccttgacacagtcgctttagtcactgtgtctaccgccgggtttgttcacgggcggtatgtcctaagtagcatctacgcggtctgtgccctggctgcgttgacttgcttcgtcattaggtttgcaaagaattgcatgtcctggcgctacgcgtgtaccagatataccaactttcttctggacactaagggcagactctatcgttggcggtcgcctgtcatcatagagaaaaggggcaaagttgaggtcgaaggtcatctgatcgacctcaaaagagttgtgcttgatggttccgtggcaacccctataaccagagtttcagcggaacaatggggtcgtccttagatgacttctgtcatgatagcacggctccacaaaaggtgcttttggcgttttctattacctacacgccagtgatgatatatgccctaaaggtgagtcgcggccgactgctagggcttctgcaccttttgatcttcctgaattgtgctttcaccttcgggtacatgactttcgcgcactttcagagtacaaataaggtcgcgctcactatgggagcagtagttgcactcctttggggggtgtactcagccatagaaacctggaaattcatcacctccagatgccgtttgtgcttgctaggccgcaagtacattctggcccctgcccaccacgttgaaagtgccgcaggctttcatccgattgcggcaaatgataaccacgcatttgtcgtccggcgtcccggctccactacggtcaacggcacattggtgcccgggttaaaaagcctcgtgttgggtggcagaaaagctgttaaacagggagtggtaaaccttgtcaaatatgccaaataacaacggcaagcagcagaatagaaagaagggggatggccagccagtcaatcagctgtgccagatgctgggtaagatcatcgctcagcaaaaccagtccagaggcaagggaccgggaaagaaaaataagaagaaaaacccggagaagccccattttcctctagcgactgaagatgatgtcagacatcactttacccctagtgagcggcaattgtgtctgtcgtcaatccagaccgcctttaatcaaggcgctgggacttgcaccctgtcagattcagggaggataagttacactgtggagtttagtttgcctacgcatcatactgtgcgcctgattcgcgtcacagcatcaccctcagcatgatgggctggcattcttgaggcatctcagtgtttgaattggaagaatgtgtggtgaatggcactgattgacattgtgcctctaagcactatatt

SEQ ID NO: 43 - protein, 183 aa, Porcine reproductive and respiratory syndrome virus
MAAATLFFLAGAQHIMVSEAFACKPCFSTHLSDIETNTTAAAGFMVLQDINCFRPHGVSAAQEKISFGKSSQCREAVGTPQYITITANVTDESYLYNADLLMLSACLFYASEMSEKGFKVIFGNVSGVVSACVNFTDYVAHVTQHTQQHHLVIDHIRLLHFLTPSAMRWATTIACLFAILLAI

SEQ ID NO: 44 - protein, 178 aa, Porcine reproductive and respiratory syndrome virus
MASSLLFLVVGFKCLLVSQAFACKPCFSSSLADIKTNTTAAASFAVLQDISCLRHRDSASEAIRKIPQCRTAIGTPVYVTITANVTDENYLHSSDLLMLSSCLFYASEMSEKGFKVVFGNVSGIVAVCVNFTSYVQHVKEFTQRSLVVDHVRLLHFMTPETMRWATVLACLFAILLAI

SEQ ID NO: 45 - DNA, 14622 bp, Porcine reproductive and respiratory syndrome virus
atgtctgggatgttctcccggtgcatgtgcaccccggctgcccgggtattttggaacgccggccaagtctattgcacacggtgtctcagtgcacggtctcttctctctccagaacttcaggacacggacctcggtgcagttggcttgtttcacaagcctaaagacaagctccattggaaagttcccattggtatcccccaggtggaatgttctccatctgggtgttgctggctgtcaaccatttttcctttagcgcgcatgacctccggcaatcacaacttccttcaacgactcgtgaaggttgctgatgtattgtaccgtgacggttgcttaacccctagacacctccgtgaactccaagtttacgagcgtggttgcaattggtatccgattacggggcctgtgcctgggatggctgtgtacgcgaactccatgcacgtgtccgaccaaccgttccctggtgccactcatgtgttaacaaattcccctttgcctcaacgggcttgtcggcagccgttctgtccgttcgaagaggcccattctagcatatacaggtgggaaaaatttgtaatttttatggattcctcctccgacggtcgatctcgcatgatgtggactccggaatccgatgactccacggctttggaagttctgccgcccgagctagaacaccaggtcaaggtccttgttcggagctttcccgcccatcaccttgtcgaccttgccgattgggagctcactgagtcccctgataacggtttttccttcagcacgtcacatccttgcggctaccttgttcgggacccggctgtatccgaaggcaagtgttggctttcctgctttttgagccagtcagccgaagtgctcagtcgcgaggcgcatctggctaccgcctatggttaccaaaccaagtggggtgtgcctggcaagtacatccagcgcagacttcaagttcacggtctccgtgctgtggtcgaccctgatggtcccattcacgttgaagcattgtcttgcccccagtcttggatcaggcacttgaccctgaatgatgatgtcaccccgggattcgttcgcctaatgtctcttcgcattgtgccgaacacagagcctaccacacaccggatctttcgttttggagtgcacaagtggtatggtgccgccggcaaacgggcccgtggcaagcgtgccgccaaaagtgagaaagactcggcttccaccctcaaggttgcccgaccgacttccaccagtggaatcgtcacctactccccacctgcggacgggtcttgtggttggcatgcccttgccgccatactgaaccggatgattaataatgacttcacgtcccctctgcctcggtacaacaggccggaggacgattgggcttctgatggtgaccttgctcaggccattcaatgtttgcaactacctgccgccatagctcggaaccgcgcctgccctaacgccaaatacctcataaaactcaacggagttcattgggaggtagaggtgaggcctggaatggctcctcgctccctctctcgtgagtgcgttgttggcgtctgctctgaaggctgtgtcgcgtcgccttacccggaggacgggttgcctaaacgtgcacttgaggccctggcgtctgcttatagactgccttcagactgtgtttgtgatggtattattgacttccttgccaatccacctccccaggagttctggactcttgacaaaatgttgacttccccgtcaccggagcagtccggcttctctagtctgtataaattgttgttagagatcttgccgcagaaatgcggatccacagaaggggaattcatctatactgttgagaggatgttgaaggattgtccgagctccaaacaggccatggccctccttgcaaaaattaaggtcccatcctcaaaggccccatccgtgactctgaacgagtgcttccccacggatgttccagtcaactctgagttaatatcttgggaagagcccaaagaccctggcgctgctgttgtcctatgtccatcggatgcaaaagaatctaaggaaacagcccctgaagaagctcaagcgagaaaccgtaaggtccttcaccctgtggtccttaccgaggaacttagcgagcaacaggtgcaggtggttgagggtgatcaggatatgccactggatttgacttggccaaccttaaccgctacggcgacccctgttagagggccggtaccggacaatttgagctctggcattggtgcccagcccgctaccgttcaagaactcattctggcgaggcctgcaccccgtcttgttgagcgctgtggcacggagtcgaacggcagcagttcatttctggatttgcctgacgtgcagacctcggaccagcctttagacctgtccctggccgcgtggcctgtaagggctaccgcgtctgaccccggttggatccacggtaggcgtgagcctgtctttgtgaagcctcgaggtgttttctctgatggcgagtcggcccttcagttcggagagctttccgaagccagttctgtcgtcgatgaccggacaaaagaagctccggtggttgacgcccccatcgatttgacaacttcgaacgagacgctctctgggtctgacccctttgaattcgccaaattcaggcgcccgcgtttctccgcgcaagctttaatcgaccgaggtggtccgcttgccgatgttcatgcaaagataaagagtcgggtatatgaacaatgccttcaagcttgtgaacctggtagtcgtgcgaccccagccaccaagaagtggctcgacaaaatgtgggacagggtggacatgaaaacttggcgctgcacctcgcagttccaagctggtcacattcttgagtccctcaaattcctccctgacatgattcaagacacaccgcctcctgttcccaggaagaaccgagctggtgacagtgccggcctgaagcaactggtggcgcagtgggataggaaatcgagtgtgacaccccccacaaaaccggttggaccggtgcttgaccaggccgtccctctgcctatggacatccagcaaggagatgccatctccgctgacaagccaccccattcgcaaaacccttctagtcaagtagatgtgggtggaggttggaaaagttttatgctctccggcacccgtttcgcggggtccgttagtcagcgccttacgacatgggtttttgaggttctctcccatctcccagcttttatgctcacacttttctcgccacggggctctatggctccaggtgattggctgtttgcaggtgctgttctacttgctctcctgctctgccgttcttacccaatactcggatgccttcccttattgggtgtcttttctggttctgtgcggtgtgttcgtttgggtgtttttggttcttggatggcttttgctgtatttttattctcgactccacccgacccagtcggttcttcttgtgaccacgattcgccggagtgtcatgctgagcttttggctcttgagcagcgccaactttgggaacctgtgcgcagccttgtggtcgggccatcgggcctcttatgcgtcattcttggcaagttactcggtgggtcacgttgtctctggtttgttctcctacgtatatgcatgctcgcagatttggcaatttctcttatttatgtggtgtcccaagggcgttgtcacaagtgttggggaaagtgtataaggacggctcctgcagaagtggcccttaatgtgtttcctttttcgcgcgccacccgctcatctcttgtgtccttgtgtgatcggttccaagcgccaaaaggagttgaccccgtgcacttggcgacaggctggcgcgggtgctggtgtggtgagagccctattcatcaatcacaccaaaaaccgatagcttatgccaacttggatgaaaagaagatatccgcccagacggtgattgctgtcccgtatgatcctagtcaggccattaaatgcctgaaagttttgcaggcaggaggggctattgtggaccagcctacgcccgaggtcgtccgtgtgtctgagattcccttctcggccccattttttccgaaggtcccagtcaacccagactgcagggttgtggtagattcggacacttttgtggctgcggtccgctgcggttattcgacagcacaactggtccttggtcggggcaactttgccaagctaaatcagacccccctcaggaactctgtccccaccaaaacaactggtggggcctcatacacccttgccgtggcccaggtatctgtgtggactcttgttcatttcatcctcggcctttggttaacgtcacctcaagtgtgtggtcgagggacctctgacccgtggtgttcgaaccctttttcgtatcctacttatggccccggagttgtgtgttcctctcgactctgcgtgtctgccgacggagttaccctgccattgttctcagccgttgcccatctttccggtagagaggtggggatttttattttggtgcttgcctccttgggcgctttagcccaccgcttggctcttaaggcagacatgtcaatggtctttttggcgttttgtgcttacgcctggcccatgagctcctggttaatttgcttctttcctatgctcttgaggtgggtaacccttcatcctctcactatgctttgggtgcactcatttttggtgttttgcctaccagctgccggcgttctctcgctgggaataaccggtcttctttgggcagttggccgtttcacccaggttgccggaattatcacaccttatgacatccaccagtatacctccggaccacgtggtgcagctgctgtagcaacggctccagaaggtacttacatggcggccgttcggagagccgctttgactggacggactttgatcttcacaccatctgcagtcggatcccttcttgaaggtgctttcagaactcaaaagccctgccttaacaccgtgaatgtcgtaggctcttcccttggttctggaggagttttcaccattgatggcagaagagtcatcgtcactgccacccatgtgttgaatggtaacacagccagggtcactggtgattcctacaaccgcatgcacacgttcaatactaatggtgattatgcctggtcccatgctgatgactggcaaggcgttgcccctatggttaagatcgctaaggggtatcgcggtcgtgcctactggcaaacgtcaaccggagtcgaacctggcatcatgggggaaggattcgccttctgtttcactaactgtggcgactcagggtcacctgtcatttcagaagctggtgaccttattggagtccataccggttcaaacaaactcggttctggtcttgtgacaacccctgaaggggagacctgctccatcaaggaaactaggctctctgacctttctagacattttgcaggtccaagcgtccctcttggggacattaagttgagcccagccatcatccctgatgtgacaactattccgagtgacttggcatcgctccttgcttctgtccccgtgatggaaggtggcctctcaactgtccagcttttgtgcgtctttttccttctctggcgcatgatgggccatgcctggacacccattgttgccgtaggcttctttttgctgaatgaaattctcccagcagtcttggtccgagctgtgttctcttttgcactctttgtacttgcatgggccaccccctggtcggcacaagtgttgatgattagactcctcacggcggctctcaaccgcaacaggttgtccctggcgttctacgcattcggaggtgtcgttggcctggccacagaaatcgggacttttgctggtggatggcctgaactgtcccaagccctctcgacatactgcttcctgcccaggttccttgctgtgactagttatgtccccaccatcatcatcggtgggctccatgccctcggcgtaattttgtggttattcaaataccgatgcctccacaacatgctggttggtgatgggagtttctcaagcgctttcttcctacggtattttgctgagggtaatcttaggaaaggcgtgtcgcagtcctgtggcatgaataacgaatccctgacagctgctttggcttgcaagttgtcgcaagctgaccttgattttttgtccagtttaacgaacttcaagtgctttgtgtccgcttcaaacatgaaaaatgcagctggccaatacatcgaggcggcgtatgctagagctctgcgtcaggagctggcctccttggttcaggttgacaagatgaaaggagtattggccaagctcgaggctttcgctgagacggccactccgtcacttgacacaggggacgtgattgttctgcttgggcaacacccccatggatccatcctcgacattaatgtggggggtgaaaggaaaactgtgtctgtgcaagaaacacgatgcctgggtggttccaaattcagtgtctgcactgtcgtgtccaacacgcccgtggataccttgaccggtatcccacttcagacgccaaccccactttttgaaaatggcccgcgccatcgcagcgaggacgacgacctcaaagttgagagaatgaaaaaacactgtgtatccctcggcttccacaaaatcaatggtaaagtttactgcaaaatttgggacaagtctaacggcgacaccttttacacggatgattcccgatacactcaagaccatgcttttcaggacaggtcaaccgactatagagacagggattatgaaggtgtacagaccgccccccaacagggattcgatccaaagtccgaagcccctgttggcactgttgtaatcggtggcattacgtataacaggcatctggtcaaaggtaaggaggtcctagttcccaaacctgacaactgccttgaagctgccagactgtcccttgagcaagctcttgctgggatgggccaaacttgtgaccttacagctaccgaagtggagaaactaaagcgcatcattagtcaactccaaggtctgaccactgaacaggctttaaactgctagccgccagcggcttgacccgctgtggccgcggcggcctagttgtaactgaaacggcggtaaaaatcgtaaaataccacagcagaactttcaccttaggctctttagacctaaaagtcacctccgaggtggaggtgaagaaatcaactgagcaggggcacgctgtcgtggcgaacttatgttccggtgtcgtcttgatgaggcctcacccaccgtcccttgttgacgttctcctcaaacccggacttgacacaacacccggcattcaaccagggcatggggccgggaatatgggcgtgaacggttctatttgggattttgaaactgcacccacaaaggtagaactagagttgtccaagcaaataatccaagcatgtgaagtcaggcgcggggacgcccctaacctccaactcccctacaagctttatcctgtcaggggggaccccgagcggcgtaaaggtcgccttgtcaacactaggtttggagatttaccttacaaaactccccaagacaccaagtccgcaattcatgcggcttgttgcctgcatcccaatggggtcctcgtgtctgatggcaaatccacgctgggtaccactcttcaacatggtttcgagctttatgtccccactgtaccttatagtgtcatggaataccttgattcacgccctgacaccccttttatgtgtactaaacatggcacttccaaggctgctgcagaggacctccaaaaatatgacctatccactcaagggtttgtcttgcctggggtcctacgcctagtgcgcaggttcatctttagccatgttggtaaggcgccaccactgttccttccatcaacctaccctgccaagaactccatggcaggggtcaatggccagaggttcccaacaaaggatgtccagagcatacctgaaattgatgaaatgtgcgcccgtgccgtcaaggaaaattggcagactgtgacaccttgcaccctcaaaaaacagtactgttccaaacctaaaactagaaccatcctaggtaccaacaacttcatagccttggctcacaggtcagcactcagtggtgtcacccaggcgttcatgaagaaggcctggaagtccccaattgccttggggaaaaacaagtttaaggaattgcattgcactgtcgccggcagatgccttgaggctgacctggcttcctgcgatcgcagcacccccgccattgtgaggtggtttgttgccaacctcctgtatgaacttgcaggatgtgaagagtacttgcctagctacgtgctcaactgttgccatgaccttgtggcaacgcaggatggcgctttcacaaaacgcggtggcctgtcgtccggggaccccgtcaccagtgtgtccaacaccgtctactcactgataatttacgcccagcacatggtgctttcggccttgaagatgggtcatgaaattggtctcaagttccttgaggaacagctcaaatttgaggaccttcttgaaatccagcccatgttagtgtattctgatgacctcgtcttgtatgcggaaagacccacttttcccaactaccattggtgggtcgagcatcttgacctgatgttgggctttaaaacggacccaaagaaaactgtcataactgataaacccagttttctcggctgcagaattgaagcaggacggcagttagtccccaatcgcgaccgtattctggctgctcttgcatatcatatgaaggcgcagaacgcctcagagtattatgcgtccgctgccgcaattctgatggattcgtgtgcttgcattgaccatgaccccgagtggtatgaggatcttatctgcggcatcgcccggtgtgctcgccaggacggttaccgttttccaggcccggcatttttcatgtccatgtgggagaagctgaaaagtcataatgaagggaagaaatgccgtcactgcggcatctgcgacgccaaagccgactatgcgtccgcctgtggacttgatttgtgtttgttccattcacactttcatcaacactgcccagtcactctgagctgtggccaccatgccggttcaaaggaatgttcgcagtgtcagtcacctgtcggggctggcaaatccccccttgacgctgtgctgaaacaaatcccgtacaaacctcctcgtaccattatcatgaaggtggacaacaaaacaacgacccttgacccgggaagatatcagtcccgtcgaggtcttgttgcagtcaaaagaggtattgcaggtaatgaggttgatctttctgatggagactaccaagtggtgcctcttttgccgacttgcaaagacataaacatggtgaaggtggcttgcaacgtactactcagcaagtttatagtagggccgccaggttccggaaaaaccacctggctactgaaccaagtccaggacgatgatgtcatttacacacctactcatcagacaatgtttgacatagtcagtgctcttaaagtttgcaggtattccatcccaggagcctcaggactcccttttccaccacctgccaggtccgggccgtgggttaggctcatcgccagcggacatgtccctggccgagtgtcatatctcgatgaggcaggatattgcaatcatctagacattctaaggctgctttccaaaacaccccttgtgtgtttgggtgaccttcagcaacttcacccggtcggctttgattcctattgttatgtgttcgatcagatgcctcagaagcagctgaccaccatttatagatttggccctaacatctgtgcagccatccagccttgttacagggagaaacttgaatccaaggccaggaacaccagagtggttttcaccacccggcctgtggcctttggtcaggtcctgacaccgtaccacaaagatcgtaccggctctgcaataactatagattcatcccagggggcgaccttcgacattgtgacattgcatctaccatcgccaaagtccctaaacaaatcccgagcacttgtagccatcactcgggcaagacatgggttgttcatttatgaccctcatgaccaactccaggagtttttcaacttaacccccgagcgcactgattgtaaccttgcgttcagccgtggggatgagctggttgttttgaatgtggataatgcggtcacaactgtagcgaaggccctagagacaggttcaccccgatttcgagtatcggacccgaggtgcaagtctctcttagccgcttgttcggccagtctagaagggagctgcatgccactaccacaagtagcacataacctggggttttacttttccccggacagcccagcttttgcacccctgccaaaagagctggcgccacattggccagtggtcacccaccagaataatcgagcgtggcctgatcgacttgtcgctagtatgcgcccaattgatgcccgctacagcaagccaatggtcggtgcagggtatgtggtcgggccatccatttttcttggcactcctggtgtggtgtcatactatctcacattatacatcgggggcgagcctcaggccctgccagaaacactcgtttcaacaggacgtatagccacagattgtcgggaatatctcgacgcggctgaggaagaggcagcgagagaacttccccacgcatttattggcgatgtcaaaggcactacgatcggggggtgtcaccacattacatcgaaatacctacctaggtccctgcctaaagactctgttgctgtggttggggtgagttcgcccggtagggctgctaaagccgtgtgcactctcaccgatgtgtacctccccgaactccgaccatatttgcaaccggagacggcatcaaaatgctggaaacttaaactggatttcagggatgttcgactgatggtctggaaaggcgccacagcctatttccagttggaagggctgacatggtcagcgctgcccgattatgctaggttcattcagctacccaaggatgccgttgtgtacatcgatccgtgtatagggccggcaacagccaatcgcaaggttgtgcgaaccacagactggcgggccgacctggcagtgacaccgtatgattacggtgctcaggtcattttgacaacagcctggttcgaggaccttgggccgcagtggaagattttggggttgcagcctttcagacgaacatttggctttgagaacactgaagattgggcaattctcgcacgccgtatgaatgacggcaaagattacactgactataattggcattgtgtacgagaacgcccacacgcaatttacgggcgcgcccgtgaccatacgtatcattttgcccttggcactgaactgcaagtagagctgggcagaccccggctgcctcctgagcaagtgccgtgaacgcggagtgatgcaatgggtttactgtggagtaaaatcagtcagttgttcgtggatgccttcactgagttccttgttagtgtggttgacattgtcatctttctcgccatattgtttgggttcactgttgcaggctggttattggtcttccttctcagagtggtttgctccgcgtttctccgttcgcgctctgccattcactcttccgaactatcgaaggtcctatgagggcttgctacccaactgcagaccggatgtcccacaattcgcagttaagcacccgttgggtatactttggcatatgcgagtctcccacctaattgacgaaatggtctctcgccgcatttaccggaccatggaacattcgggtcaagcggcctggaagcaggttgttagtgaagccactctcacaaaactgtcaaggcttgacgtagtcactcatttccaacacctggccgcagtggaggctgattcttgccgcttccttagctcacgactcgcgatgctgaaaaaccttgccgttggcaatgtgagcctggagtacaacactactttggaccgcgttgagctcatctttcccacaccaggtacgaggcccaagttgaccgattttaggcaatggcttatcagcgtgcacgcttccatcttctcctctgtggcttcgtctgttaccttgttcacagtgctttggcttcgaattccagctctacgctatgtttttggtttccattggcccacggcaacacatcattcgaactaactatcaattacactatatgtaagccatgccctaccagtcaagctgcccaacaaagactcgagcctggccgtaacgtgtggtgcaaaatagggcacgacaggtgtgaggaacgtgaccatgatgagttgtcaatgtccattccgtccgggtacgacaacctcaaacttgagggttattatgcttggctggcttttttgtccttttcctacgcggcccaattccatccggagctgttcggaataggaaacgtgtcgcgcgtctttgtggataagcgacaccagttcatttgcgccgagcatgatggacaaaattcaaccatatctgccagacacaacatctccgcgtcgtatgcggtgtattaccatcatcaaatagacgggggcaattggtttcatttggaatggctgcgaccattcttttcctcctggctggtgctcaacatctcatggtttctgaggcgttcgcctgcaagccctgcttctcgacgcatctatcagatattaagaccaacacgaccgcggctgccggtttcatggtccttcagaacatcaattgtttccaatctcacagggcctcaacagcgcaaggtaccactcccctcaggaggtcgtcccaatgtcgtgaagccgtcggcattccccagtacatcacgataacggctaatgtgaccgatgaatcgtatttgtacaacgcggacttgctgatgctttccgcgtgccttttctacgcctcggaaatgagcgagaaaggcttcaaagtcatctttgggaatatttctggcgttgtttccgcttgtgttaatttcacagattatgtggcccatgtgacccaacacactcagcagcaccatttggtaattgatcacattcggttactacacttcttgacaccgtctacgatgaggtgggctacaaccattgcttgtttgcttgccattcttttggcggtatgaaatgttcttgcaagttggggcatttcttgactcctcactcttgcttctggtggctttttttgctgtgtaccggcttgtcttggtcctttgtcgatggcaacgacgacagctcgacatcccaatacatatataatttgacgatatgcgagctgaatgggaccgaatggttgtccggtcattttgattgggcagtcgaaacctttgtgctttacccagttgccactcatatcatttcactgggttttctcacaacaagccatttccttgatgcgctcggtctcggcgctgtgtccgccacaggattcattggcgagcggtatgtacttagcagcatgtacggcgtttgcgccttcgcggcgttcgtatgttttgtcatccgtgctgctaaaaattgcatggcttgccgctatgcccgcacccggtttaccaacttcatcgtggacgaccggggaagaatccatcgatggaagtcttcaatagtggtggagaaattgggcaaagctgaagtcggtggtgaccttgtcaacattaagcatgttgtcctcgaaggggttaaagctcaacctttgacgaggacttcggctgagcaatgggaagcctagacgacttttgcaacgatcccaccgccgcacaaaaactcgtgctggcctttagcatcacatatacacccataatgatatacgcccttaaggtgtcacgcggccgactcctggggctgttgcacatcttgatatttctgaattgttcctttacttttgggtacatgacatatgtgcattttcaatccaccaaccgtgtcgcattcactctgggggctgtagtcgcccttttgtggggtgtttacagcctcacagagtcatggaagttcatcacttccagatgcagattgtgttgcctaggccggcgatacattctggcccctgcccatcacgtagaaagtgctgcaggcctccattcaatcccagcgtctggtaaccgagcatacgctgtgagaaagcccggactaacatcagtgaacggcactctagtacctgggcttcggagcctcgtgctgggcggcaaacgagctgttaaacgaggagtggttaacctcgtcaagtatggccggtaagaaccagagccagaagaaaagaagaaatgcagctccgatggggaaaggccagccagtcaatcaactgtgccagttgctgggtacaatgataaagtcccagcgccagcaatctaggggaggacaggccaaaaagaagaagcctgagaagccacattttcccctagctgctgaagatgacattcggcaccatctcacccaggccgaacgttccctctgcttgcaatcgatccagacggctttcaatcaaggcgcaggaactgcgtcgctttcatccagcgggaaggtcagtttccaggttgagttcatgctgccggttgctcatacagtgcgcctgattcgcgtgacttctacatccgccagtcagggtgcaaattaa

SEQ ID NO: 46 - DNA, 221 bp, Porcine reproductive and respiratory syndrome virus
atgatgtgtagggtattccccctacatacacgacactcttagtgtttgtgtaccttggaggcgtgggtacagccctgccccaccctttggtccctgttctagcccgacaggtacccttctctctcggggcgagcgcgccgcctgctgctcccttgcggcgggaaggacctcccgagtatttccggagagcacctgctttacgggatctccgccctttaacc

SEQ ID NO: 47 - DNA, 114 bp, Porcine reproductive and respiratory syndrome virus
tttgacagtcaggtgaatggccgcgattgacgtgtggcctctaagtcacctattcaattagggcgatcacatgggggtcaaacttaattaggcaggaaccatgtgaccgaaatt

SEQ ID NO: 48 - DNA, 14984 bp, Porcine reproductive and respiratory syndrome virus
atgatgtgtagggtattccccctacatacacgacactcttagtgtttgtgtaccttggaggcgtgggtacagccctgccccaccctttggtccctgttctagcccgacaggtacccttctctctcggggcgagcgcgccgcctgctgctcccttgcggcgggaaggacctcccgagtatttccggagagcacctgctttacgggatctccgccctttaaccatgtctgggatgttctcccggtgcatgtgcaccccggctgcccgggtattttggaacgccggccaagtctattgcacacggtgtctcagtgcacggtctcttctctctccagaacttcaggacacggacctcggtgcagttggcttgtttcacaagcctaaagacaagctccattggaaagttcccattggtatcccccaggtggaatgttctccatctgggtgttgctggctgtcaaccatttttcctttagcgcgcatgacctccggcaatcacaacttccttcaacgactcgtgaaggttgctgatgtattgtaccgtgacggttgcttaacccctagacacctccgtgaactccaagtttacgagcgtggttgcaattggtatccgattacggggcctgtgcctgggatggctgtgtacgcgaactccatgcacgtgtccgaccaaccgttccctggtgccactcatgtgttaacaaattcccctttgcctcaacgggcttgtcggcagccgttctgtccgttcgaagaggcccattctagcatatacaggtgggaaaaatttgtaatttttatggattcctcctccgacggtcgatctcgcatgatgtggactccggaatccgatgactccacggctttggaagttctgccgcccgagctagaacaccaggtcaaggtccttgttcggagctttcccgcccatcaccttgtcgaccttgccgattgggagctcactgagtcccctgataacggtttttccttcagcacgtcacatccttgcggctaccttgttcgggacccggctgtatccgaaggcaagtgttggctttcctgctttttgagccagtcagccgaagtgctcagtcgcgaggcgcatctggctaccgcctatggttaccaaaccaagtggggtgtgcctggcaagtacatccagcgcagacttcaagttcacggtctccgtgctgtggtcgaccctgatggtcccattcacgttgaagcattgtcttgcccccagtcttggatcaggcacttgaccctgaatgatgatgtcaccccgggattcgttcgcctaatgtctcttcgcattgtgccgaacacagagcctaccacacaccggatctttcgttttggagtgcacaagtggtatggtgccgccggcaaacgggcccgtggcaagcgtgccgccaaaagtgagaaagactcggcttccaccctcaaggttgcccgaccgacttccaccagtggaatcgtcacctactccccacctgcggacgggtcttgtggttggcatgcccttgccgccatactgaaccggatgattaataatgacttcacgtcccctctgcctcggtacaacaggccggaggacgattgggcttctgatggtgaccttgctcaggccattcaatgtttgcaactacctgccgccatagctcggaaccgcgcctgccctaacgccaaatacctcataaaactcaacggagttcattgggaggtagaggtgaggcctggaatggctcctcgctccctctctcgtgagtgcgttgttggcgtctgctctgaaggctgtgtcgcgtcgccttacccggaggacgggttgcctaaacgtgcacttgaggccctggcgtctgcttatagactgccttcagactgtgtttgtgatggtattattgacttccttgccaatccacctccccaggagttctggactcttgacaaaatgttgacttccccgtcaccggagcagtccggcttctctagtctgtataaattgttgttagagatcttgccgcagaaatgcggatccacagaaggggaattcatctatactgttgagaggatgttgaaggattgtccgagctccaaacaggccatggccctccttgcaaaaattaaggtcccatcctcaaaggccccatccgtgactctgaacgagtgcttccccacggatgttccagtcaactctgagttaatatcttgggaagagcccaaagaccctggcgctgctgttgtcctatgtccatcggatgcaaaagaatctaaggaaacagcccctgaagaagctcaagcgagaaaccgtaaggtccttcaccctgtggtccttaccgaggaacttagcgagcaacaggtgcaggtggttgagggtgatcaggatatgccactggatttgacttggccaaccttaaccgctacggcgacccctgttagagggccggtaccggacaatttgagctctggcattggtgcccagcccgctaccgttcaagaactcattctggcgaggcctgcaccccgtcttgttgagcgctgtggcacggagtcgaacggcagcagttcatttctggatttgcctgacgtgcagacctcggaccagcctttagacctgtccctggccgcgtggcctgtaagggctaccgcgtctgaccccggttggatccacggtaggcgtgagcctgtctttgtgaagcctcgaggtgttttctctgatggcgagtcggcccttcagttcggagagctttccgaagccagttctgtcgtcgatgaccggacaaaagaagctccggtggttgacgcccccatcgatttgacaacttcgaacgagacgctctctgggtctgacccctttgaattcgccaaattcaggcgcccgcgtttctccgcgcaagctttaatcgaccgaggtggtccgcttgccgatgttcatgcaaagataaagagtcgggtatatgaacaatgccttcaagcttgtgaacctggtagtcgtgcgaccccagccaccaagaagtggctcgacaaaatgtgggacagggtggacatgaaaacttggcgctgcacctcgcagttccaagctggtcacattcttgagtccctcaaattcctccctgacatgattcaagacacaccgcctcctgttcccaggaagaaccgagctggtgacagtgccggcctgaagcaactggtggcgcagtgggataggaaatcgagtgtgacaccccccacaaaaccggttggaccggtgcttgaccaggccgtccctctgcctatggacatccagcaaggagatgccatctccgctgacaagccaccccattcgcaaaacccttctagtcaagtagatgtgggtggaggttggaaaagttttatgctctccggcacccgtttcgcggggtccgttagtcagcgccttacgacatgggtttttgaggttctctcccatctcccagcttttatgctcacacttttctcgccacggggctctatggctccaggtgattggctgtttgcaggtgctgttctacttgctctcctgctctgccgttcttacccaatactcggatgccttcccttattgggtgtcttttctggttctgtgcggtgtgttcgtttgggtgtttttggttcttggatggcttttgctgtatttttattctcgactccacccgacccagtcggttcttcttgtgaccacgattcgccggagtgtcatgctgagcttttggctcttgagcagcgccaactttgggaacctgtgcgcagccttgtggtcgggccatcgggcctcttatgcgtcattcttggcaagttactcggtgggtcacgttgtctctggtttgttctcctacgtatatgcatgctcgcagatttggcaatttctcttatttatgtggtgtcccaagggcgttgtcacaagtgttggggaaagtgtataaggacggctcctgcagaagtggcccttaatgtgtttcctttttcgcgcgccacccgctcatctcttgtgtccttgtgtgatcggttccaagcgccaaaaggagttgaccccgtgcacttggcgacaggctggcgcgggtgctggtgtggtgagagccctattcatcaatcacaccaaaaaccgatagcttatgccaacttggatgaaaagaagatatccgcccagacggtgattgctgtcccgtatgatcctagtcaggccattaaatgcctgaaagttttgcaggcaggaggggctattgtggaccagcctacgcccgaggtcgtccgtgtgtctgagattcccttctcggccccattttttccgaaggtcccagtcaacccagactgcagggttgtggtagattcggacacttttgtggctgcggtccgctgcggttattcgacagcacaactggtccttggtcggggcaactttgccaagctaaatcagacccccctcaggaactctgtccccaccaaaacaactggtggggcctcatacacccttgccgtggcccaggtatctgtgtggactcttgttcatttcatcctcggcctttggttaacgtcacctcaagtgtgtggtcgagggacctctgacccgtggtgttcgaaccctttttcgtatcctacttatggccccggagttgtgtgttcctctcgactctgcgtgtctgccgacggagttaccctgccattgttctcagccgttgcccatctttccggtagagaggtggggatttttattttggtgcttgcctccttgggcgctttagcccaccgcttggctcttaaggcagacatgtcaatggtctttttggcgttttgtgcttacgcctggcccatgagctcctggttaatttgcttctttcctatgctcttgaggtgggtaacccttcatcctctcactatgctttgggtgcactcatttttggtgttttgcctaccagctgccggcgttctctcgctgggaataaccggtcttctttgggcagttggccgtttcacccaggttgccggaattatcacaccttatgacatccaccagtatacctccggaccacgtggtgcagctgctgtagcaacggctccagaaggtacttacatggcggccgttcggagagccgctttgactggacggactttgatcttcacaccatctgcagtcggatcccttcttgaaggtgctttcagaactcaaaagccctgccttaacaccgtgaatgtcgtaggctcttcccttggttctggaggagttttcaccattgatggcagaagagtcatcgtcactgccacccatgtgttgaatggtaacacagccagggtcactggtgattcctacaaccgcatgcacacgttcaatactaatggtgattatgcctggtcccatgctgatgactggcaaggcgttgcccctatggttaagatcgctaaggggtatcgcggtcgtgcctactggcaaacgtcaaccggagtcgaacctggcatcatgggggaaggattcgccttctgtttcactaactgtggcgactcagggtcacctgtcatttcagaagctggtgaccttattggagtccataccggttcaaacaaactcggttctggtcttgtgacaacccctgaaggggagacctgctccatcaaggaaactaggctctctgacctttctagacattttgcaggtccaagcgtccctcttggggacattaagttgagcccagccatcatccctgatgtgacaactattccgagtgacttggcatcgctccttgcttctgtccccgtgatggaaggtggcctctcaactgtccagcttttgtgcgtctttttccttctctggcgcatgatgggccatgcctggacacccattgttgccgtaggcttctttttgctgaatgaaattctcccagcagtcttggtccgagctgtgttctcttttgcactctttgtacttgcatgggccaccccctggtcggcacaagtgttgatgattagactcctcacggcggctctcaaccgcaacaggttgtccctggcgttctacgcattcggaggtgtcgttggcctggccacagaaatcgggacttttgctggtggatggcctgaactgtcccaagccctctcgacatactgcttcctgcccaggttccttgctgtgactagttatgtccccaccatcatcatcggtgggctccatgccctcggcgtaattttgtggttattcaaataccgatgcctccacaacatgctggttggtgatgggagtttctcaagcgctttcttcctacggtattttgctgagggtaatcttaggaaaggcgtgtcgcagtcctgtggcatgaataacgaatccctgacagctgctttggcttgcaagttgtcgcaagctgaccttgattttttgtccagtttaacgaacttcaagtgctttgtgtccgcttcaaacatgaaaaatgcagctggccaatacatcgaggcggcgtatgctagagctctgcgtcaggagctggcctccttggttcaggttgacaagatgaaaggagtattggccaagctcgaggctttcgctgagacggccactccgtcacttgacacaggggacgtgattgttctgcttgggcaacacccccatggatccatcctcgacattaatgtggggggtgaaaggaaaactgtgtctgtgcaagaaacacgatgcctgggtggttccaaattcagtgtctgcactgtcgtgtccaacacgcccgtggataccttgaccggtatcccacttcagacgccaaccccactttttgaaaatggcccgcgccatcgcagcgaggacgacgacctcaaagttgagagaatgaaaaaacactgtgtatccctcggcttccacaaaatcaatggtaaagtttactgcaaaatttgggacaagtctaacggcgacaccttttacacggatgattcccgatacactcaagaccatgcttttcaggacaggtcaaccgactatagagacagggattatgaaggtgtacagaccgccccccaacagggattcgatccaaagtccgaagcccctgttggcactgttgtaatcggtggcattacgtataacaggcatctggtcaaaggtaaggaggtcctagttcccaaacctgacaactgccttgaagctgccagactgtcccttgagcaagctcttgctgggatgggccaaacttgtgaccttacagctaccgaagtggagaaactaaagcgcatcattagtcaactccaaggtctgaccactgaacaggctttaaactgctagccgccagcggcttgacccgctgtggccgcggcggcctagttgtaactgaaacggcggtaaaaatcgtaaaataccacagcagaactttcaccttaggctctttagacctaaaagtcacctccgaggtggaggtgaagaaatcaactgagcaggggcacgctgtcgtggcgaacttatgttccggtgtcgtcttgatgaggcctcacccaccgtcccttgttgacgttctcctcaaacccggacttgacacaacacccggcattcaaccagggcatggggccgggaatatgggcgtgaacggttctatttgggattttgaaactgcacccacaaaggtagaactagagttgtccaagcaaataatccaagcatgtgaagtcaggcgcggggacgcccctaacctccaactcccctacaagctttatcctgtcaggggggaccccgagcggcgtaaaggtcgccttgtcaacactaggtttggagatttaccttacaaaactccccaagacaccaagtccgcaattcatgcggcttgttgcctgcatcccaatggggtcctcgtgtctgatggcaaatccacgctgggtaccactcttcaacatggtttcgagctttatgtccccactgtaccttatagtgtcatggaataccttgattcacgccctgacaccccttttatgtgtactaaacatggcacttccaaggctgctgcagaggacctccaaaaatatgacctatccactcaagggtttgtcttgcctggggtcctacgcctagtgcgcaggttcatctttagccatgttggtaaggcgccaccactgttccttccatcaacctaccctgccaagaactccatggcaggggtcaatggccagaggttcccaacaaaggatgtccagagcatacctgaaattgatgaaatgtgcgcccgtgccgtcaaggaaaattggcagactgtgacaccttgcaccctcaaaaaacagtactgttccaaacctaaaactagaaccatcctaggtaccaacaacttcatagccttggctcacaggtcagcactcagtggtgtcacccaggcgttcatgaagaaggcctggaagtccccaattgccttggggaaaaacaagtttaaggaattgcattgcactgtcgccggcagatgccttgaggctgacctggcttcctgcgatcgcagcacccccgccattgtgaggtggtttgttgccaacctcctgtatgaacttgcaggatgtgaagagtacttgcctagctacgtgctcaactgttgccatgaccttgtggcaacgcaggatggcgctttcacaaaacgcggtggcctgtcgtccggggaccccgtcaccagtgtgtccaacaccgtctactcactgataatttacgcccagcacatggtgctttcggccttgaagatgggtcatgaaattggtctcaagttccttgaggaacagctcaaatttgaggaccttcttgaaatccagcccatgttagtgtattctgatgacctcgtcttgtatgcggaaagacccacttttcccaactaccattggtgggtcgagcatcttgacctgatgttgggctttaaaacggacccaaagaaaactgtcataactgataaacccagttttctcggctgcagaattgaagcaggacggcagttagtccccaatcgcgaccgtattctggctgctcttgcatatcatatgaaggcgcagaacgcctcagagtattatgcgtccgctgccgcaattctgatggattcgtgtgcttgcattgaccatgaccccgagtggtatgaggatcttatctgcggcatcgcccggtgtgctcgccaggacggttaccgttttccaggcccggcatttttcatgtccatgtgggagaagctgaaaagtcataatgaagggaagaaatgccgtcactgcggcatctgcgacgccaaagccgactatgcgtccgcctgtggacttgatttgtgtttgttccattcacactttcatcaacactgcccagtcactctgagctgtggccaccatgccggttcaaaggaatgttcgcagtgtcagtcacctgtcggggctggcaaatccccccttgacgctgtgctgaaacaaatcccgtacaaacctcctcgtaccattatcatgaaggtggacaacaaaacaacgacccttgacccgggaagatatcagtcccgtcgaggtcttgttgcagtcaaaagaggtattgcaggtaatgaggttgatctttctgatggagactaccaagtggtgcctcttttgccgacttgcaaagacataaacatggtgaaggtggcttgcaacgtactactcagcaagtttatagtagggccgccaggttccggaaaaaccacctggctactgaaccaagtccaggacgatgatgtcatttacacacctactcatcagacaatgtttgacatagtcagtgctcttaaagtttgcaggtattccatcccaggagcctcaggactcccttttccaccacctgccaggtccgggccgtgggttaggctcatcgccagcggacatgtccctggccgagtgtcatatctcgatgaggcaggatattgcaatcatctagacattctaaggctgctttccaaaacaccccttgtgtgtttgggtgaccttcagcaacttcacccggtcggctttgattcctattgttatgtgttcgatcagatgcctcagaagcagctgaccaccatttatagatttggccctaacatctgtgcagccatccagccttgttacagggagaaacttgaatccaaggccaggaacaccagagtggttttcaccacccggcctgtggcctttggtcaggtcctgacaccgtaccacaaagatcgtaccggctctgcaataactatagattcatcccagggggcgaccttcgacattgtgacattgcatctaccatcgccaaagtccctaaacaaatcccgagcacttgtagccatcactcgggcaagacatgggttgttcatttatgaccctcatgaccaactccaggagtttttcaacttaacccccgagcgcactgattgtaaccttgcgttcagccgtggggatgagctggttgttttgaatgtggataatgcggtcacaactgtagcgaaggccctagagacaggttcaccccgatttcgagtatcggacccgaggtgcaagtctctcttagccgcttgttcggccagtctagaagggagctgcatgccactaccacaagtagcacataacctggggttttacttttccccggacagcccagcttttgcacccctgccaaaagagctggcgccacattggccagtggtcacccaccagaataatcgagcgtggcctgatcgacttgtcgctagtatgcgcccaattgatgcccgctacagcaagccaatggtcggtgcagggtatgtggtcgggccatccatttttcttggcactcctggtgtggtgtcatactatctcacattatacatcgggggcgagcctcaggccctgccagaaacactcgtttcaacaggacgtatagccacagattgtcgggaatatctcgacgcggctgaggaagaggcagcgagagaacttccccacgcatttattggcgatgtcaaaggcactacgatcggggggtgtcaccacattacatcgaaatacctacctaggtccctgcctaaagactctgttgctgtggttggggtgagttcgcccggtagggctgctaaagccgtgtgcactctcaccgatgtgtacctccccgaactccgaccatatttgcaaccggagacggcatcaaaatgctggaaacttaaactggatttcagggatgttcgactgatggtctggaaaggcgccacagcctatttccagttggaagggctgacatggtcagcgctgcccgattatgctaggttcattcagctacccaaggatgccgttgtgtacatcgatccgtgtatagggccggcaacagccaatcgcaaggttgtgcgaaccacagactggcgggccgacctggcagtgacaccgtatgattacggtgctcaggtcattttgacaacagcctggttcgaggaccttgggccgcagtggaagattttggggttgcagcctttcagacgaacatttggctttgagaacactgaagattgggcaattctcgcacgccgtatgaatgacggcaaagattacactgactataattggcattgtgtacgagaacgcccacacgcaatttacgggcgcgcccgtgaccatacgtatcattttgcccttggcactgaactgcaagtagagctgggcagaccccggctgcctcctgagcaagtgccgtgaacgcggagtgatgcaatgggtttactgtggagtaaaatcagtcagttgttcgtggatgccttcactgagttccttgttagtgtggttgacattgtcatctttctcgccatattgtttgggttcactgttgcaggctggttattggtcttccttctcagagtggtttgctccgcgtttctccgttcgcgctctgccattcactcttccgaactatcgaaggtcctatgagggcttgctacccaactgcagaccggatgtcccacaattcgcagttaagcacccgttgggtatactttggcatatgcgagtctcccacctaattgacgaaatggtctctcgccgcatttaccggaccatggaacattcgggtcaagcggcctggaagcaggttgttagtgaagccactctcacaaaactgtcaaggcttgacgtagtcactcatttccaacacctggccgcagtggaggctgattcttgccgcttccttagctcacgactcgcgatgctgaaaaaccttgccgttggcaatgtgagcctggagtacaacactactttggaccgcgttgagctcatctttcccacaccaggtacgaggcccaagttgaccgattttaggcaatggcttatcagcgtgcacgcttccatcttctcctctgtggcttcgtctgttaccttgttcacagtgctttggcttcgaattccagctctacgctatgtttttggtttccattggcccacggcaacacatcattcgaactaactatcaattacactatatgtaagccatgccctaccagtcaagctgcccaacaaagactcgagcctggccgtaacgtgtggtgcaaaatagggcacgacaggtgtgaggaacgtgaccatgatgagttgtcaatgtccattccgtccgggtacgacaacctcaaacttgagggttattatgcttggctggcttttttgtccttttcctacgcggcccaattccatccggagctgttcggaataggaaacgtgtcgcgcgtctttgtggataagcgacaccagttcatttgcgccgagcatgatggacaaaattcaaccatatctgccagacacaacatctccgcgtcgtatgcggtgtattaccatcatcaaatagacgggggcaattggtttcatttggaatggctgcgaccattcttttcctcctggctggtgctcaacatctcatggtttctgaggcgttcgcctgcaagccctgcttctcgacgcatctatcagatattaagaccaacacgaccgcggctgccggtttcatggtccttcagaacatcaattgtttccaatctcacagggcctcaacagcgcaaggtaccactcccctcaggaggtcgtcccaatgtcgtgaagccgtcggcattccccagtacatcacgataacggctaatgtgaccgatgaatcgtatttgtacaacgcggacttgctgatgctttccgcgtgccttttctacgcctcggaaatgagcgagaaaggcttcaaagtcatctttgggaatatttctggcgttgtttccgcttgtgttaatttcacagattatgtggcccatgtgacccaacacactcagcagcaccatttggtaattgatcacattcggttactacacttcttgacaccgtctacgatgaggtgggctacaaccattgcttgtttgcttgccattcttttggcggtatgaaatgttcttgcaagttggggcatttcttgactcctcactcttgcttctggtggctttttttgctgtgtaccggcttgtcttggtcctttgtcgatggcaacgacgacagctcgacatcccaatacatatataatttgacgatatgcgagctgaatgggaccgaatggttgtccggtcattttgattgggcagtcgaaacctttgtgctttacccagttgccactcatatcatttcactgggttttctcacaacaagccatttccttgatgcgctcggtctcggcgctgtgtccgccacaggattcattggcgagcggtatgtacttagcagcatgtacggcgtttgcgccttcgcggcgttcgtatgttttgtcatccgtgctgctaaaaattgcatggcttgccgctatgcccgcacccggtttaccaacttcatcgtggacgaccggggaagaatccatcgatggaagtcttcaatagtggtggagaaattgggcaaagctgaagtcggtggtgaccttgtcaacattaagcatgttgtcctcgaaggggttaaagctcaacctttgacgaggacttcggctgagcaatgggaagcctagacgacttttgcaacgatcccaccgccgcacaaaaactcgtgctggcctttagcatcacatatacacccataatgatatacgcccttaaggtgtcacgcggccgactcctggggctgttgcacatcttgatatttctgaattgttcctttacttttgggtacatgacatatgtgcattttcaatccaccaaccgtgtcgcattcactctgggggctgtagtcgcccttttgtggggtgtttacagcctcacagagtcatggaagttcatcacttccagatgcagattgtgttgcctaggccggcgatacattctggcccctgcccatcacgtagaaagtgctgcaggcctccattcaatcccagcgtctggtaaccgagcatacgctgtgagaaagcccggactaacatcagtgaacggcactctagtacctgggcttcggagcctcgtgctgggcggcaaacgagctgttaaacgaggagtggttaacctcgtcaagtatggccggtaagaaccagagccagaagaaaagaagaaatgcagctccgatggggaaaggccagccagtcaatcaactgtgccagttgctgggtacaatgataaagtcccagcgccagcaatctaggggaggacaggccaaaaagaagaagcctgagaagccacattttcccctagctgctgaagatgacattcggcaccatctcacccaggccgaacgttccctctgcttgcaatcgatccagacggctttcaatcaaggcgcaggaactgcgtcgctttcatccagcgggaaggtcagtttccaggttgagttcatgctgccggttgctcatacagtgcgcctgattcgcgtgacttctacatccgccagtcagggtgcaaattaatttgacagtcaggtgaatggccgcgattgacgtgtggcctctaagtcacctattcaattagggcgatcacatgggggtcaaacttaattaggcaggaaccatgtgaccgaaattaaaaaaaaaaaaaaaaaaaaaaaaaaa

SEQ ID NO: 49 - DNA, 14945 bp, Porcine reproductive and respiratory syndrome virus
atgatgtgtagggtattccccctacatacacgacactcttagtgtttgtgtaccttggaggcgtgggtacagccctgccccaccctttggtccctgttctagcccgacaggtacccttctctctcggggcgagcgcgccgcctgctgctcccttgcggcgggaaggacctcccgagtatttccggagagcacctgctttacgggatctccgccctttaaccatgtctgggatgttctcccggtgcatgtgcaccccggctgcccgggtattttggaacgccggccaagtctattgcacacggtgtctcagtgcacggtctcttctctctccagaacttcaggacacggacctcggtgcagttggcttgtttcacaagcctaaagacaagctccattggaaagttcccattggtatcccccaggtggaatgttctccatctgggtgttgctggctgtcaaccatttttcctttagcgcgcatgacctccggcaatcacaacttccttcaacgactcgtgaaggttgctgatgtattgtaccgtgacggttgcttaacccctagacacctccgtgaactccaagtttacgagcgtggttgcaattggtatccgattacggggcctgtgcctgggatggctgtgtacgcgaactccatgcacgtgtccgaccaaccgttccctggtgccactcatgtgttaacaaattcccctttgcctcaacgggcttgtcggcagccgttctgtccgttcgaagaggcccattctagcatatacaggtgggaaaaatttgtaatttttatggattcctcctccgacggtcgatctcgcatgatgtggactccggaatccgatgactccacggctttggaagttctgccgcccgagctagaacaccaggtcaaggtccttgttcggagctttcccgcccatcaccttgtcgaccttgccgattgggagctcactgagtcccctgataacggtttttccttcagcacgtcacatccttgcggctaccttgttcgggacccggctgtatccgaaggcaagtgttggctttcctgctttttgagccagtcagccgaagtgctcagtcgcgaggcgcatctggctaccgcctatggttaccaaaccaagtggggtgtgcctggcaagtacatccagcgcagacttcaagttcacggtctccgtgctgtggtcgaccctgatggtcccattcacgttgaagcattgtcttgcccccagtcttggatcaggcacttgaccctgaatgatgatgtcaccccgggattcgttcgcctaatgtctcttcgcattgtgccgaacacagagcctaccacacaccggatctttcgttttggagtgcacaagtggtatggtgccgccggcaaacgggcccgtggcaagcgtgccgccaaaagtgagaaagactcggcttccaccctcaaggttgcccgaccgacttccaccagtggaatcgtcacctactccccacctgcggacgggtcttgtggttggcatgcccttgccgccatactgaaccggatgattaataatgacttcacgtcccctctgcctcggtacaacaggccggaggacgattgggcttctgatggtgaccttgctcaggccattcaatgtttgcaactacctgccgccatagctcggaaccgcgcctgccctaacgccaaatacctcataaaactcaacggagttcattgggaggtagaggtgaggcctggaatggctcctcgctccctctctcgtgagtgcgttgttggcgtctgctctgaaggctgtgtcgcgtcgccttacccggaggacgggttgcctaaacgtgcacttgaggccctggcgtctgcttatagactgccttcagactgtgtttgtgatggtattattgacttccttgccaatccacctccccaggagttctggactcttgacaaaatgttgacttccccgtcaccggagcagtccggcttctctagtctgtataaattgttgttagagatcttgccgcagaaatgcggatccacagaaggggaattcatctatactgttgagaggatgttgaaggattgtccgagctccaaacaggccatggccctccttgcaaaaattaaggtcccatcctcaaaggccccatccgtgactctgaacgagtgcttccccacggatgttccagtcaactctgagttaatatcttgggaagagcccaaagaccctggcgctgctgttgtcctatgtccatcggatgcaaaagaatctaaggaaacagcccctgaagaagctcaagcgagaaaccgtaaggtccttcaccctgtggtccttaccgaggaacttagcgagcaacaggtgcaggtggttgagggtgatcaggatatgccactggatttgacttggccaaccttaaccgctacggcgacccctgttagagggccggtaccggacaatttgagctctggcattggtgcccagcccgctaccgttcaagaactcattctggcgaggcctgcaccccgtcttgttgagcgctgtggcacggagtcgaacggcagcagttcatttctggatttgcctgacgtgcagacctcggaccagcctttagacctgtccctggccgcgtggcctgtaagggctaccgcgtctgaccccggttggatccacggtaggcgtgagcctgtctttgtgaagcctcgaggtgttttctctgatggcgagtcggcccttcagttcggagagctttccgaagccagttctgtcgtcgatgaccggacaaaagaagctccggtggttgacgcccccatcgatttgacaacttcgaacgagacgctctctgggtctgacccctttgaattcgccaaattcaggcgcccgcgtttctccgcgcaagctttaatcgaccgaggtggtccgcttgccgatgttcatgcaaagataaagagtcgggtatatgaacaatgccttcaagcttgtgaacctggtagtcgtgcgaccccagccaccaagaagtggctcgacaaaatgtgggacagggtggacatgaaaacttggcgctgcacctcgcagttccaagctggtcacattcttgagtccctcaaattcctccctgacatgattcaagacacaccgcctcctgttcccaggaagaaccgagctggtgacagtgccggcctgaagcaactggtggcgcagtgggataggaaatcgagtgtgacaccccccacaaaaccggttggaccggtgcttgaccaggccgtccctctgcctatggacatccagcaaggagatgccatctccgctgacaagccaccccattcgcaaaacccttctagtcaagtagatgtgggtggaggttggaaaagttttatgctctccggcacccgtttcgcggggtccgttagtcagcgccttacgacatgggtttttgaggttctctcccatctcccagcttttatgctcacacttttctcgccacggggctctatggctccaggtgattggctgtttgcaggtgctgttctacttgctctcctgctctgccgttcttacccaatactcggatgccttcccttattgggtgtcttttctggttctgtgcggtgtgttcgtttgggtgtttttggttcttggatggcttttgctgtatttttattctcgactccacccgacccagtcggttcttcttgtgaccacgattcgccggagtgtcatgctgagcttttggctcttgagcagcgccaactttgggaacctgtgcgcagccttgtggtcgggccatcgggcctcttatgcgtcattcttggcaagttactcggtgggtcacgttgtctctggtttgttctcctacgtatatgcatgctcgcagatttggcaatttctcttatttatgtggtgtcccaagggcgttgtcacaagtgttggggaaagtgtataaggacggctcctgcagaagtggcccttaatgtgtttcctttttcgcgcgccacccgctcatctcttgtgtccttgtgtgatcggttccaagcgccaaaaggagttgaccccgtgcacttggcgacaggctggcgcgggtgctggtgtggtgagagccctattcatcaatcacaccaaaaaccgatagcttatgccaacttggatgaaaagaagatatccgcccagacggtgattgctgtcccgtatgatcctagtcaggccattaaatgcctgaaagttttgcaggcaggaggggctattgtggaccagcctacgcccgaggtcgtccgtgtgtctgagattcccttctcggccccattttttccgaaggtcccagtcaacccagactgcagggttgtggtagattcggacacttttgtggctgcggtccgctgcggttattcgacagcacaactggtccttggtcggggcaactttgccaagctaaatcagacccccctcaggaactctgtccccaccaaaacaactggtggggcctcatacacccttgccgtggcccaggtatctgtgtggactcttgttcatttcatcctcggcctttggttaacgtcacctcaagtgtgtggtcgagggacctctgacccgtggtgttcgaaccctttttcgtatcctacttatggccccggagttgtgtgttcctctcgactctgcgtgtctgccgacggagttaccctgccattgttctcagccgttgcccatctttccggtagagaggtggggatttttattttggtgcttgcctccttgggcgctttagcccaccgcttggctcttaaggcagacatgtcaatggtctttttggcgttttgtgcttacgcctggcccatgagctcctggttaatttgcttctttcctatgctcttgaggtgggtaacccttcatcctctcactatgctttgggtgcactcatttttggtgttttgcctaccagctgccggcgttctctcgctgggaataaccggtcttctttgggcagttggccgtttcacccaggttgccggaattatcacaccttatgacatccaccagtatacctccggaccacgtggtgcagctgctgtagcaacggctccagaaggtacttacatggcggccgttcggagagccgctttgactggacggactttgatcttcacaccatctgcagtcggatcccttcttgaaggtgctttcagaactcaaaagccctgccttaacaccgtgaatgtcgtaggctcttcccttggttctggaggagttttcaccattgatggcagaagagtcatcgtcactgccacccatgtgttgaatggtaacacagccagggtcactggtgattcctacaaccgcatgcacacgttcaatactaatggtgattatgcctggtcccatgctgatgactggcaaggcgttgcccctatggttaagatcgctaaggggtatcgcggtcgtgcctactggcaaacgtcaaccggagtcgaacctggcatcatgggggaaggattcgccttctgtttcactaactgtggcgactcagggtcacctgtcatttcagaagctggtgaccttattggagtccataccggttcaaacaaactcggttctggtcttgtgacaacccctgaaggggagacctgctccatcaaggaaactaggctctctgacctttctagacattttgcaggtccaagcgtccctcttggggacattaagttgagcccagccatcatccctgatgtgacaactattccgagtgacttggcatcgctccttgcttctgtccccgtgatggaaggtggcctctcaactgtccagcttttgtgcgtctttttccttctctggcgcatgatgggccatgcctggacacccattgttgccgtaggcttctttttgctgaatgaaattctcccagcagtcttggtccgagctgtgttctcttttgcactctttgtacttgcatgggccaccccctggtcggcacaagtgttgatgattagactcctcacggcggctctcaaccgcaacaggttgtccctggcgttctacgcattcggaggtgtcgttggcctggccacagaaatcgggacttttgctggtggatggcctgaactgtcccaagccctctcgacatactgcttcctgcccaggttccttgctgtgactagttatgtccccaccatcatcatcggtgggctccatgccctcggcgtaattttgtggttattcaaataccgatgcctccacaacatgctggttggtgatgggagtttctcaagcgctttcttcctacggtattttgctgagggtaatcttaggaaaggcgtgtcgcagtcctgtggcatgaataacgaatccctgacagctgctttggcttgcaagttgtcgcaagctgaccttgattttttgtccagtttaacgaacttcaagtgctttgtgtccgcttcaaacatgaaaaatgcagctggccaatacatcgaggcggcgtatgctagagctctgcgtcaggagctggcctccttggttcaggttgacaagatgaaaggagtattggccaagctcgaggctttcgctgagacggccactccgtcacttgacacaggggacgtgattgttctgcttgggcaacacccccatggatccatcctcgacattaatgtggggggtgaaaggaaaactgtgtctgtgcaagaaacacgatgcctgggtggttccaaattcagtgtctgcactgtcgtgtccaacacgcccgtggataccttgaccggtatcccacttcagacgccaaccccactttttgaaaatggcccgcgccatcgcagcgaggacgacgacctcaaagttgagagaatgaaaaaacactgtgtatccctcggcttccacaaaatcaatggtaaagtttactgcaaaatttgggacaagtctaacggcgacaccttttacacggatgattcccgatacactcaagaccatgcttttcaggacaggtcaaccgactatagagacagggattatgaaggtgtacagaccgccccccaacagggattcgatccaaagtccgaagcccctgttggcactgttgtaatcggtggcattacgtataacaggcatctggtcaaaggtaaggaggtcctagttcccaaacctgacaactgccttgaagctgccagactgtcccttgagcaagctcttgctgggatgggccaaacttgtgaccttacagctaccgaagtggagaaactaaagcgcatcattagtcaactccaaggtctgaccactgaacaggctttaaactgctagccgccagcggcttgacccgctgtggccgcggcggcctagttgtaactgaaacggcggtaaaaatcgtaaaataccacagcagaactttcaccttaggctctttagacctaaaagtcacctccgaggtggaggtgaagaaatcaactgagcaggggcacgctgtcgtggcgaacttatgttccggtgtcgtcttgatgaggcctcacccaccgtcccttgttgacgttctcctcaaacccggacttgacacaacacccggcattcaaccagggcatggggccgggaatatgggcgtgaacggttctatttgggattttgaaactgcacccacaaaggtagaactagagttgtccaagcaaataatccaagcatgtgaagtcaggcgcggggacgcccctaacctccaactcccctacaagctttatcctgtcaggggggaccccgagcggcgtaaaggtcgccttgtcaacactaggtttggagatttaccttacaaaactccccaagacaccaagtccgcaattcatgcggcttgttgcctgcatcccaatggggtcctcgtgtctgatggcaaatccacgctgggtaccactcttcaacatggtttcgagctttatgtccccactgtaccttatagtgtcatggaataccttgattcacgccctgacaccccttttatgtgtactaaacatggcacttccaaggctgctgcagaggacctccaaaaatatgacctatccactcaagggtttgtcttgcctggggtcctacgcctagtgcgcaggttcatctttagccatgttggtaaggcgccaccactgttccttccatcaacctaccctgccaagaactccatggcaggggtcaatggccagaggttcccaacaaaggatgtccagagcatacctgaaattgatgaaatgtgcgcccgtgccgtcaaggaaaattggcagactgtgacaccttgcaccctcaaaaaacagtactgttccaaacctaaaactagaaccatcctaggtaccaacaacttcatagccttggctcacaggtcagcactcagtggtgtcacccaggcgttcatgaagaaggcctggaagtccccaattgccttggggaaaaacaagtttaaggaattgcattgcactgtcgccggcagatgccttgaggctgacctggcttcctgcgatcgcagcacccccgccattgtgaggtggtttgttgccaacctcctgtatgaacttgcaggatgtgaagagtacttgcctagctacgtgctcaactgttgccatgaccttgtggcaacgcaggatggcgctttcacaaaacgcggtggcctgtcgtccggggaccccgtcaccagtgtgtccaacaccgtctactcactgataatttacgcccagcacatggtgctttcggccttgaagatgggtcatgaaattggtctcaagttccttgaggaacagctcaaatttgaggaccttcttgaaatccagcccatgttagtgtattctgatgacctcgtcttgtatgcggaaagacccacttttcccaactaccattggtgggtcgagcatcttgacctgatgttgggctttaaaacggacccaaagaaaactgtcataactgataaacccagttttctcggctgcagaattgaagcaggacggcagttagtccccaatcgcgaccgtattctggctgctcttgcatatcatatgaaggcgcagaacgcctcagagtattatgcgtccgctgccgcaattctgatggattcgtgtgcttgcattgaccatgaccccgagtggtatgaggatcttatctgcggcatcgcccggtgtgctcgccaggacggttaccgttttccaggcccggcatttttcatgtccatgtgggagaagctgaaaagtcataatgaagggaagaaatgccgtcactgcggcatctgcgacgccaaagccgactatgcgtccgcctgtggacttgatttgtgtttgttccattcacactttcatcaacactgcccagtcactctgagctgtggccaccatgccggttcaaaggaatgttcgcagtgtcagtcacctgtcggggctggcaaatccccccttgacgctgtgctgaaacaaatcccgtacaaacctcctcgtaccattatcatgaaggtggacaacaaaacaacgacccttgacccgggaagatatcagtcccgtcgaggtcttgttgcagtcaaaagaggtattgcaggtaatgaggttgatctttctgatggagactaccaagtggtgcctcttttgccgacttgcaaagacataaacatggtgaaggtggcttgcaacgtactactcagcaagtttatagtagggccgccaggttccggaaaaaccacctggctactgaaccaagtccaggacgatgatgtcatttacacacctactcatcagacaatgtttgacatagtcagtgctcttaaagtttgcaggtattccatcccaggagcctcaggactcccttttccaccacctgccaggtccgggccgtgggttaggctcatcgccagcggacatgtccctggccgagtgtcatatctcgatgaggcaggatattgcaatcatctagacattctaaggctgctttccaaaacaccccttgtgtgtttgggtgaccttcagcaacttcacccggtcggctttgattcctattgttatgtgttcgatcagatgcctcagaagcagctgaccaccatttatagatttggccctaacatctgtgcagccatccagccttgttacagggagaaacttgaatccaaggccaggaacaccagagtggttttcaccacccggcctgtggcctttggtcaggtcctgacaccgtaccacaaagatcgtaccggctctgcaataactatagattcatcccagggggcgaccttcgacattgtgacattgcatctaccatcgccaaagtccctaaacaaatcccgagcacttgtagccatcactcgggcaagacatgggttgttcatttatgaccctcatgaccaactccaggagtttttcaacttaacccccgagcgcactgattgtaaccttgcgttcagccgtggggatgagctggttgttttgaatgtggataatgcggtcacaactgtagcgaaggccctagagacaggttcaccccgatttcgagtatcggacccgaggtgcaagtctctcttagccgcttgttcggccagtctagaagggagctgcatgccactaccacaagtagcacataacctggggttttacttttccccggacagcccagcttttgcacccctgccaaaagagctggcgccacattggccagtggtcacccaccagaataatcgagcgtggcctgatcgacttgtcgctagtatgcgcccaattgatgcccgctacagcaagccaatggtcggtgcagggtatgtggtcgggccatccatttttcttggcactcctggtgtggtgtcatactatctcacattatacatcgggggcgagcctcaggccctgccagaaacactcgtttcaacaggacgtatagccacagattgtcgggaatatctcgacgcggctgaggaagaggcagcgagagaacttccccacgcatttattggcgatgtcaaaggcactacgatcggggggtgtcaccacattacatcgaaatacctacctaggtccctgcctaaagactctgttgctgtggttggggtgagttcgcccggtagggctgctaaagccgtgtgcactctcaccgatgtgtacctccccgaactccgaccatatttgcaaccggagacggcatcaaaatgctggaaacttaaactggatttcagggatgttcgactgatggtctggaaaggcgccacagcctatttccagttggaagggctgacatggtcagcgctgcccgattatgctaggttcattcagctacccaaggatgccgttgtgtacatcgatccgtgtatagggccggcaacagccaatcgcaaggttgtgcgaaccacagactggcgggccgacctggcagtgacaccgtatgattacggtgctcaggtcattttgacaacagcctggttcgaggaccttgggccgcagtggaagattttggggttgcagcctttcagacgaacatttggctttgagaacactgaagattgggcaattctcgcacgccgtatgaatgacggcaaagattacactgactataattggcattgtgtacgagaacgcccacacgcaatttacgggcgcgcccgtgaccatacgtatcattttgcccttggcactgaactgcaagtagagctgggcagaccccggctgcctcctgagcaagtgccgtgaacgcggagtgatgcaatgggtttactgtggagtaaaatcagtcagttgttcgtggatgccttcactgagttccttgttagtgtggttgacattgtcatctttctcgccatattgtttgggttcactgttgcaggctggttattggtcttccttctcagagtggtttgctccgcgtttctccgttcgcgctctgccattcactcttccgaactatcgaaggtcctatgagggcttgctacccaactgcagaccggatgtcccacaattcgcagttaagcacccgttgggtatactttggcatatgcgagtctcccacctaattgacgaaatggtctctcgccgcatttaccggaccatggaacattcgggtcaagcggcctggaagcaggttgttagtgaagccactctcacaaaactgtcaaggcttgacgtagtcactcatttccaacacctggccgcagtggaggctgattcttgccgcttccttagctcacgactcgcgatgctgaaaaaccttgccgttggcaatgtgagcctggagtacaacactactttggaccgcgttgagctcatctttcccacaccaggtacgaggcccaagttgaccgattttaggcaatggcttatcagcgtgcacgcttccatcttctcctctgtggcttcgtctgttaccttgttcacagtgctttggcttcgaattccagctctacgctatgtttttggtttccattggcccacggcaacacatcattcgaactaactatcaattacactatatgtaagccatgccctaccagtcaagctgcccaacaaagactcgagcctggccgtaacgtgtggtgcaaaatagggcacgacaggtgtgaggaacgtgaccatgatgagttgtcaatgtccattccgtccgggtacgacaacctcaaacttgagggttattatgcttggctggcttttttgtccttttcctacgcggcccaattccatccggagctgttcggaataggaaacgtgtcgcgcgtctttgtggataagcgacaccagttcatttgcgccgagcatgatggacaaaattcaaccatatctgccagacacaacatctccgcgtcgtatgcggtgtattaccatcatcaaatagacgggggcaattggtttcatttggaatggctgcgaccattcttttcctcctggctggtgctcaacatctcatggtttctgaggcgttcgcctgcaagccctgcttctcgacgcatctatcagatattaagaccaacacgaccgcggctgccggtttcatggtccttcagaacatcaattgtttccaatctcactcgtcccaatgtcgtgaagccgtcggcattccccagtacatcacgataacggctaatgtgaccgatgaatcgtatttgtacaacgcggacttgctgatgctttccgcgtgccttttctacgcctcggaaatgagcgagaaaggcttcaaagtcatctttgggaatatttctggcgttgtttccgcttgtgttaatttcacagattatgtggcccatgtgacccaacacactcagcagcaccatttggtaattgatcacattcggttactacacttcttgacaccgtctacgatgaggtgggctacaaccattgcttgtttgcttgccattcttttggcggtatgaaatgttcttgcaagttggggcatttcttgactcctcactcttgcttctggtggctttttttgctgtgtaccggcttgtcttggtcctttgtcgatggcaacgacgacagctcgacatcccaatacatatataatttgacgatatgcgagctgaatgggaccgaatggttgtccggtcattttgattgggcagtcgaaacctttgtgctttacccagttgccactcatatcatttcactgggttttctcacaacaagccatttccttgatgcgctcggtctcggcgctgtgtccgccacaggattcattggcgagcggtatgtacttagcagcatgtacggcgtttgcgccttcgcggcgttcgtatgttttgtcatccgtgctgctaaaaattgcatggcttgccgctatgcccgcacccggtttaccaacttcatcgtggacgaccggggaagaatccatcgatggaagtcttcaatagtggtggagaaattgggcaaagctgaagtcggtggtgaccttgtcaacattaagcatgttgtcctcgaaggggttaaagctcaacctttgacgaggacttcggctgagcaatgggaagcctagacgacttttgcaacgatcccaccgccgcacaaaaactcgtgctggcctttagcatcacatatacacccataatgatatacgcccttaaggtgtcacgcggccgactcctggggctgttgcacatcttgatatttctgaattgttcctttacttttgggtacatgacatatgtgcattttcaatccaccaaccgtgtcgcattcactctgggggctgtagtcgcccttttgtggggtgtttacagcctcacagagtcatggaagttcatcacttccagatgcagattgtgttgcctaggccggcgatacattctggcccctgcccatcacgtagaaagtgctgcaggcctccattcaatcccagcgtctggtaaccgagcatacgctgtgagaaagcccggactaacatcagtgaacggcactctagtacctgggcttcggagcctcgtgctgggcggcaaacgagctgttaaacgaggagtggttaacctcgtcaagtatggccggtaagaaccagagccagaagaaaagaagaaatgcagctccgatggggaaaggccagccagtcaatcaactgtgccagttgctgggtacaatgataaagtcccagcgccagcaatctaggggaggacaggccaaaaagaagaagcctgagaagccacattttcccctagctgctgaagatgacattcggcaccatctcacccaggccgaacgttccctctgcttgcaatcgatccagacggctttcaatcaaggcgcaggaactgcgtcgctttcatccagcgggaaggtcagtttccaggttgagttcatgctgccggttgctcatacagtgcgcctgattcgcgtgacttctacatccgccagtcagggtgcaaattaatttgacagtcaggtgaatggccgcgattgacgtgtggcctctaagtcacctattcaattagggcgatcacatgggggtcaaacttaattaggcaggaaccatgtgaccgaaattaaaaaaaaaaaaaaaaaaaaaaaaaaa

SEQ ID NO: 50 - protein, 17 aa, Artificial Sequence
  SEQ ID NO:39 with substitution N->Q at position 9
SSHLQLIYQLTICELNG

SEQ ID NO: 51 - protein, 11 aa, Porcine reproductive and respiratory syndrome virus
SSHLQLIYNLT

SEQ ID NO: 52 - protein, 11 aa, Artificial Sequence
  SEQ ID NO:51 with substitution N->Q at position 9
SSHLQLIYQLT

SEQ ID NO: 53 - protein, 13 aa, Artificial Sequence
  SEQ ID NO:51 with Gly-Gly linker
GSSHLQLIYNLTG

SEQ ID NO: 54 - protein, 13 aa, Artificial Sequence
  SEQ ID NO:52 with Gly-Gly linker
GSSHLQLIYQLTG

SEQ ID NO: 55 - protein, 14 aa, Artificial Sequence
  SEQ ID NO:53 with N-terminal P
PGSSHLQLIYNLTG

SEQ ID NO: 56 - DNA, 14984 bp, Artificial Sequence
  SEQ ID NO:49 with insert coding for SEQ ID NO:53
atgatgtgtagggtattccccctacatacacgacactcttagtgtttgtgtaccttggaggcgtgggtacagccctgccccaccctttggtccctgttctagcccgacaggtacccttctctctcggggcgagcgcgccgcctgctgctcccttgcggcgggaaggacctcccgagtatttccggagagcacctgctttacgggatctccgccctttaaccatgtctgggatgttctcccggtgcatgtgcaccccggctgcccgggtattttggaacgccggccaagtctattgcacacggtgtctcagtgcacggtctcttctctctccagaacttcaggacacggacctcggtgcagttggcttgtttcacaagcctaaagacaagctccattggaaagttcccattggtatcccccaggtggaatgttctccatctgggtgttgctggctgtcaaccatttttcctttagcgcgcatgacctccggcaatcacaacttccttcaacgactcgtgaaggttgctgatgtattgtaccgtgacggttgcttaacccctagacacctccgtgaactccaagtttacgagcgtggttgcaattggtatccgattacggggcctgtgcctgggatggctgtgtacgcgaactccatgcacgtgtccgaccaaccgttccctggtgccactcatgtgttaacaaattcccctttgcctcaacgggcttgtcggcagccgttctgtccgttcgaagaggcccattctagcatatacaggtgggaaaaatttgtaatttttatggattcctcctccgacggtcgatctcgcatgatgtggactccggaatccgatgactccacggctttggaagttctgccgcccgagctagaacaccaggtcaaggtccttgttcggagctttcccgcccatcaccttgtcgaccttgccgattgggagctcactgagtcccctgataacggtttttccttcagcacgtcacatccttgcggctaccttgttcgggacccggctgtatccgaaggcaagtgttggctttcctgctttttgagccagtcagccgaagtgctcagtcgcgaggcgcatctggctaccgcctatggttaccaaaccaagtggggtgtgcctggcaagtacatccagcgcagacttcaagttcacggtctccgtgctgtggtcgaccctgatggtcccattcacgttgaagcattgtcttgcccccagtcttggatcaggcacttgaccctgaatgatgatgtcaccccgggattcgttcgcctaatgtctcttcgcattgtgccgaacacagagcctaccacacaccggatctttcgttttggagtgcacaagtggtatggtgccgccggcaaacgggcccgtggcaagcgtgccgccaaaagtgagaaagactcggcttccaccctcaaggttgcccgaccgacttccaccagtggaatcgtcacctactccccacctgcggacgggtcttgtggttggcatgcccttgccgccatactgaaccggatgattaataatgacttcacgtcccctctgcctcggtacaacaggccggaggacgattgggcttctgatggtgaccttgctcaggccattcaatgtttgcaactacctgccgccatagctcggaaccgcgcctgccctaacgccaaatacctcataaaactcaacggagttcattgggaggtagaggtgaggcctggaatggctcctcgctccctctctcgtgagtgcgttgttggcgtctgctctgaaggctgtgtcgcgtcgccttacccggaggacgggttgcctaaacgtgcacttgaggccctggcgtctgcttatagactgccttcagactgtgtttgtgatggtattattgacttccttgccaatccacctccccaggagttctggactcttgacaaaatgttgacttccccgtcaccggagcagtccggcttctctagtctgtataaattgttgttagagatcttgccgcagaaatgcggatccacagaaggggaattcatctatactgttgagaggatgttgaaggattgtccgagctccaaacaggccatggccctccttgcaaaaattaaggtcccatcctcaaaggccccatccgtgactctgaacgagtgcttccccacggatgttccagtcaactctgagttaatatcttgggaagagcccaaagaccctggcgctgctgttgtcctatgtccatcggatgcaaaagaatctaaggaaacagcccctgaagaagctcaagcgagaaaccgtaaggtccttcaccctgtggtccttaccgaggaacttagcgagcaacaggtgcaggtggttgagggtgatcaggatatgccactggatttgacttggccaaccttaaccgctacggcgacccctgttagagggccggtaccggacaatttgagctctggcattggtgcccagcccgctaccgttcaagaactcattctggcgaggcctgcaccccgtcttgttgagcgctgtggcacggagtcgaacggcagcagttcatttctggatttgcctgacgtgcagacctcggaccagcctttagacctgtccctggccgcgtggcctgtaagggctaccgcgtctgaccccggttggatccacggtaggcgtgagcctgtctttgtgaagcctcgaggtgttttctctgatggcgagtcggcccttcagttcggagagctttccgaagccagttctgtcgtcgatgaccggacaaaagaagctccggtggttgacgcccccatcgatttgacaacttcgaacgagacgctctctgggtctgacccctttgaattcgccaaattcaggcgcccgcgtttctccgcgcaagctttaatcgaccgaggtggtccgcttgccgatgttcatgcaaagataaagagtcgggtatatgaacaatgccttcaagcttgtgaacctggtagtcgtgcgaccccagccaccaagaagtggctcgacaaaatgtgggacagggtggacatgaaaacttggcgctgcacctcgcagttccaagctggtcacattcttgagtccctcaaattcctccctgacatgattcaagacacaccgcctcctgttcccaggaagaaccgagctggtgacagtgccggcctgaagcaactggtggcgcagtgggataggaaatcgagtgtgacaccccccacaaaaccggttggaccggtgcttgaccaggccgtccctctgcctatggacatccagcaaggagatgccatctccgctgacaagccaccccattcgcaaaacccttctagtcaagtagatgtgggtggaggttggaaaagttttatgctctccggcacccgtttcgcggggtccgttagtcagcgccttacgacatgggtttttgaggttctctcccatctcccagcttttatgctcacacttttctcgccacggggctctatggctccaggtgattggctgtttgcaggtgctgttctacttgctctcctgctctgccgttcttacccaatactcggatgccttcccttattgggtgtcttttctggttctgtgcggtgtgttcgtttgggtgtttttggttcttggatggcttttgctgtatttttattctcgactccacccgacccagtcggttcttcttgtgaccacgattcgccggagtgtcatgctgagcttttggctcttgagcagcgccaactttgggaacctgtgcgcagccttgtggtcgggccatcgggcctcttatgcgtcattcttggcaagttactcggtgggtcacgttgtctctggtttgttctcctacgtatatgcatgctcgcagatttggcaatttctcttatttatgtggtgtcccaagggcgttgtcacaagtgttggggaaagtgtataaggacggctcctgcagaagtggcccttaatgtgtttcctttttcgcgcgccacccgctcatctcttgtgtccttgtgtgatcggttccaagcgccaaaaggagttgaccccgtgcacttggcgacaggctggcgcgggtgctggtgtggtgagagccctattcatcaatcacaccaaaaaccgatagcttatgccaacttggatgaaaagaagatatccgcccagacggtgattgctgtcccgtatgatcctagtcaggccattaaatgcctgaaagttttgcaggcaggaggggctattgtggaccagcctacgcccgaggtcgtccgtgtgtctgagattcccttctcggccccattttttccgaaggtcccagtcaacccagactgcagggttgtggtagattcggacacttttgtggctgcggtccgctgcggttattcgacagcacaactggtccttggtcggggcaactttgccaagctaaatcagacccccctcaggaactctgtccccaccaaaacaactggtggggcctcatacacccttgccgtggcccaggtatctgtgtggactcttgttcatttcatcctcggcctttggttaacgtcacctcaagtgtgtggtcgagggacctctgacccgtggtgttcgaaccctttttcgtatcctacttatggccccggagttgtgtgttcctctcgactctgcgtgtctgccgacggagttaccctgccattgttctcagccgttgcccatctttccggtagagaggtggggatttttattttggtgcttgcctccttgggcgctttagcccaccgcttggctcttaaggcagacatgtcaatggtctttttggcgttttgtgcttacgcctggcccatgagctcctggttaatttgcttctttcctatgctcttgaggtgggtaacccttcatcctctcactatgctttgggtgcactcatttttggtgttttgcctaccagctgccggcgttctctcgctgggaataaccggtcttctttgggcagttggccgtttcacccaggttgccggaattatcacaccttatgacatccaccagtatacctccggaccacgtggtgcagctgctgtagcaacggctccagaaggtacttacatggcggccgttcggagagccgctttgactggacggactttgatcttcacaccatctgcagtcggatcccttcttgaaggtgctttcagaactcaaaagccctgccttaacaccgtgaatgtcgtaggctcttcccttggttctggaggagttttcaccattgatggcagaagagtcatcgtcactgccacccatgtgttgaatggtaacacagccagggtcactggtgattcctacaaccgcatgcacacgttcaatactaatggtgattatgcctggtcccatgctgatgactggcaaggcgttgcccctatggttaagatcgctaaggggtatcgcggtcgtgcctactggcaaacgtcaaccggagtcgaacctggcatcatgggggaaggattcgccttctgtttcactaactgtggcgactcagggtcacctgtcatttcagaagctggtgaccttattggagtccataccggttcaaacaaactcggttctggtcttgtgacaacccctgaaggggagacctgctccatcaaggaaactaggctctctgacctttctagacattttgcaggtccaagcgtccctcttggggacattaagttgagcccagccatcatccctgatgtgacaactattccgagtgacttggcatcgctccttgcttctgtccccgtgatggaaggtggcctctcaactgtccagcttttgtgcgtctttttccttctctggcgcatgatgggccatgcctggacacccattgttgccgtaggcttctttttgctgaatgaaattctcccagcagtcttggtccgagctgtgttctcttttgcactctttgtacttgcatgggccaccccctggtcggcacaagtgttgatgattagactcctcacggcggctctcaaccgcaacaggttgtccctggcgttctacgcattcggaggtgtcgttggcctggccacagaaatcgggacttttgctggtggatggcctgaactgtcccaagccctctcgacatactgcttcctgcccaggttccttgctgtgactagttatgtccccaccatcatcatcggtgggctccatgccctcggcgtaattttgtggttattcaaataccgatgcctccacaacatgctggttggtgatgggagtttctcaagcgctttcttcctacggtattttgctgagggtaatcttaggaaaggcgtgtcgcagtcctgtggcatgaataacgaatccctgacagctgctttggcttgcaagttgtcgcaagctgaccttgattttttgtccagtttaacgaacttcaagtgctttgtgtccgcttcaaacatgaaaaatgcagctggccaatacatcgaggcggcgtatgctagagctctgcgtcaggagctggcctccttggttcaggttgacaagatgaaaggagtattggccaagctcgaggctttcgctgagacggccactccgtcacttgacacaggggacgtgattgttctgcttgggcaacacccccatggatccatcctcgacattaatgtggggggtgaaaggaaaactgtgtctgtgcaagaaacacgatgcctgggtggttccaaattcagtgtctgcactgtcgtgtccaacacgcccgtggataccttgaccggtatcccacttcagacgccaaccccactttttgaaaatggcccgcgccatcgcagcgaggacgacgacctcaaagttgagagaatgaaaaaacactgtgtatccctcggcttccacaaaatcaatggtaaagtttactgcaaaatttgggacaagtctaacggcgacaccttttacacggatgattcccgatacactcaagaccatgcttttcaggacaggtcaaccgactatagagacagggattatgaaggtgtacagaccgccccccaacagggattcgatccaaagtccgaagcccctgttggcactgttgtaatcggtggcattacgtataacaggcatctggtcaaaggtaaggaggtcctagttcccaaacctgacaactgccttgaagctgccagactgtcccttgagcaagctcttgctgggatgggccaaacttgtgaccttacagctaccgaagtggagaaactaaagcgcatcattagtcaactccaaggtctgaccactgaacaggctttaaactgctagccgccagcggcttgacccgctgtggccgcggcggcctagttgtaactgaaacggcggtaaaaatcgtaaaataccacagcagaactttcaccttaggctctttagacctaaaagtcacctccgaggtggaggtgaagaaatcaactgagcaggggcacgctgtcgtggcgaacttatgttccggtgtcgtcttgatgaggcctcacccaccgtcccttgttgacgttctcctcaaacccggacttgacacaacacccggcattcaaccagggcatggggccgggaatatgggcgtgaacggttctatttgggattttgaaactgcacccacaaaggtagaactagagttgtccaagcaaataatccaagcatgtgaagtcaggcgcggggacgcccctaacctccaactcccctacaagctttatcctgtcaggggggaccccgagcggcgtaaaggtcgccttgtcaacactaggtttggagatttaccttacaaaactccccaagacaccaagtccgcaattcatgcggcttgttgcctgcatcccaatggggtcctcgtgtctgatggcaaatccacgctgggtaccactcttcaacatggtttcgagctttatgtccccactgtaccttatagtgtcatggaataccttgattcacgccctgacaccccttttatgtgtactaaacatggcacttccaaggctgctgcagaggacctccaaaaatatgacctatccactcaagggtttgtcttgcctggggtcctacgcctagtgcgcaggttcatctttagccatgttggtaaggcgccaccactgttccttccatcaacctaccctgccaagaactccatggcaggggtcaatggccagaggttcccaacaaaggatgtccagagcatacctgaaattgatgaaatgtgcgcccgtgccgtcaaggaaaattggcagactgtgacaccttgcaccctcaaaaaacagtactgttccaaacctaaaactagaaccatcctaggtaccaacaacttcatagccttggctcacaggtcagcactcagtggtgtcacccaggcgttcatgaagaaggcctggaagtccccaattgccttggggaaaaacaagtttaaggaattgcattgcactgtcgccggcagatgccttgaggctgacctggcttcctgcgatcgcagcacccccgccattgtgaggtggtttgttgccaacctcctgtatgaacttgcaggatgtgaagagtacttgcctagctacgtgctcaactgttgccatgaccttgtggcaacgcaggatggcgctttcacaaaacgcggtggcctgtcgtccggggaccccgtcaccagtgtgtccaacaccgtctactcactgataatttacgcccagcacatggtgctttcggccttgaagatgggtcatgaaattggtctcaagttccttgaggaacagctcaaatttgaggaccttcttgaaatccagcccatgttagtgtattctgatgacctcgtcttgtatgcggaaagacccacttttcccaactaccattggtgggtcgagcatcttgacctgatgttgggctttaaaacggacccaaagaaaactgtcataactgataaacccagttttctcggctgcagaattgaagcaggacggcagttagtccccaatcgcgaccgtattctggctgctcttgcatatcatatgaaggcgcagaacgcctcagagtattatgcgtccgctgccgcaattctgatggattcgtgtgcttgcattgaccatgaccccgagtggtatgaggatcttatctgcggcatcgcccggtgtgctcgccaggacggttaccgttttccaggcccggcatttttcatgtccatgtgggagaagctgaaaagtcataatgaagggaagaaatgccgtcactgcggcatctgcgacgccaaagccgactatgcgtccgcctgtggacttgatttgtgtttgttccattcacactttcatcaacactgcccagtcactctgagctgtggccaccatgccggttcaaaggaatgttcgcagtgtcagtcacctgtcggggctggcaaatccccccttgacgctgtgctgaaacaaatcccgtacaaacctcctcgtaccattatcatgaaggtggacaacaaaacaacgacccttgacccgggaagatatcagtcccgtcgaggtcttgttgcagtcaaaagaggtattgcaggtaatgaggttgatctttctgatggagactaccaagtggtgcctcttttgccgacttgcaaagacataaacatggtgaaggtggcttgcaacgtactactcagcaagtttatagtagggccgccaggttccggaaaaaccacctggctactgaaccaagtccaggacgatgatgtcatttacacacctactcatcagacaatgtttgacatagtcagtgctcttaaagtttgcaggtattccatcccaggagcctcaggactcccttttccaccacctgccaggtccgggccgtgggttaggctcatcgccagcggacatgtccctggccgagtgtcatatctcgatgaggcaggatattgcaatcatctagacattctaaggctgctttccaaaacaccccttgtgtgtttgggtgaccttcagcaacttcacccggtcggctttgattcctattgttatgtgttcgatcagatgcctcagaagcagctgaccaccatttatagatttggccctaacatctgtgcagccatccagccttgttacagggagaaacttgaatccaaggccaggaacaccagagtggttttcaccacccggcctgtggcctttggtcaggtcctgacaccgtaccacaaagatcgtaccggctctgcaataactatagattcatcccagggggcgaccttcgacattgtgacattgcatctaccatcgccaaagtccctaaacaaatcccgagcacttgtagccatcactcgggcaagacatgggttgttcatttatgaccctcatgaccaactccaggagtttttcaacttaacccccgagcgcactgattgtaaccttgcgttcagccgtggggatgagctggttgttttgaatgtggataatgcggtcacaactgtagcgaaggccctagagacaggttcaccccgatttcgagtatcggacccgaggtgcaagtctctcttagccgcttgttcggccagtctagaagggagctgcatgccactaccacaagtagcacataacctggggttttacttttccccggacagcccagcttttgcacccctgccaaaagagctggcgccacattggccagtggtcacccaccagaataatcgagcgtggcctgatcgacttgtcgctagtatgcgcccaattgatgcccgctacagcaagccaatggtcggtgcagggtatgtggtcgggccatccatttttcttggcactcctggtgtggtgtcatactatctcacattatacatcgggggcgagcctcaggccctgccagaaacactcgtttcaacaggacgtatagccacagattgtcgggaatatctcgacgcggctgaggaagaggcagcgagagaacttccccacgcatttattggcgatgtcaaaggcactacgatcggggggtgtcaccacattacatcgaaatacctacctaggtccctgcctaaagactctgttgctgtggttggggtgagttcgcccggtagggctgctaaagccgtgtgcactctcaccgatgtgtacctccccgaactccgaccatatttgcaaccggagacggcatcaaaatgctggaaacttaaactggatttcagggatgttcgactgatggtctggaaaggcgccacagcctatttccagttggaagggctgacatggtcagcgctgcccgattatgctaggttcattcagctacccaaggatgccgttgtgtacatcgatccgtgtatagggccggcaacagccaatcgcaaggttgtgcgaaccacagactggcgggccgacctggcagtgacaccgtatgattacggtgctcaggtcattttgacaacagcctggttcgaggaccttgggccgcagtggaagattttggggttgcagcctttcagacgaacatttggctttgagaacactgaagattgggcaattctcgcacgccgtatgaatgacggcaaagattacactgactataattggcattgtgtacgagaacgcccacacgcaatttacgggcgcgcccgtgaccatacgtatcattttgcccttggcactgaactgcaagtagagctgggcagaccccggctgcctcctgagcaagtgccgtgaacgcggagtgatgcaatgggtttactgtggagtaaaatcagtcagttgttcgtggatgccttcactgagttccttgttagtgtggttgacattgtcatctttctcgccatattgtttgggttcactgttgcaggctggttattggtcttccttctcagagtggtttgctccgcgtttctccgttcgcgctctgccattcactcttccgaactatcgaaggtcctatgagggcttgctacccaactgcagaccggatgtcccacaattcgcagttaagcacccgttgggtatactttggcatatgcgagtctcccacctaattgacgaaatggtctctcgccgcatttaccggaccatggaacattcgggtcaagcggcctggaagcaggttgttagtgaagccactctcacaaaactgtcaaggcttgacgtagtcactcatttccaacacctggccgcagtggaggctgattcttgccgcttccttagctcacgactcgcgatgctgaaaaaccttgccgttggcaatgtgagcctggagtacaacactactttggaccgcgttgagctcatctttcccacaccaggtacgaggcccaagttgaccgattttaggcaatggcttatcagcgtgcacgcttccatcttctcctctgtggcttcgtctgttaccttgttcacagtgctttggcttcgaattccagctctacgctatgtttttggtttccattggcccacggcaacacatcattcgaactaactatcaattacactatatgtaagccatgccctaccagtcaagctgcccaacaaagactcgagcctggccgtaacgtgtggtgcaaaatagggcacgacaggtgtgaggaacgtgaccatgatgagttgtcaatgtccattccgtccgggtacgacaacctcaaacttgagggttattatgcttggctggcttttttgtccttttcctacgcggcccaattccatccggagctgttcggaataggaaacgtgtcgcgcgtctttgtggataagcgacaccagttcatttgcgccgagcatgatggacaaaattcaaccatatctgccagacacaacatctccgcgtcgtatgcggtgtattaccatcatcaaatagacgggggcaattggtttcatttggaatggctgcgaccattcttttcctcctggctggtgctcaacatctcatggtttctgaggcgttcgcctgcaagccctgcttctcgacgcatctatcagatattaagaccaacacgaccgcggctgccggtttcatggtccttcagaacatcaattgtttccaatctcacggtagctcccatttacagttgatttataacttaacgggctcatcccaatgtcgtgaagccgtcggcattccccagtacatcacgataacggctaatgtgaccgatgaatcgtatttgtacaacgcggacttgctgatgctttccgcgtgccttttctacgcctcggaaatgagcgagaaaggcttcaaagtcatctttgggaatatttctggcgttgtttccgcttgtgttaatttcacagattatgtggcccatgtgacccaacacactcagcagcaccatttggtaattgatcacattcggttactacacttcttgacaccgtctacgatgaggtgggctacaaccattgcttgtttgcttgccattcttttggcggtatgaaatgttcttgcaagttggggcatttcttgactcctcactcttgcttctggtggctttttttgctgtgtaccggcttgtcttggtcctttgtcgatggcaacgacgacagctcgacatcccaatacatatataatttgacgatatgcgagctgaatgggaccgaatggttgtccggtcattttgattgggcagtcgaaacctttgtgctttacccagttgccactcatatcatttcactgggttttctcacaacaagccatttccttgatgcgctcggtctcggcgctgtgtccgccacaggattcattggcgagcggtatgtacttagcagcatgtacggcgtttgcgccttcgcggcgttcgtatgttttgtcatccgtgctgctaaaaattgcatggcttgccgctatgcccgcacccggtttaccaacttcatcgtggacgaccggggaagaatccatcgatggaagtcttcaatagtggtggagaaattgggcaaagctgaagtcggtggtgaccttgtcaacattaagcatgttgtcctcgaaggggttaaagctcaacctttgacgaggacttcggctgagcaatgggaagcctagacgacttttgcaacgatcccaccgccgcacaaaaactcgtgctggcctttagcatcacatatacacccataatgatatacgcccttaaggtgtcacgcggccgactcctggggctgttgcacatcttgatatttctgaattgttcctttacttttgggtacatgacatatgtgcattttcaatccaccaaccgtgtcgcattcactctgggggctgtagtcgcccttttgtggggtgtttacagcctcacagagtcatggaagttcatcacttccagatgcagattgtgttgcctaggccggcgatacattctggcccctgcccatcacgtagaaagtgctgcaggcctccattcaatcccagcgtctggtaaccgagcatacgctgtgagaaagcccggactaacatcagtgaacggcactctagtacctgggcttcggagcctcgtgctgggcggcaaacgagctgttaaacgaggagtggttaacctcgtcaagtatggccggtaagaaccagagccagaagaaaagaagaaatgcagctccgatggggaaaggccagccagtcaatcaactgtgccagttgctgggtacaatgataaagtcccagcgccagcaatctaggggaggacaggccaaaaagaagaagcctgagaagccacattttcccctagctgctgaagatgacattcggcaccatctcacccaggccgaacgttccctctgcttgcaatcgatccagacggctttcaatcaaggcgcaggaactgcgtcgctttcatccagcgggaaggtcagtttccaggttgagttcatgctgccggttgctcatacagtgcgcctgattcgcgtgacttctacatccgccagtcagggtgcaaattaatttgacagtcaggtgaatggccgcgattgacgtgtggcctctaagtcacctattcaattagggcgatcacatgggggtcaaacttaattaggcaggaaccatgtgaccgaaattaaaaaaaaaaaaaaaaaaaaaaaaaaa

SEQ ID NO: 57 - DNA, 14984 bp, Artificial Sequence
  SEQ ID NO:49 with insert coding for SEQ ID NO:54
atgatgtgtagggtattccccctacatacacgacactcttagtgtttgtgtaccttggaggcgtgggtacagccctgccccaccctttggtccctgttctagcccgacaggtacccttctctctcggggcgagcgcgccgcctgctgctcccttgcggcgggaaggacctcccgagtatttccggagagcacctgctttacgggatctccgccctttaaccatgtctgggatgttctcccggtgcatgtgcaccccggctgcccgggtattttggaacgccggccaagtctattgcacacggtgtctcagtgcacggtctcttctctctccagaacttcaggacacggacctcggtgcagttggcttgtttcacaagcctaaagacaagctccattggaaagttcccattggtatcccccaggtggaatgttctccatctgggtgttgctggctgtcaaccatttttcctttagcgcgcatgacctccggcaatcacaacttccttcaacgactcgtgaaggttgctgatgtattgtaccgtgacggttgcttaacccctagacacctccgtgaactccaagtttacgagcgtggttgcaattggtatccgattacggggcctgtgcctgggatggctgtgtacgcgaactccatgcacgtgtccgaccaaccgttccctggtgccactcatgtgttaacaaattcccctttgcctcaacgggcttgtcggcagccgttctgtccgttcgaagaggcccattctagcatatacaggtgggaaaaatttgtaatttttatggattcctcctccgacggtcgatctcgcatgatgtggactccggaatccgatgactccacggctttggaagttctgccgcccgagctagaacaccaggtcaaggtccttgttcggagctttcccgcccatcaccttgtcgaccttgccgattgggagctcactgagtcccctgataacggtttttccttcagcacgtcacatccttgcggctaccttgttcgggacccggctgtatccgaaggcaagtgttggctttcctgctttttgagccagtcagccgaagtgctcagtcgcgaggcgcatctggctaccgcctatggttaccaaaccaagtggggtgtgcctggcaagtacatccagcgcagacttcaagttcacggtctccgtgctgtggtcgaccctgatggtcccattcacgttgaagcattgtcttgcccccagtcttggatcaggcacttgaccctgaatgatgatgtcaccccgggattcgttcgcctaatgtctcttcgcattgtgccgaacacagagcctaccacacaccggatctttcgttttggagtgcacaagtggtatggtgccgccggcaaacgggcccgtggcaagcgtgccgccaaaagtgagaaagactcggcttccaccctcaaggttgcccgaccgacttccaccagtggaatcgtcacctactccccacctgcggacgggtcttgtggttggcatgcccttgccgccatactgaaccggatgattaataatgacttcacgtcccctctgcctcggtacaacaggccggaggacgattgggcttctgatggtgaccttgctcaggccattcaatgtttgcaactacctgccgccatagctcggaaccgcgcctgccctaacgccaaatacctcataaaactcaacggagttcattgggaggtagaggtgaggcctggaatggctcctcgctccctctctcgtgagtgcgttgttggcgtctgctctgaaggctgtgtcgcgtcgccttacccggaggacgggttgcctaaacgtgcacttgaggccctggcgtctgcttatagactgccttcagactgtgtttgtgatggtattattgacttccttgccaatccacctccccaggagttctggactcttgacaaaatgttgacttccccgtcaccggagcagtccggcttctctagtctgtataaattgttgttagagatcttgccgcagaaatgcggatccacagaaggggaattcatctatactgttgagaggatgttgaaggattgtccgagctccaaacaggccatggccctccttgcaaaaattaaggtcccatcctcaaaggccccatccgtgactctgaacgagtgcttccccacggatgttccagtcaactctgagttaatatcttgggaagagcccaaagaccctggcgctgctgttgtcctatgtccatcggatgcaaaagaatctaaggaaacagcccctgaagaagctcaagcgagaaaccgtaaggtccttcaccctgtggtccttaccgaggaacttagcgagcaacaggtgcaggtggttgagggtgatcaggatatgccactggatttgacttggccaaccttaaccgctacggcgacccctgttagagggccggtaccggacaatttgagctctggcattggtgcccagcccgctaccgttcaagaactcattctggcgaggcctgcaccccgtcttgttgagcgctgtggcacggagtcgaacggcagcagttcatttctggatttgcctgacgtgcagacctcggaccagcctttagacctgtccctggccgcgtggcctgtaagggctaccgcgtctgaccccggttggatccacggtaggcgtgagcctgtctttgtgaagcctcgaggtgttttctctgatggcgagtcggcccttcagttcggagagctttccgaagccagttctgtcgtcgatgaccggacaaaagaagctccggtggttgacgcccccatcgatttgacaacttcgaacgagacgctctctgggtctgacccctttgaattcgccaaattcaggcgcccgcgtttctccgcgcaagctttaatcgaccgaggtggtccgcttgccgatgttcatgcaaagataaagagtcgggtatatgaacaatgccttcaagcttgtgaacctggtagtcgtgcgaccccagccaccaagaagtggctcgacaaaatgtgggacagggtggacatgaaaacttggcgctgcacctcgcagttccaagctggtcacattcttgagtccctcaaattcctccctgacatgattcaagacacaccgcctcctgttcccaggaagaaccgagctggtgacagtgccggcctgaagcaactggtggcgcagtgggataggaaatcgagtgtgacaccccccacaaaaccggttggaccggtgcttgaccaggccgtccctctgcctatggacatccagcaaggagatgccatctccgctgacaagccaccccattcgcaaaacccttctagtcaagtagatgtgggtggaggttggaaaagttttatgctctccggcacccgtttcgcggggtccgttagtcagcgccttacgacatgggtttttgaggttctctcccatctcccagcttttatgctcacacttttctcgccacggggctctatggctccaggtgattggctgtttgcaggtgctgttctacttgctctcctgctctgccgttcttacccaatactcggatgccttcccttattgggtgtcttttctggttctgtgcggtgtgttcgtttgggtgtttttggttcttggatggcttttgctgtatttttattctcgactccacccgacccagtcggttcttcttgtgaccacgattcgccggagtgtcatgctgagcttttggctcttgagcagcgccaactttgggaacctgtgcgcagccttgtggtcgggccatcgggcctcttatgcgtcattcttggcaagttactcggtgggtcacgttgtctctggtttgttctcctacgtatatgcatgctcgcagatttggcaatttctcttatttatgtggtgtcccaagggcgttgtcacaagtgttggggaaagtgtataaggacggctcctgcagaagtggcccttaatgtgtttcctttttcgcgcgccacccgctcatctcttgtgtccttgtgtgatcggttccaagcgccaaaaggagttgaccccgtgcacttggcgacaggctggcgcgggtgctggtgtggtgagagccctattcatcaatcacaccaaaaaccgatagcttatgccaacttggatgaaaagaagatatccgcccagacggtgattgctgtcccgtatgatcctagtcaggccattaaatgcctgaaagttttgcaggcaggaggggctattgtggaccagcctacgcccgaggtcgtccgtgtgtctgagattcccttctcggccccattttttccgaaggtcccagtcaacccagactgcagggttgtggtagattcggacacttttgtggctgcggtccgctgcggttattcgacagcacaactggtccttggtcggggcaactttgccaagctaaatcagacccccctcaggaactctgtccccaccaaaacaactggtggggcctcatacacccttgccgtggcccaggtatctgtgtggactcttgttcatttcatcctcggcctttggttaacgtcacctcaagtgtgtggtcgagggacctctgacccgtggtgttcgaaccctttttcgtatcctacttatggccccggagttgtgtgttcctctcgactctgcgtgtctgccgacggagttaccctgccattgttctcagccgttgcccatctttccggtagagaggtggggatttttattttggtgcttgcctccttgggcgctttagcccaccgcttggctcttaaggcagacatgtcaatggtctttttggcgttttgtgcttacgcctggcccatgagctcctggttaatttgcttctttcctatgctcttgaggtgggtaacccttcatcctctcactatgctttgggtgcactcatttttggtgttttgcctaccagctgccggcgttctctcgctgggaataaccggtcttctttgggcagttggccgtttcacccaggttgccggaattatcacaccttatgacatccaccagtatacctccggaccacgtggtgcagctgctgtagcaacggctccagaaggtacttacatggcggccgttcggagagccgctttgactggacggactttgatcttcacaccatctgcagtcggatcccttcttgaaggtgctttcagaactcaaaagccctgccttaacaccgtgaatgtcgtaggctcttcccttggttctggaggagttttcaccattgatggcagaagagtcatcgtcactgccacccatgtgttgaatggtaacacagccagggtcactggtgattcctacaaccgcatgcacacgttcaatactaatggtgattatgcctggtcccatgctgatgactggcaaggcgttgcccctatggttaagatcgctaaggggtatcgcggtcgtgcctactggcaaacgtcaaccggagtcgaacctggcatcatgggggaaggattcgccttctgtttcactaactgtggcgactcagggtcacctgtcatttcagaagctggtgaccttattggagtccataccggttcaaacaaactcggttctggtcttgtgacaacccctgaaggggagacctgctccatcaaggaaactaggctctctgacctttctagacattttgcaggtccaagcgtccctcttggggacattaagttgagcccagccatcatccctgatgtgacaactattccgagtgacttggcatcgctccttgcttctgtccccgtgatggaaggtggcctctcaactgtccagcttttgtgcgtctttttccttctctggcgcatgatgggccatgcctggacacccattgttgccgtaggcttctttttgctgaatgaaattctcccagcagtcttggtccgagctgtgttctcttttgcactctttgtacttgcatgggccaccccctggtcggcacaagtgttgatgattagactcctcacggcggctctcaaccgcaacaggttgtccctggcgttctacgcattcggaggtgtcgttggcctggccacagaaatcgggacttttgctggtggatggcctgaactgtcccaagccctctcgacatactgcttcctgcccaggttccttgctgtgactagttatgtccccaccatcatcatcggtgggctccatgccctcggcgtaattttgtggttattcaaataccgatgcctccacaacatgctggttggtgatgggagtttctcaagcgctttcttcctacggtattttgctgagggtaatcttaggaaaggcgtgtcgcagtcctgtggcatgaataacgaatccctgacagctgctttggcttgcaagttgtcgcaagctgaccttgattttttgtccagtttaacgaacttcaagtgctttgtgtccgcttcaaacatgaaaaatgcagctggccaatacatcgaggcggcgtatgctagagctctgcgtcaggagctggcctccttggttcaggttgacaagatgaaaggagtattggccaagctcgaggctttcgctgagacggccactccgtcacttgacacaggggacgtgattgttctgcttgggcaacacccccatggatccatcctcgacattaatgtggggggtgaaaggaaaactgtgtctgtgcaagaaacacgatgcctgggtggttccaaattcagtgtctgcactgtcgtgtccaacacgcccgtggataccttgaccggtatcccacttcagacgccaaccccactttttgaaaatggcccgcgccatcgcagcgaggacgacgacctcaaagttgagagaatgaaaaaacactgtgtatccctcggcttccacaaaatcaatggtaaagtttactgcaaaatttgggacaagtctaacggcgacaccttttacacggatgattcccgatacactcaagaccatgcttttcaggacaggtcaaccgactatagagacagggattatgaaggtgtacagaccgccccccaacagggattcgatccaaagtccgaagcccctgttggcactgttgtaatcggtggcattacgtataacaggcatctggtcaaaggtaaggaggtcctagttcccaaacctgacaactgccttgaagctgccagactgtcccttgagcaagctcttgctgggatgggccaaacttgtgaccttacagctaccgaagtggagaaactaaagcgcatcattagtcaactccaaggtctgaccactgaacaggctttaaactgctagccgccagcggcttgacccgctgtggccgcggcggcctagttgtaactgaaacggcggtaaaaatcgtaaaataccacagcagaactttcaccttaggctctttagacctaaaagtcacctccgaggtggaggtgaagaaatcaactgagcaggggcacgctgtcgtggcgaacttatgttccggtgtcgtcttgatgaggcctcacccaccgtcccttgttgacgttctcctcaaacccggacttgacacaacacccggcattcaaccagggcatggggccgggaatatgggcgtgaacggttctatttgggattttgaaactgcacccacaaaggtagaactagagttgtccaagcaaataatccaagcatgtgaagtcaggcgcggggacgcccctaacctccaactcccctacaagctttatcctgtcaggggggaccccgagcggcgtaaaggtcgccttgtcaacactaggtttggagatttaccttacaaaactccccaagacaccaagtccgcaattcatgcggcttgttgcctgcatcccaatggggtcctcgtgtctgatggcaaatccacgctgggtaccactcttcaacatggtttcgagctttatgtccccactgtaccttatagtgtcatggaataccttgattcacgccctgacaccccttttatgtgtactaaacatggcacttccaaggctgctgcagaggacctccaaaaatatgacctatccactcaagggtttgtcttgcctggggtcctacgcctagtgcgcaggttcatctttagccatgttggtaaggcgccaccactgttccttccatcaacctaccctgccaagaactccatggcaggggtcaatggccagaggttcccaacaaaggatgtccagagcatacctgaaattgatgaaatgtgcgcccgtgccgtcaaggaaaattggcagactgtgacaccttgcaccctcaaaaaacagtactgttccaaacctaaaactagaaccatcctaggtaccaacaacttcatagccttggctcacaggtcagcactcagtggtgtcacccaggcgttcatgaagaaggcctggaagtccccaattgccttggggaaaaacaagtttaaggaattgcattgcactgtcgccggcagatgccttgaggctgacctggcttcctgcgatcgcagcacccccgccattgtgaggtggtttgttgccaacctcctgtatgaacttgcaggatgtgaagagtacttgcctagctacgtgctcaactgttgccatgaccttgtggcaacgcaggatggcgctttcacaaaacgcggtggcctgtcgtccggggaccccgtcaccagtgtgtccaacaccgtctactcactgataatttacgcccagcacatggtgctttcggccttgaagatgggtcatgaaattggtctcaagttccttgaggaacagctcaaatttgaggaccttcttgaaatccagcccatgttagtgtattctgatgacctcgtcttgtatgcggaaagacccacttttcccaactaccattggtgggtcgagcatcttgacctgatgttgggctttaaaacggacccaaagaaaactgtcataactgataaacccagttttctcggctgcagaattgaagcaggacggcagttagtccccaatcgcgaccgtattctggctgctcttgcatatcatatgaaggcgcagaacgcctcagagtattatgcgtccgctgccgcaattctgatggattcgtgtgcttgcattgaccatgaccccgagtggtatgaggatcttatctgcggcatcgcccggtgtgctcgccaggacggttaccgttttccaggcccggcatttttcatgtccatgtgggagaagctgaaaagtcataatgaagggaagaaatgccgtcactgcggcatctgcgacgccaaagccgactatgcgtccgcctgtggacttgatttgtgtttgttccattcacactttcatcaacactgcccagtcactctgagctgtggccaccatgccggttcaaaggaatgttcgcagtgtcagtcacctgtcggggctggcaaatccccccttgacgctgtgctgaaacaaatcccgtacaaacctcctcgtaccattatcatgaaggtggacaacaaaacaacgacccttgacccgggaagatatcagtcccgtcgaggtcttgttgcagtcaaaagaggtattgcaggtaatgaggttgatctttctgatggagactaccaagtggtgcctcttttgccgacttgcaaagacataaacatggtgaaggtggcttgcaacgtactactcagcaagtttatagtagggccgccaggttccggaaaaaccacctggctactgaaccaagtccaggacgatgatgtcatttacacacctactcatcagacaatgtttgacatagtcagtgctcttaaagtttgcaggtattccatcccaggagcctcaggactcccttttccaccacctgccaggtccgggccgtgggttaggctcatcgccagcggacatgtccctggccgagtgtcatatctcgatgaggcaggatattgcaatcatctagacattctaaggctgctttccaaaacaccccttgtgtgtttgggtgaccttcagcaacttcacccggtcggctttgattcctattgttatgtgttcgatcagatgcctcagaagcagctgaccaccatttatagatttggccctaacatctgtgcagccatccagccttgttacagggagaaacttgaatccaaggccaggaacaccagagtggttttcaccacccggcctgtggcctttggtcaggtcctgacaccgtaccacaaagatcgtaccggctctgcaataactatagattcatcccagggggcgaccttcgacattgtgacattgcatctaccatcgccaaagtccctaaacaaatcccgagcacttgtagccatcactcgggcaagacatgggttgttcatttatgaccctcatgaccaactccaggagtttttcaacttaacccccgagcgcactgattgtaaccttgcgttcagccgtggggatgagctggttgttttgaatgtggataatgcggtcacaactgtagcgaaggccctagagacaggttcaccccgatttcgagtatcggacccgaggtgcaagtctctcttagccgcttgttcggccagtctagaagggagctgcatgccactaccacaagtagcacataacctggggttttacttttccccggacagcccagcttttgcacccctgccaaaagagctggcgccacattggccagtggtcacccaccagaataatcgagcgtggcctgatcgacttgtcgctagtatgcgcccaattgatgcccgctacagcaagccaatggtcggtgcagggtatgtggtcgggccatccatttttcttggcactcctggtgtggtgtcatactatctcacattatacatcgggggcgagcctcaggccctgccagaaacactcgtttcaacaggacgtatagccacagattgtcgggaatatctcgacgcggctgaggaagaggcagcgagagaacttccccacgcatttattggcgatgtcaaaggcactacgatcggggggtgtcaccacattacatcgaaatacctacctaggtccctgcctaaagactctgttgctgtggttggggtgagttcgcccggtagggctgctaaagccgtgtgcactctcaccgatgtgtacctccccgaactccgaccatatttgcaaccggagacggcatcaaaatgctggaaacttaaactggatttcagggatgttcgactgatggtctggaaaggcgccacagcctatttccagttggaagggctgacatggtcagcgctgcccgattatgctaggttcattcagctacccaaggatgccgttgtgtacatcgatccgtgtatagggccggcaacagccaatcgcaaggttgtgcgaaccacagactggcgggccgacctggcagtgacaccgtatgattacggtgctcaggtcattttgacaacagcctggttcgaggaccttgggccgcagtggaagattttggggttgcagcctttcagacgaacatttggctttgagaacactgaagattgggcaattctcgcacgccgtatgaatgacggcaaagattacactgactataattggcattgtgtacgagaacgcccacacgcaatttacgggcgcgcccgtgaccatacgtatcattttgcccttggcactgaactgcaagtagagctgggcagaccccggctgcctcctgagcaagtgccgtgaacgcggagtgatgcaatgggtttactgtggagtaaaatcagtcagttgttcgtggatgccttcactgagttccttgttagtgtggttgacattgtcatctttctcgccatattgtttgggttcactgttgcaggctggttattggtcttccttctcagagtggtttgctccgcgtttctccgttcgcgctctgccattcactcttccgaactatcgaaggtcctatgagggcttgctacccaactgcagaccggatgtcccacaattcgcagttaagcacccgttgggtatactttggcatatgcgagtctcccacctaattgacgaaatggtctctcgccgcatttaccggaccatggaacattcgggtcaagcggcctggaagcaggttgttagtgaagccactctcacaaaactgtcaaggcttgacgtagtcactcatttccaacacctggccgcagtggaggctgattcttgccgcttccttagctcacgactcgcgatgctgaaaaaccttgccgttggcaatgtgagcctggagtacaacactactttggaccgcgttgagctcatctttcccacaccaggtacgaggcccaagttgaccgattttaggcaatggcttatcagcgtgcacgcttccatcttctcctctgtggcttcgtctgttaccttgttcacagtgctttggcttcgaattccagctctacgctatgtttttggtttccattggcccacggcaacacatcattcgaactaactatcaattacactatatgtaagccatgccctaccagtcaagctgcccaacaaagactcgagcctggccgtaacgtgtggtgcaaaatagggcacgacaggtgtgaggaacgtgaccatgatgagttgtcaatgtccattccgtccgggtacgacaacctcaaacttgagggttattatgcttggctggcttttttgtccttttcctacgcggcccaattccatccggagctgttcggaataggaaacgtgtcgcgcgtctttgtggataagcgacaccagttcatttgcgccgagcatgatggacaaaattcaaccatatctgccagacacaacatctccgcgtcgtatgcggtgtattaccatcatcaaatagacgggggcaattggtttcatttggaatggctgcgaccattcttttcctcctggctggtgctcaacatctcatggtttctgaggcgttcgcctgcaagccctgcttctcgacgcatctatcagatattaagaccaacacgaccgcggctgccggtttcatggtccttcagaacatcaattgtttccaatctcacggtagctcccatttacagttgatttatcagttaacgggctcatcccaatgtcgtgaagccgtcggcattccccagtacatcacgataacggctaatgtgaccgatgaatcgtatttgtacaacgcggacttgctgatgctttccgcgtgccttttctacgcctcggaaatgagcgagaaaggcttcaaagtcatctttgggaatatttctggcgttgtttccgcttgtgttaatttcacagattatgtggcccatgtgacccaacacactcagcagcaccatttggtaattgatcacattcggttactacacttcttgacaccgtctacgatgaggtgggctacaaccattgcttgtttgcttgccattcttttggcggtatgaaatgttcttgcaagttggggcatttcttgactcctcactcttgcttctggtggctttttttgctgtgtaccggcttgtcttggtcctttgtcgatggcaacgacgacagctcgacatcccaatacatatataatttgacgatatgcgagctgaatgggaccgaatggttgtccggtcattttgattgggcagtcgaaacctttgtgctttacccagttgccactcatatcatttcactgggttttctcacaacaagccatttccttgatgcgctcggtctcggcgctgtgtccgccacaggattcattggcgagcggtatgtacttagcagcatgtacggcgtttgcgccttcgcggcgttcgtatgttttgtcatccgtgctgctaaaaattgcatggcttgccgctatgcccgcacccggtttaccaacttcatcgtggacgaccggggaagaatccatcgatggaagtcttcaatagtggtggagaaattgggcaaagctgaagtcggtggtgaccttgtcaacattaagcatgttgtcctcgaaggggttaaagctcaacctttgacgaggacttcggctgagcaatgggaagcctagacgacttttgcaacgatcccaccgccgcacaaaaactcgtgctggcctttagcatcacatatacacccataatgatatacgcccttaaggtgtcacgcggccgactcctggggctgttgcacatcttgatatttctgaattgttcctttacttttgggtacatgacatatgtgcattttcaatccaccaaccgtgtcgcattcactctgggggctgtagtcgcccttttgtggggtgtttacagcctcacagagtcatggaagttcatcacttccagatgcagattgtgttgcctaggccggcgatacattctggcccctgcccatcacgtagaaagtgctgcaggcctccattcaatcccagcgtctggtaaccgagcatacgctgtgagaaagcccggactaacatcagtgaacggcactctagtacctgggcttcggagcctcgtgctgggcggcaaacgagctgttaaacgaggagtggttaacctcgtcaagtatggccggtaagaaccagagccagaagaaaagaagaaatgcagctccgatggggaaaggccagccagtcaatcaactgtgccagttgctgggtacaatgataaagtcccagcgccagcaatctaggggaggacaggccaaaaagaagaagcctgagaagccacattttcccctagctgctgaagatgacattcggcaccatctcacccaggccgaacgttccctctgcttgcaatcgatccagacggctttcaatcaaggcgcaggaactgcgtcgctttcatccagcgggaaggtcagtttccaggttgagttcatgctgccggttgctcatacagtgcgcctgattcgcgtgacttctacatccgccagtcagggtgcaaattaatttgacagtcaggtgaatggccgcgattgacgtgtggcctctaagtcacctattcaattagggcgatcacatgggggtcaaacttaattaggcaggaaccatgtgaccgaaattaaaaaaaaaaaaaaaaaaaaaaaaaaa

SEQ ID NO: 58 - DNA, 14984 bp, Artificial Sequence
  SEQ ID NO:48 with deletion encoding ORF4 protein with deletion of 14 aa (aa 56-69), wherein insert coding for SEQ ID NO:55 is included
atgatgtgtagggtattccccctacatacacgacactcttagtgtttgtgtaccttggaggcgtgggtacagccctgccccaccctttggtccctgttctagcccgacaggtacccttctctctcggggcgagcgcgccgcctgctgctcccttgcggcgggaaggacctcccgagtatttccggagagcacctgctttacgggatctccgccctttaaccatgtctgggatgttctcccggtgcatgtgcaccccggctgcccgggtattttggaacgccggccaagtctattgcacacggtgtctcagtgcacggtctcttctctctccagaacttcaggacacggacctcggtgcagttggcttgtttcacaagcctaaagacaagctccattggaaagttcccattggtatcccccaggtggaatgttctccatctgggtgttgctggctgtcaaccatttttcctttagcgcgcatgacctccggcaatcacaacttccttcaacgactcgtgaaggttgctgatgtattgtaccgtgacggttgcttaacccctagacacctccgtgaactccaagtttacgagcgtggttgcaattggtatccgattacggggcctgtgcctgggatggctgtgtacgcgaactccatgcacgtgtccgaccaaccgttccctggtgccactcatgtgttaacaaattcccctttgcctcaacgggcttgtcggcagccgttctgtccgttcgaagaggcccattctagcatatacaggtgggaaaaatttgtaatttttatggattcctcctccgacggtcgatctcgcatgatgtggactccggaatccgatgactccacggctttggaagttctgccgcccgagctagaacaccaggtcaaggtccttgttcggagctttcccgcccatcaccttgtcgaccttgccgattgggagctcactgagtcccctgataacggtttttccttcagcacgtcacatccttgcggctaccttgttcgggacccggctgtatccgaaggcaagtgttggctttcctgctttttgagccagtcagccgaagtgctcagtcgcgaggcgcatctggctaccgcctatggttaccaaaccaagtggggtgtgcctggcaagtacatccagcgcagacttcaagttcacggtctccgtgctgtggtcgaccctgatggtcccattcacgttgaagcattgtcttgcccccagtcttggatcaggcacttgaccctgaatgatgatgtcaccccgggattcgttcgcctaatgtctcttcgcattgtgccgaacacagagcctaccacacaccggatctttcgttttggagtgcacaagtggtatggtgccgccggcaaacgggcccgtggcaagcgtgccgccaaaagtgagaaagactcggcttccaccctcaaggttgcccgaccgacttccaccagtggaatcgtcacctactccccacctgcggacgggtcttgtggttggcatgcccttgccgccatactgaaccggatgattaataatgacttcacgtcccctctgcctcggtacaacaggccggaggacgattgggcttctgatggtgaccttgctcaggccattcaatgtttgcaactacctgccgccatagctcggaaccgcgcctgccctaacgccaaatacctcataaaactcaacggagttcattgggaggtagaggtgaggcctggaatggctcctcgctccctctctcgtgagtgcgttgttggcgtctgctctgaaggctgtgtcgcgtcgccttacccggaggacgggttgcctaaacgtgcacttgaggccctggcgtctgcttatagactgccttcagactgtgtttgtgatggtattattgacttccttgccaatccacctccccaggagttctggactcttgacaaaatgttgacttccccgtcaccggagcagtccggcttctctagtctgtataaattgttgttagagatcttgccgcagaaatgcggatccacagaaggggaattcatctatactgttgagaggatgttgaaggattgtccgagctccaaacaggccatggccctccttgcaaaaattaaggtcccatcctcaaaggccccatccgtgactctgaacgagtgcttccccacggatgttccagtcaactctgagttaatatcttgggaagagcccaaagaccctggcgctgctgttgtcctatgtccatcggatgcaaaagaatctaaggaaacagcccctgaagaagctcaagcgagaaaccgtaaggtccttcaccctgtggtccttaccgaggaacttagcgagcaacaggtgcaggtggttgagggtgatcaggatatgccactggatttgacttggccaaccttaaccgctacggcgacccctgttagagggccggtaccggacaatttgagctctggcattggtgcccagcccgctaccgttcaagaactcattctggcgaggcctgcaccccgtcttgttgagcgctgtggcacggagtcgaacggcagcagttcatttctggatttgcctgacgtgcagacctcggaccagcctttagacctgtccctggccgcgtggcctgtaagggctaccgcgtctgaccccggttggatccacggtaggcgtgagcctgtctttgtgaagcctcgaggtgttttctctgatggcgagtcggcccttcagttcggagagctttccgaagccagttctgtcgtcgatgaccggacaaaagaagctccggtggttgacgcccccatcgatttgacaacttcgaacgagacgctctctgggtctgacccctttgaattcgccaaattcaggcgcccgcgtttctccgcgcaagctttaatcgaccgaggtggtccgcttgccgatgttcatgcaaagataaagagtcgggtatatgaacaatgccttcaagcttgtgaacctggtagtcgtgcgaccccagccaccaagaagtggctcgacaaaatgtgggacagggtggacatgaaaacttggcgctgcacctcgcagttccaagctggtcacattcttgagtccctcaaattcctccctgacatgattcaagacacaccgcctcctgttcccaggaagaaccgagctggtgacagtgccggcctgaagcaactggtggcgcagtgggataggaaatcgagtgtgacaccccccacaaaaccggttggaccggtgcttgaccaggccgtccctctgcctatggacatccagcaaggagatgccatctccgctgacaagccaccccattcgcaaaacccttctagtcaagtagatgtgggtggaggttggaaaagttttatgctctccggcacccgtttcgcggggtccgttagtcagcgccttacgacatgggtttttgaggttctctcccatctcccagcttttatgctcacacttttctcgccacggggctctatggctccaggtgattggctgtttgcaggtgctgttctacttgctctcctgctctgccgttcttacccaatactcggatgccttcccttattgggtgtcttttctggttctgtgcggtgtgttcgtttgggtgtttttggttcttggatggcttttgctgtatttttattctcgactccacccgacccagtcggttcttcttgtgaccacgattcgccggagtgtcatgctgagcttttggctcttgagcagcgccaactttgggaacctgtgcgcagccttgtggtcgggccatcgggcctcttatgcgtcattcttggcaagttactcggtgggtcacgttgtctctggtttgttctcctacgtatatgcatgctcgcagatttggcaatttctcttatttatgtggtgtcccaagggcgttgtcacaagtgttggggaaagtgtataaggacggctcctgcagaagtggcccttaatgtgtttcctttttcgcgcgccacccgctcatctcttgtgtccttgtgtgatcggttccaagcgccaaaaggagttgaccccgtgcacttggcgacaggctggcgcgggtgctggtgtggtgagagccctattcatcaatcacaccaaaaaccgatagcttatgccaacttggatgaaaagaagatatccgcccagacggtgattgctgtcccgtatgatcctagtcaggccattaaatgcctgaaagttttgcaggcaggaggggctattgtggaccagcctacgcccgaggtcgtccgtgtgtctgagattcccttctcggccccattttttccgaaggtcccagtcaacccagactgcagggttgtggtagattcggacacttttgtggctgcggtccgctgcggttattcgacagcacaactggtccttggtcggggcaactttgccaagctaaatcagacccccctcaggaactctgtccccaccaaaacaactggtggggcctcatacacccttgccgtggcccaggtatctgtgtggactcttgttcatttcatcctcggcctttggttaacgtcacctcaagtgtgtggtcgagggacctctgacccgtggtgttcgaaccctttttcgtatcctacttatggccccggagttgtgtgttcctctcgactctgcgtgtctgccgacggagttaccctgccattgttctcagccgttgcccatctttccggtagagaggtggggatttttattttggtgcttgcctccttgggcgctttagcccaccgcttggctcttaaggcagacatgtcaatggtctttttggcgttttgtgcttacgcctggcccatgagctcctggttaatttgcttctttcctatgctcttgaggtgggtaacccttcatcctctcactatgctttgggtgcactcatttttggtgttttgcctaccagctgccggcgttctctcgctgggaataaccggtcttctttgggcagttggccgtttcacccaggttgccggaattatcacaccttatgacatccaccagtatacctccggaccacgtggtgcagctgctgtagcaacggctccagaaggtacttacatggcggccgttcggagagccgctttgactggacggactttgatcttcacaccatctgcagtcggatcccttcttgaaggtgctttcagaactcaaaagccctgccttaacaccgtgaatgtcgtaggctcttcccttggttctggaggagttttcaccattgatggcagaagagtcatcgtcactgccacccatgtgttgaatggtaacacagccagggtcactggtgattcctacaaccgcatgcacacgttcaatactaatggtgattatgcctggtcccatgctgatgactggcaaggcgttgcccctatggttaagatcgctaaggggtatcgcggtcgtgcctactggcaaacgtcaaccggagtcgaacctggcatcatgggggaaggattcgccttctgtttcactaactgtggcgactcagggtcacctgtcatttcagaagctggtgaccttattggagtccataccggttcaaacaaactcggttctggtcttgtgacaacccctgaaggggagacctgctccatcaaggaaactaggctctctgacctttctagacattttgcaggtccaagcgtccctcttggggacattaagttgagcccagccatcatccctgatgtgacaactattccgagtgacttggcatcgctccttgcttctgtccccgtgatggaaggtggcctctcaactgtccagcttttgtgcgtctttttccttctctggcgcatgatgggccatgcctggacacccattgttgccgtaggcttctttttgctgaatgaaattctcccagcagtcttggtccgagctgtgttctcttttgcactctttgtacttgcatgggccaccccctggtcggcacaagtgttgatgattagactcctcacggcggctctcaaccgcaacaggttgtccctggcgttctacgcattcggaggtgtcgttggcctggccacagaaatcgggacttttgctggtggatggcctgaactgtcccaagccctctcgacatactgcttcctgcccaggttccttgctgtgactagttatgtccccaccatcatcatcggtgggctccatgccctcggcgtaattttgtggttattcaaataccgatgcctccacaacatgctggttggtgatgggagtttctcaagcgctttcttcctacggtattttgctgagggtaatcttaggaaaggcgtgtcgcagtcctgtggcatgaataacgaatccctgacagctgctttggcttgcaagttgtcgcaagctgaccttgattttttgtccagtttaacgaacttcaagtgctttgtgtccgcttcaaacatgaaaaatgcagctggccaatacatcgaggcggcgtatgctagagctctgcgtcaggagctggcctccttggttcaggttgacaagatgaaaggagtattggccaagctcgaggctttcgctgagacggccactccgtcacttgacacaggggacgtgattgttctgcttgggcaacacccccatggatccatcctcgacattaatgtggggggtgaaaggaaaactgtgtctgtgcaagaaacacgatgcctgggtggttccaaattcagtgtctgcactgtcgtgtccaacacgcccgtggataccttgaccggtatcccacttcagacgccaaccccactttttgaaaatggcccgcgccatcgcagcgaggacgacgacctcaaagttgagagaatgaaaaaacactgtgtatccctcggcttccacaaaatcaatggtaaagtttactgcaaaatttgggacaagtctaacggcgacaccttttacacggatgattcccgatacactcaagaccatgcttttcaggacaggtcaaccgactatagagacagggattatgaaggtgtacagaccgccccccaacagggattcgatccaaagtccgaagcccctgttggcactgttgtaatcggtggcattacgtataacaggcatctggtcaaaggtaaggaggtcctagttcccaaacctgacaactgccttgaagctgccagactgtcccttgagcaagctcttgctgggatgggccaaacttgtgaccttacagctaccgaagtggagaaactaaagcgcatcattagtcaactccaaggtctgaccactgaacaggctttaaactgctagccgccagcggcttgacccgctgtggccgcggcggcctagttgtaactgaaacggcggtaaaaatcgtaaaataccacagcagaactttcaccttaggctctttagacctaaaagtcacctccgaggtggaggtgaagaaatcaactgagcaggggcacgctgtcgtggcgaacttatgttccggtgtcgtcttgatgaggcctcacccaccgtcccttgttgacgttctcctcaaacccggacttgacacaacacccggcattcaaccagggcatggggccgggaatatgggcgtgaacggttctatttgggattttgaaactgcacccacaaaggtagaactagagttgtccaagcaaataatccaagcatgtgaagtcaggcgcggggacgcccctaacctccaactcccctacaagctttatcctgtcaggggggaccccgagcggcgtaaaggtcgccttgtcaacactaggtttggagatttaccttacaaaactccccaagacaccaagtccgcaattcatgcggcttgttgcctgcatcccaatggggtcctcgtgtctgatggcaaatccacgctgggtaccactcttcaacatggtttcgagctttatgtccccactgtaccttatagtgtcatggaataccttgattcacgccctgacaccccttttatgtgtactaaacatggcacttccaaggctgctgcagaggacctccaaaaatatgacctatccactcaagggtttgtcttgcctggggtcctacgcctagtgcgcaggttcatctttagccatgttggtaaggcgccaccactgttccttccatcaacctaccctgccaagaactccatggcaggggtcaatggccagaggttcccaacaaaggatgtccagagcatacctgaaattgatgaaatgtgcgcccgtgccgtcaaggaaaattggcagactgtgacaccttgcaccctcaaaaaacagtactgttccaaacctaaaactagaaccatcctaggtaccaacaacttcatagccttggctcacaggtcagcactcagtggtgtcacccaggcgttcatgaagaaggcctggaagtccccaattgccttggggaaaaacaagtttaaggaattgcattgcactgtcgccggcagatgccttgaggctgacctggcttcctgcgatcgcagcacccccgccattgtgaggtggtttgttgccaacctcctgtatgaacttgcaggatgtgaagagtacttgcctagctacgtgctcaactgttgccatgaccttgtggcaacgcaggatggcgctttcacaaaacgcggtggcctgtcgtccggggaccccgtcaccagtgtgtccaacaccgtctactcactgataatttacgcccagcacatggtgctttcggccttgaagatgggtcatgaaattggtctcaagttccttgaggaacagctcaaatttgaggaccttcttgaaatccagcccatgttagtgtattctgatgacctcgtcttgtatgcggaaagacccacttttcccaactaccattggtgggtcgagcatcttgacctgatgttgggctttaaaacggacccaaagaaaactgtcataactgataaacccagttttctcggctgcagaattgaagcaggacggcagttagtccccaatcgcgaccgtattctggctgctcttgcatatcatatgaaggcgcagaacgcctcagagtattatgcgtccgctgccgcaattctgatggattcgtgtgcttgcattgaccatgaccccgagtggtatgaggatcttatctgcggcatcgcccggtgtgctcgccaggacggttaccgttttccaggcccggcatttttcatgtccatgtgggagaagctgaaaagtcataatgaagggaagaaatgccgtcactgcggcatctgcgacgccaaagccgactatgcgtccgcctgtggacttgatttgtgtttgttccattcacactttcatcaacactgcccagtcactctgagctgtggccaccatgccggttcaaaggaatgttcgcagtgtcagtcacctgtcggggctggcaaatccccccttgacgctgtgctgaaacaaatcccgtacaaacctcctcgtaccattatcatgaaggtggacaacaaaacaacgacccttgacccgggaagatatcagtcccgtcgaggtcttgttgcagtcaaaagaggtattgcaggtaatgaggttgatctttctgatggagactaccaagtggtgcctcttttgccgacttgcaaagacataaacatggtgaaggtggcttgcaacgtactactcagcaagtttatagtagggccgccaggttccggaaaaaccacctggctactgaaccaagtccaggacgatgatgtcatttacacacctactcatcagacaatgtttgacatagtcagtgctcttaaagtttgcaggtattccatcccaggagcctcaggactcccttttccaccacctgccaggtccgggccgtgggttaggctcatcgccagcggacatgtccctggccgagtgtcatatctcgatgaggcaggatattgcaatcatctagacattctaaggctgctttccaaaacaccccttgtgtgtttgggtgaccttcagcaacttcacccggtcggctttgattcctattgttatgtgttcgatcagatgcctcagaagcagctgaccaccatttatagatttggccctaacatctgtgcagccatccagccttgttacagggagaaacttgaatccaaggccaggaacaccagagtggttttcaccacccggcctgtggcctttggtcaggtcctgacaccgtaccacaaagatcgtaccggctctgcaataactatagattcatcccagggggcgaccttcgacattgtgacattgcatctaccatcgccaaagtccctaaacaaatcccgagcacttgtagccatcactcgggcaagacatgggttgttcatttatgaccctcatgaccaactccaggagtttttcaacttaacccccgagcgcactgattgtaaccttgcgttcagccgtggggatgagctggttgttttgaatgtggataatgcggtcacaactgtagcgaaggccctagagacaggttcaccccgatttcgagtatcggacccgaggtgcaagtctctcttagccgcttgttcggccagtctagaagggagctgcatgccactaccacaagtagcacataacctggggttttacttttccccggacagcccagcttttgcacccctgccaaaagagctggcgccacattggccagtggtcacccaccagaataatcgagcgtggcctgatcgacttgtcgctagtatgcgcccaattgatgcccgctacagcaagccaatggtcggtgcagggtatgtggtcgggccatccatttttcttggcactcctggtgtggtgtcatactatctcacattatacatcgggggcgagcctcaggccctgccagaaacactcgtttcaacaggacgtatagccacagattgtcgggaatatctcgacgcggctgaggaagaggcagcgagagaacttccccacgcatttattggcgatgtcaaaggcactacgatcggggggtgtcaccacattacatcgaaatacctacctaggtccctgcctaaagactctgttgctgtggttggggtgagttcgcccggtagggctgctaaagccgtgtgcactctcaccgatgtgtacctccccgaactccgaccatatttgcaaccggagacggcatcaaaatgctggaaacttaaactggatttcagggatgttcgactgatggtctggaaaggcgccacagcctatttccagttggaagggctgacatggtcagcgctgcccgattatgctaggttcattcagctacccaaggatgccgttgtgtacatcgatccgtgtatagggccggcaacagccaatcgcaaggttgtgcgaaccacagactggcgggccgacctggcagtgacaccgtatgattacggtgctcaggtcattttgacaacagcctggttcgaggaccttgggccgcagtggaagattttggggttgcagcctttcagacgaacatttggctttgagaacactgaagattgggcaattctcgcacgccgtatgaatgacggcaaagattacactgactataattggcattgtgtacgagaacgcccacacgcaatttacgggcgcgcccgtgaccatacgtatcattttgcccttggcactgaactgcaagtagagctgggcagaccccggctgcctcctgagcaagtgccgtgaacgcggagtgatgcaatgggtttactgtggagtaaaatcagtcagttgttcgtggatgccttcactgagttccttgttagtgtggttgacattgtcatctttctcgccatattgtttgggttcactgttgcaggctggttattggtcttccttctcagagtggtttgctccgcgtttctccgttcgcgctctgccattcactcttccgaactatcgaaggtcctatgagggcttgctacccaactgcagaccggatgtcccacaattcgcagttaagcacccgttgggtatactttggcatatgcgagtctcccacctaattgacgaaatggtctctcgccgcatttaccggaccatggaacattcgggtcaagcggcctggaagcaggttgttagtgaagccactctcacaaaactgtcaaggcttgacgtagtcactcatttccaacacctggccgcagtggaggctgattcttgccgcttccttagctcacgactcgcgatgctgaaaaaccttgccgttggcaatgtgagcctggagtacaacactactttggaccgcgttgagctcatctttcccacaccaggtacgaggcccaagttgaccgattttaggcaatggcttatcagcgtgcacgcttccatcttctcctctgtggcttcgtctgttaccttgttcacagtgctttggcttcgaattccagctctacgctatgtttttggtttccattggcccacggcaacacatcattcgaactaactatcaattacactatatgtaagccatgccctaccagtcaagctgcccaacaaagactcgagcctggccgtaacgtgtggtgcaaaatagggcacgacaggtgtgaggaacgtgaccatgatgagttgtcaatgtccattccgtccgggtacgacaacctcaaacttgagggttattatgcttggctggcttttttgtccttttcctacgcggcccaattccatccggagctgttcggaataggaaacgtgtcgcgcgtctttgtggataagcgacaccagttcatttgcgccgagcatgatggacaaaattcaaccatatctgccagacacaacatctccgcgtcgtatgcggtgtattaccatcatcaaatagacgggggcaattggtttcatttggaatggctgcgaccattcttttcctcctggctggtgctcaacatctcatggtttctgaggcgttcgcctgcaagccctgcttctcgacgcatctatcagatattaagaccaacacgaccgcggctgccggtttcatggtccttcagaacatcaattgtttccaatctcccggtagctcccatttacagttgatttataacttaacgggctcatcccaatgtcgtgaagccgtcggcattccccagtacatcacgataacggctaatgtgaccgatgaatcgtatttgtacaacgcggacttgctgatgctttccgcgtgccttttctacgcctcggaaatgagcgagaaaggcttcaaagtcatctttgggaatatttctggcgttgtttccgcttgtgttaatttcacagattatgtggcccatgtgacccaacacactcagcagcaccatttggtaattgatcacattcggttactacacttcttgacaccgtctacgatgaggtgggctacaaccattgcttgtttgcttgccattcttttggcggtatgaaatgttcttgcaagttggggcatttcttgactcctcactcttgcttctggtggctttttttgctgtgtaccggcttgtcttggtcctttgtcgatggcaacgacgacagctcgacatcccaatacatatataatttgacgatatgcgagctgaatgggaccgaatggttgtccggtcattttgattgggcagtcgaaacctttgtgctttacccagttgccactcatatcatttcactgggttttctcacaacaagccatttccttgatgcgctcggtctcggcgctgtgtccgccacaggattcattggcgagcggtatgtacttagcagcatgtacggcgtttgcgccttcgcggcgttcgtatgttttgtcatccgtgctgctaaaaattgcatggcttgccgctatgcccgcacccggtttaccaacttcatcgtggacgaccggggaagaatccatcgatggaagtcttcaatagtggtggagaaattgggcaaagctgaagtcggtggtgaccttgtcaacattaagcatgttgtcctcgaaggggttaaagctcaacctttgacgaggacttcggctgagcaatgggaagcctagacgacttttgcaacgatcccaccgccgcacaaaaactcgtgctggcctttagcatcacatatacacccataatgatatacgcccttaaggtgtcacgcggccgactcctggggctgttgcacatcttgatatttctgaattgttcctttacttttgggtacatgacatatgtgcattttcaatccaccaaccgtgtcgcattcactctgggggctgtagtcgcccttttgtggggtgtttacagcctcacagagtcatggaagttcatcacttccagatgcagattgtgttgcctaggccggcgatacattctggcccctgcccatcacgtagaaagtgctgcaggcctccattcaatcccagcgtctggtaaccgagcatacgctgtgagaaagcccggactaacatcagtgaacggcactctagtacctgggcttcggagcctcgtgctgggcggcaaacgagctgttaaacgaggagtggttaacctcgtcaagtatggccggtaagaaccagagccagaagaaaagaagaaatgcagctccgatggggaaaggccagccagtcaatcaactgtgccagttgctgggtacaatgataaagtcccagcgccagcaatctaggggaggacaggccaaaaagaagaagcctgagaagccacattttcccctagctgctgaagatgacattcggcaccatctcacccaggccgaacgttccctctgcttgcaatcgatccagacggctttcaatcaaggcgcaggaactgcgtcgctttcatccagcgggaaggtcagtttccaggttgagttcatgctgccggttgctcatacagtgcgcctgattcgcgtgacttctacatccgccagtcagggtgcaaattaatttgacagtcaggtgaatggccgcgattgacgtgtggcctctaagtcacctattcaattagggcgatcacatgggggtcaaacttaattaggcaggaaccatgtgaccgaaattaaaaaaaaaaaaaaaaaaaaaaaaaaa